European Patent Specification EP 3 896 091 B1, published September 27, 2023. Title: CHIMERIC ANTIGEN RECEPTORS TARGETING BCMA AND METHODS OF USE THEREOF. Applicant: Legend Biotech Ireland Limited. Application Divisional Application of EP17838777.5. The sequence listing filed with the application follows.

SEQUENCE LISTING (399 sequences)

SEQ ID NO: 1 - protein, 6 aa, Artificial Sequence
  Synthetic Construct
DYYAIG

SEQ ID NO: 2 - protein, 5 aa, Artificial Sequence
  Synthetic Construct
TYGMA

SEQ ID NO: 3 - protein, 5 aa, Artificial Sequence
  Synthetic Construct
TFTMG

SEQ ID NO: 4 - protein, 5 aa, Artificial Sequence
  Synthetic Construct
INAMG

SEQ ID NO: 5 - protein, 5 aa, Artificial Sequence
  Synthetic Construct
SIVMG

SEQ ID NO: 6 - protein, 5 aa, Artificial Sequence
  Synthetic Construct
RAVIV

SEQ ID NO: 7 - protein, 5 aa, Artificial Sequence
  Synthetic Construct
SDVMG

SEQ ID NO: 8 - protein, 5 aa, Artificial Sequence
  Synthetic Construct
NDHMA

SEQ ID NO: 9 - protein, 5 aa, Artificial Sequence
  Synthetic Construct
KNTVA

SEQ ID NO: 10 - protein, 5 aa, Artificial Sequence
  Synthetic Construct
SHVMG

SEQ ID NO: 11 - protein, 5 aa, Artificial Sequence
  Synthetic Construct
TYFMA

SEQ ID NO: 12 - protein, 5 aa, Artificial Sequence
  Synthetic Construct
INVMA

SEQ ID NO: 13 - protein, 5 aa, Artificial Sequence
  Synthetic Construct
TFTMG

SEQ ID NO: 14 - protein, 5 aa, Artificial Sequence
  Synthetic Construct
INAMG

SEQ ID NO: 15 - protein, 5 aa, Artificial Sequence
  Synthetic Construct
KNTVA

SEQ ID NO: 16 - protein, 5 aa, Artificial Sequence
  Synthetic Construct
SIVMG

SEQ ID NO: 17 - protein, 5 aa, Artificial Sequence
  Synthetic Construct
TFTMG

SEQ ID NO: 18 - protein, 5 aa, Artificial Sequence
  Synthetic Construct
KNTVA

SEQ ID NO: 19 - protein, 5 aa, Artificial Sequence
  Synthetic Construct
INTMD

SEQ ID NO: 20 - protein, 5 aa, Artificial Sequence
  Synthetic Construct
KNTVA

SEQ ID NO: 21 - protein, 5 aa, Artificial Sequence
  Synthetic Construct
DYWMH

SEQ ID NO: 22 - protein, 5 aa, Artificial Sequence
  Synthetic Construct
SNTMA

SEQ ID NO: 23 - protein, 5 aa, Artificial Sequence
  Synthetic Construct
TFTMG

SEQ ID NO: 24 - protein, 6 aa, Artificial Sequence
  Synthetic Construct
VAAISL

SEQ ID NO: 25 - protein, 5 aa, Artificial Sequence
  Synthetic Construct
KNTVA

SEQ ID NO: 26 - protein, 5 aa, Artificial Sequence
  Synthetic Construct
TFTMG

SEQ ID NO: 27 - protein, 5 aa, Artificial Sequence
  Synthetic Construct
TFTMG

SEQ ID NO: 28 - protein, 5 aa, Artificial Sequence
  Synthetic Construct
SIVMG

SEQ ID NO: 29 - protein, 5 aa, Artificial Sequence
  Synthetic Construct
TFTMG

SEQ ID NO: 30 - protein, 5 aa, Artificial Sequence
  Synthetic Construct
TFTMG

SEQ ID NO: 31 - protein, 5 aa, Artificial Sequence
  Synthetic Construct
TFTMG

SEQ ID NO: 32 - protein, 5 aa, Artificial Sequence
  Synthetic Construct
TFTMG

SEQ ID NO: 33 - protein, 5 aa, Artificial Sequence
  Synthetic Construct
TFTMG

SEQ ID NO: 34 - protein, 5 aa, Artificial Sequence
  Synthetic Construct
NHVMG

SEQ ID NO: 35 - protein, 5 aa, Artificial Sequence
  Synthetic Construct
NYILA

SEQ ID NO: 36 - protein, 5 aa, Artificial Sequence
  Synthetic Construct
TFTMG

SEQ ID NO: 37 - protein, 5 aa, Artificial Sequence
  Synthetic Construct
TFTMG

SEQ ID NO: 38 - protein, 6 aa, Artificial Sequence
  Synthetic Construct
NNFVMG

SEQ ID NO: 39 - protein, 17 aa, Artificial Sequence
  Synthetic Construct
CISRSDGSTYYADSVKG

SEQ ID NO: 40 - protein, 19 aa, Artificial Sequence
  Synthetic Construct
SKASMNYSGRTYYADSVKG

SEQ ID NO: 41 - protein, 17 aa, Artificial Sequence
  Synthetic Construct
AISLSPTLAYYAESVKG

SEQ ID NO: 42 - protein, 16 aa, Artificial Sequence
  Synthetic Construct
SIRGLGRTNYDDSVKG

SEQ ID NO: 43 - protein, 17 aa, Artificial Sequence
  Synthetic Construct
AIMWNDGITYLQDSVKG

SEQ ID NO: 44 - protein, 17 aa, Artificial Sequence
  Synthetic Construct
FIKPSDGTIYYIDSLKG

SEQ ID NO: 45 - protein, 17 aa, Artificial Sequence
  Synthetic Construct
AIMWNDGITYLQDSVKG

SEQ ID NO: 46 - protein, 17 aa, Artificial Sequence
  Synthetic Construct
AIDWSGRTTNYADPVEG

SEQ ID NO: 47 - protein, 17 aa, Artificial Sequence
  Synthetic Construct
SITWDGRTTYYADSVKG

SEQ ID NO: 48 - protein, 17 aa, Artificial Sequence
  Synthetic Construct
VIGWRDISTSYADSVKG

SEQ ID NO: 49 - protein, 17 aa, Artificial Sequence
  Synthetic Construct
GIAWSGGSTAYADSVKG

SEQ ID NO: 50 - protein, 16 aa, Artificial Sequence
  Synthetic Construct
AVTRDGRKSCGDSVKG

SEQ ID NO: 51 - protein, 17 aa, Artificial Sequence
  Synthetic Construct
SITWDGRSAYYAESVKG

SEQ ID NO: 52 - protein, 16 aa, Artificial Sequence
  Synthetic Construct
TITRGGSTNYGPSVKG

SEQ ID NO: 53 - protein, 17 aa, Artificial Sequence
  Synthetic Construct
SITCDGRTTYYANSVNG

SEQ ID NO: 54 - protein, 17 aa, Artificial Sequence
  Synthetic Construct
AIMWNDGLTYLQGSVKG

SEQ ID NO: 55 - protein, 17 aa, Artificial Sequence
  Synthetic Construct
AISLSPTLAYYAESVKG

SEQ ID NO: 56 - protein, 17 aa, Artificial Sequence
  Synthetic Construct
SITWDGRTTYYADSVKG

SEQ ID NO: 57 - protein, 17 aa, Artificial Sequence
  Synthetic Construct
AISLSPTLAYYAESVKG

SEQ ID NO: 58 - protein, 17 aa, Artificial Sequence
  Synthetic Construct
SITCDGRTTYYANSVKG

SEQ ID NO: 59 - protein, 17 aa, Artificial Sequence
  Synthetic Construct
SIDTSGQTTYYADSLKG

SEQ ID NO: 60 - protein, 17 aa, Artificial Sequence
  Synthetic Construct
STTWNGRSTYYADSVKG

SEQ ID NO: 61 - protein, 15 aa, Artificial Sequence
  Synthetic Construct
DISGGRTNYADSVKG

SEQ ID NO: 62 - protein, 21 aa, Artificial Sequence
  Synthetic Construct
FTISRDNAKNTVVLQMNSLKP

SEQ ID NO: 63 - protein, 17 aa, Artificial Sequence
  Synthetic Construct
SITWDGRTTYYADSVKG

SEQ ID NO: 64 - protein, 17 aa, Artificial Sequence
  Synthetic Construct
AISLSPTLAYYAESVKG

SEQ ID NO: 65 - protein, 19 aa, Artificial Sequence
  Synthetic Construct
AISLSPTLAYYAESVKGKG

SEQ ID NO: 66 - protein, 17 aa, Artificial Sequence
  Synthetic Construct
AIMWNDGITYLQDSVKG

SEQ ID NO: 67 - protein, 17 aa, Artificial Sequence
  Synthetic Construct
AINLSPTLTYYAESVKG

SEQ ID NO: 68 - protein, 17 aa, Artificial Sequence
  Synthetic Construct
SITLIPTFPYYAYSVKG

SEQ ID NO: 69 - protein, 17 aa, Artificial Sequence
  Synthetic Construct
AISLSPTLAYYAESVKG

SEQ ID NO: 70 - protein, 17 aa, Artificial Sequence
  Synthetic Construct
AISLSPTLAYYAESVKG

SEQ ID NO: 71 - protein, 17 aa, Artificial Sequence
  Synthetic Construct
VIGWRDINASYADSVKG

SEQ ID NO: 72 - protein, 17 aa, Artificial Sequence
  Synthetic Construct
VIGWRDISTSYADSVKG

SEQ ID NO: 73 - protein, 17 aa, Artificial Sequence
  Synthetic Construct
HISRSGGKSGYGDSVKG

SEQ ID NO: 74 - protein, 17 aa, Artificial Sequence
  Synthetic Construct
AISLSPTLAYYAESVKG

SEQ ID NO: 75 - protein, 17 aa, Artificial Sequence
  Synthetic Construct
AISLSPTLAYYAEPVKG

SEQ ID NO: 76 - protein, 17 aa, Artificial Sequence
  Synthetic Construct
AISLSPTLAYYVESVKG

SEQ ID NO: 77 - protein, 14 aa, Artificial Sequence
  Synthetic Construct
AGADCSGYLRDYEF

SEQ ID NO: 78 - protein, 18 aa, Artificial Sequence
  Synthetic Construct
AGTGCSTYGCFDAQIIDY

SEQ ID NO: 79 - protein, 13 aa, Artificial Sequence
  Synthetic Construct
ADRKSVMSIRPDY

SEQ ID NO: 80 - protein, 13 aa, Artificial Sequence
  Synthetic Construct
VYVTLLGGVNRDY

SEQ ID NO: 81 - protein, 11 aa, Artificial Sequence
  Synthetic Construct
ASKGRYSEYEY

SEQ ID NO: 82 - protein, 17 aa, Artificial Sequence
  Synthetic Construct
ASPEDWYTDWIDWSIYR

SEQ ID NO: 83 - protein, 11 aa, Artificial Sequence
  Synthetic Construct
ASKGRYSEYEY

SEQ ID NO: 84 - protein, 12 aa, Artificial Sequence
  Synthetic Construct
VLRAWISYDNDY

SEQ ID NO: 85 - protein, 12 aa, Artificial Sequence
  Synthetic Construct
DLGKWPAGPADY

SEQ ID NO: 86 - protein, 11 aa, Artificial Sequence
  Synthetic Construct
ARRIDAADFDS

SEQ ID NO: 87 - protein, 11 aa, Artificial Sequence
  Synthetic Construct
SRGIEVEEFGA

SEQ ID NO: 88 - protein, 16 aa, Artificial Sequence
  Synthetic Construct
DGWGATTLDYTYGMDY

SEQ ID NO: 89 - protein, 12 aa, Artificial Sequence
  Synthetic Construct
DRKSVMSIRPDY

SEQ ID NO: 90 - protein, 14 aa, Artificial Sequence
  Synthetic Construct
ERLDGSGYGYEYDY

SEQ ID NO: 91 - protein, 12 aa, Artificial Sequence
  Synthetic Construct
YRKSIMSIQPDY

SEQ ID NO: 92 - protein, 12 aa, Artificial Sequence
  Synthetic Construct
DRKSVMSIRPDY

SEQ ID NO: 93 - protein, 10 aa, Artificial Sequence
  Synthetic Construct
RRIDAADFDS

SEQ ID NO: 94 - protein, 11 aa, Artificial Sequence
  Synthetic Construct
LGKWPAGPADY

SEQ ID NO: 95 - protein, 12 aa, Artificial Sequence
  Synthetic Construct
DRKSVMSIRPDY

SEQ ID NO: 96 - protein, 11 aa, Artificial Sequence
  Synthetic Construct
LGKWPAGSADY

SEQ ID NO: 97 - protein, 12 aa, Artificial Sequence
  Synthetic Construct
RYRGGTWYGMAN

SEQ ID NO: 98 - protein, 11 aa, Artificial Sequence
  Synthetic Construct
LGKWPAGPADY

SEQ ID NO: 99 - protein, 12 aa, Artificial Sequence
  Synthetic Construct
DRKSVMSIRPDY

SEQ ID NO: 100 - protein, 12 aa, Artificial Sequence
  Synthetic Construct
DRKSVMSIRPDY

SEQ ID NO: 101 - protein, 16 aa, Artificial Sequence
  Synthetic Construct
TASCHLFGLGSGAFVS

SEQ ID NO: 102 - protein, 10 aa, Artificial Sequence
  Synthetic Construct
SKDRYSEYEY

SEQ ID NO: 103 - protein, 8 aa, Artificial Sequence
  Synthetic Construct
KNGGPVDY

SEQ ID NO: 104 - protein, 10 aa, Artificial Sequence
  Synthetic Construct
SKGRYSEYEY

SEQ ID NO: 105 - protein, 12 aa, Artificial Sequence
  Synthetic Construct
ERKSVMAIPPDY

SEQ ID NO: 106 - protein, 12 aa, Artificial Sequence
  Synthetic Construct
YRKYLMSILPDY

SEQ ID NO: 107 - protein, 18 aa, Artificial Sequence
  Synthetic Construct
NRNSQRVIAALSWIGMNY

SEQ ID NO: 108 - protein, 10 aa, Artificial Sequence
  Synthetic Construct
RRIDAADFDS

SEQ ID NO: 109 - protein, 10 aa, Artificial Sequence
  Synthetic Construct
RRIDATDFDS

SEQ ID NO: 110 - protein, 10 aa, Artificial Sequence
  Synthetic Construct
RRIDAADFDS

SEQ ID NO: 111 - protein, 12 aa, Artificial Sequence
  Synthetic Construct
PLWYGSPTLIDY

SEQ ID NO: 112 - protein, 12 aa, Artificial Sequence
  Synthetic Construct
DRKSVMSIRPDY

SEQ ID NO: 113 - protein, 12 aa, Artificial Sequence
  Synthetic Construct
DRKSVMSIRPDY

SEQ ID NO: 114 - protein, 12 aa, Artificial Sequence
  Synthetic Construct
DRKSVMSIRPDY

SEQ ID NO: 115 - protein, 122 aa, Artificial Sequence
  Synthetic Construct
QVQLVESGGGLVQPGGSLRLSCEASGFTLDYYAIGWFRQAPGKEREGVICISRSDGSTYYADSVKGRFTISRDNAKKTVYLQMISLKPEDTAAYYCAAGADCSGYLRDYEFRGQGTQVTVSS

SEQ ID NO: 116 - protein, 128 aa, Artificial Sequence
  Synthetic Construct
QVKLEESGGRLVQPRGSLRLSCAGSGRTFSTYGMAWFRQAPGKEREFVASKASMNYSGRTYYADSVKGRFTIARDNAKNMVFLQMNNLKPEDTAVYYCAAGTGCSTYGCFDAQIIDYWGKGTLVTVSS

SEQ ID NO: 117 - protein, 118 aa, Artificial Sequence
  Synthetic Construct
EVQLVESGGGLVQAGGSLRLSCAASGRTFTMGWFRQAPGKEREFVAAISLSPTLAYYAESVKGRFTISRDNAKNTVVLQMNSLKPEDTALYYCAADRKSVMSIRPDYWGQGTQVTVSS

SEQ ID NO: 118 - protein, 120 aa, Artificial Sequence
  Synthetic Construct
AVQLVDSGGGLVQPGGSLRLSCVASGGIFVINAMGWYRQAPGKQRELVASIRGLGRTNYDDSVKGRFTISRDNANNTVYLQMNSLEPEDTAVYYCTVYVTLLGGVNRDYWGQGTQVTVSS

SEQ ID NO: 119 - protein, 119 aa, Artificial Sequence
  Synthetic Construct
EVQLVESGGGLVQAGGSLRLSCAASGRTFSSIVMGWFRQAPGKEREFVGAIMWNDGITYLQDSVKGRFTIFRDNAKNTVYLQMNSLKLEDTAVYYCAASKGRYSEYEYWGQGTQVTVSS

SEQ ID NO: 120 - protein, 128 aa, Artificial Sequence
  Synthetic Construct
EVQLVESGGGVVQAGGSLTVSCTASGFTFDRAVIVWFRQAPGKGREGVSFIKPSDGTIYYIDSLKGRFTISSDIAKNTVYLQMKSLESEDSAVYYCAASPEDWYTDWIDWSIYRWQHWGQGTQVTVSS

SEQ ID NO: 121 - protein, 119 aa, Artificial Sequence
  Synthetic Construct
EVQLVESGGGMVQAGDSLRLSCVQSTYTVNSDVMGWFRQAPGKEREFVGAIMWNDGITYLQDSVKGRFTIFRDNAKNTVYLQMNSLKLEDTAVYYCAASKGRYSEYEYWGQGTQVTVSS

SEQ ID NO: 122 - protein, 120 aa, Artificial Sequence
  Synthetic Construct
AVQLVESGGGLVQAGDSLRLSCTASGATLTNDHMAWFRQAPGKGREFVAAIDWSGRTTNYADPVEGRFTISRNNAKNTVYLEMNSLKLEDTAVYYCAVLRAWISYDNDYWGQGTQVTVSS

SEQ ID NO: 123 - protein, 120 aa, Artificial Sequence
  Synthetic Construct
QVQLVESGGGLVQAGGSLRLSCAASGGTLSKNTVAWFRQAPGKERGFVASITWDGRTTYYADSVKGRFTISRDNAKNTVYLQMNSLKPEDTAVYVCADLGKWPAGPADYWGQGTQVTVSS

SEQ ID NO: 124 - protein, 119 aa, Artificial Sequence
  Synthetic Construct
QVKLEESGGGLVQAGRSLRLSCAASEHTFSSHVMGWFRQAPGKERESVAVIGWRDISTSYADSVKGRFTISRDNAKKTLYLQMNSLKPEDTAVYYCAARRIDAADFDSWGQGTQVTVSS

SEQ ID NO: 125 - protein, 119 aa, Artificial Sequence
  Synthetic Construct
AVQLVESGGGLVQAGDSLRLTCTASGRAFSTYFMAWFRQAPGKEREFVAGIAWSGGSTAYADSVKGRFTISRDNAKNTVYLQMNSLKSEDTAVYYCASRGIEVEEFGAWGQGTQVTVSS

SEQ ID NO: 126 - protein, 124 aa, Artificial Sequence
  Synthetic Construct
EVQLVESGGGLVPPGGSLRLSCTASGSTVSINVMAWYRQVSGKQRELVAAVTRDGRKSCGDSVKGRFTISRDGAKNAVYLQMNSLKPEDTAVYLCGADGWGATTLDYTYGMDYWGKGTQVTVSS

SEQ ID NO: 127 - protein, 118 aa, Artificial Sequence
  Synthetic Construct
AVQLVESGGGLVQAGGSLRLSCAASGRTFTMGWFRQAPGKERGFVASITWDGRSAYYAESVKGRFTISRDNAKNTVVLQMNSLKPEDTALYYCAADRKSVMSIRPDYWGQGTQVTVSS

SEQ ID NO: 128 - protein, 122 aa, Artificial Sequence
  Synthetic Construct
QVQLVESGGGLVQPGGSLRLACEAPGSGNSINAMGWYRQTPGKRRELVATITRGGSTNYGPSVKGRFTITRDNVKNTVHLQMNSLKPDDTAVYYCNAERLDGSGYGYEYDYWGQGTQVTVSS

SEQ ID NO: 129 - protein, 121 aa, Artificial Sequence
  Synthetic Construct
QVKLEESGGGLVQAGGSLRLSCAASGGTLSKNTVAWVRQAPGKERGFVTSITCDGRTTYYANSVNGRFPINRNNAENLVVLQMNSLKPDDTALYYCAAYRKSIMSIQPDYWGQGTQVTVSS

SEQ ID NO: 130 - protein, 121 aa, Artificial Sequence
  Synthetic Construct
DVQLVESGGGLVQAGGSLRLSCAASGRTFSSIVMGWFRQAPGKEREFVGAIMWNDGLTYLQGSVKGRFTISRDNAKNTVVLQMNSLKPEDTALYYCAADRKSVMSIRPDYWGQGTQVTVSS

SEQ ID NO: 131 - protein, 116 aa, Artificial Sequence
  Synthetic Construct
QVQLVESGGGLVQAGGSLRLSCAASGRTFTMGWFRQAPGKEREFVAAISLSPTLAYYAESVKGRFTISRDNAKNTVVLQMNSLKPEDTAVYYCAARRIDAADFDSWGQGTQVTVSS

SEQ ID NO: 132 - protein, 120 aa, Artificial Sequence; identical to SEQ ID NO: 123
  Synthetic Construct

SEQ ID NO: 133 - protein, 121 aa, Artificial Sequence
  Synthetic Construct
QVQLVESGGGLVQPGGSLTLSCAASGSIDSINTMDWFRQAPGKEREFVAAISLSPTLAYYAESVKGRFTISRDNAKNTVVLQMNSLKPEDTALYYCAADRKSVMSIRPDYWGQGTQVTVSS

SEQ ID NO: 134 - protein, 120 aa, Artificial Sequence
  Synthetic Construct
DVQLVESGGGLVQAGGSLRLSCAASGGTLSKNTVAWVRQAPGKERGFVTSITCDGRTTYYANSVKGRFPISRDNAENTVYLQMNSLKPEDTAGYVCADLGKWPAGSADYWGQGTHVTVSS

SEQ ID NO: 135 - protein, 121 aa, Artificial Sequence
  Synthetic Construct
QVKLEESGGGLVQPGGSLRLSCTASEFTFSDYWMHWVRQAPGKGLEWVASIDTSGQTTYYADSLKGRFTISRDNAKSTLYLQMNSLKSEDTGVYFCAKRYRGGTWYGMANWGKGTQVTVSS

SEQ ID NO: 136 - protein, 120 aa, Artificial Sequence
  Synthetic Construct
QVQLVESGGGLVQAGGSLRLSCAASGRTLSSNTMAWFRQAPGKEREFVASTTWNGRSTYYADSVKGRFTISRDNAKNTMYLQMNSLKPEDTAVYVCADLGKWPAGPADYWGQGTQVTVSS

SEQ ID NO: 137 - protein, 116 aa, Artificial Sequence
  Synthetic Construct
QVQLVESGGGLVQAGGSLRLSCAASGRTFTMGWFRQAPGKQRELVADISGGRTNYADSVKGRFTISRDNAKNTVYLQMNSLKPEDTAVYYCAADRKSVMSIRPDYWGQGTQVTVSS

SEQ ID NO: 138 - protein, 104 aa, Artificial Sequence
  Synthetic Construct
QVQLVESGGGLVQAGASLRLSCAASGRTFTVAAISLSPTLAYYAESVKGRFTISRDNAKNTVVLQMNSLKPEDTALYYCAADRKSVMSIRPDYWGQGTQVTVSS

SEQ ID NO: 139 - protein, 125 aa, Artificial Sequence
  Synthetic Construct
DVQLVESGGGLEQAGGSLRLSCAASGGTLSKNTVAWFRQAPGKERGFVASITWDGRTTYYADSVKGRFTISRDNAKNTVYLQMNSLKPEDTAVYYCASTASCHLFGLGSGAFVSWGRGTQVTVSS

SEQ ID NO: 140 - protein, 116 aa, Artificial Sequence
  Synthetic Construct
AVQLVESGGGLVQAGGSLRLSCAASGRTFTMGWFHQAPGKEREFVAAISLSPTLAYYAESVKGRFTISRDNAKNTVVLQMNSLKPEDTALYYCAASKDRYSEYEYWGQGTQVTVSS

SEQ ID NO: 141 - protein, 114 aa, Artificial Sequence
  Synthetic Construct
QVKLEESGGGLVQAGGSLRLSCAASGRTFTMGWFRQAPGKEREFVAAISLSPTLAYYAESVKGRFTISRDNAKNTVVLQMNSLKPEDTALYYCAKKNGGPVDYWGKGTQVTVSS

SEQ ID NO: 142 - protein, 119 aa, Artificial Sequence
  Synthetic Construct
DVQLVESGGGLVQPGGSLRLSCAASGRTFSSIVMGWFRQAPGKEREFVGAIMWNDGITYLQDSVKGRFTIFRDNAKNTVYLQMNSLKLEDTAVYYCAASKGRYSEYEYWGQGTQVTVSS

SEQ ID NO: 143 - protein, 118 aa, Artificial Sequence
  Synthetic Construct
QVKLEESGGRLVQAGGSLKLSWAASGRTFTMGWFRQAPGKEREFVTAINLSPTLTYYAESVKGRFPISRNNAQNTVVLQMNSLKPEDTALYYCAAERKSVMAIPPDYWGQGTQVTVSS

SEQ ID NO: 144 - protein, 118 aa, Artificial Sequence
  Synthetic Construct
EVQLVESGGGLVQAGGSLRLSCAASGRTFTMGGFRRVPRDEREFVASITLIPTFPYYAYSVKGRFALFRDNPNNTVILLMISLKPEDPDLYYCASYRKYLMSILPDYWGQGTQGTVSS

SEQ ID NO: 145 - protein, 124 aa, Artificial Sequence
  Synthetic Construct
QVKLEESGGGLVQAGGSLRLSCAASGRTFTMGWFRQAPGKEREFVAAISLSPTLAYYAESVKGRFTISRDNAKNTVDLQMNSLKPEDTAVYFCAANRNSQRVIAALSWIGMNYWGEWTQVTVSS

SEQ ID NO: 146 - protein, 116 aa, Artificial Sequence
  Synthetic Construct
QVQLVESGGGLVQAGGSLRLSCAASGRTFTMGWFRQAPGKEREFVAAISLSPTLAYYAESVKGRFTISRDNAKKTLYLRMNSLKPEDTAVYYCAARRIDAADFDSWGQGTQVTVSS

SEQ ID NO: 147 - protein, 116 aa, Artificial Sequence
  Synthetic Construct
QVKLEESGGGLVQAGGSLRLSCAASGRTFTMGWFRRAPGKERESVAVIGWRDINASYADSVKGRFAISRDNAKKTLYLQMNSLKPEDTAVYYCAARRIDATDFDSWGQGTQVTVSS

SEQ ID NO: 148 - protein, 119 aa, Artificial Sequence
  Synthetic Construct
QVKLEESGGGLVQTGGSLRLSCAASEHTFSNHVMGWFRQAPGKERESVAVIGWRDISTSYADSVKGRFTISRDNAKKTLYLQMNSLKPEDTAVYYCAARRIDAADFDSRGQGTQVTVSS

SEQ ID NO: 149 - protein, 123 aa, Artificial Sequence
  Synthetic Construct
AVQLVDSGGGLVQAGGSLRISCAVSGRTSSNYILAWFRQAPGKERDFVAHISRSGGKSGYGDSVKGRFTISRDNAENTVRVYLQMNSLKPGDTAVYYCNRPLWYGSPTLIDYWGQGTQVTVSS

SEQ ID NO: 150 - protein, 118 aa, Artificial Sequence
  Synthetic Construct
QVQLVESGGGLVQAGGSLRLSCAASGRTFTMGWFRQAPGKEREFVAAISLSPTLAYYAESVKGRFTISRDNAKNTVVLQMNSLKPEDTALYYCAADRKSVMSIRPDYWGQGTQVTVSS

SEQ ID NO: 151 - protein, 118 aa, Artificial Sequence
  Synthetic Construct
AVQLVDSGGGLVQAGGSLRLSCAASGRTFTMGWFRQAPGKEREFVAAISLSPTLAYYAEPVKGRFTISRDNAKNTVVLQMNSLKPEDTALYYCAADRKSVMSIRPDYWGQGTQVTVSS

SEQ ID NO: 152 - protein, 121 aa, Artificial Sequence
  Synthetic Construct
DVQLVESGGGSVQTGGSLRLSCTASGRTLNNFVMGWFRQAPGKEREFVAAISLSPTLAYYVESVKGRFTISRDNAKNTVVLQMNSLKPEDTALYYCAADRKSVMSIRPDYWGQGTQVTVSS

SEQ ID NO: 153 - DNA, 366 bp, Artificial Sequence
  Synthetic Construct
caggtgcagctggtggagtctgggggaggcttggtgcagcctgggggttctctgaggctctcctgtgaagcctctggattcactttggattattatgccataggctggttccgccaggccccagggaaggagcgcgagggggtcatatgtattagtagaagtgatggtagcacatactatgcagactccgtgaagggccgattcaccatctccagagacaacgccaagaaaacggtgtatctgcaaatgatcagcctgaaacctgaggacacggccgcttattactgtgcagcaggggccgattgttcggggtacctacgagattatgagttccgggggcaggggacccaggtcaccgtctcctca

SEQ ID NO: 154 - DNA, 384 bp, Artificial Sequence
  Synthetic Construct
caggtaaagctggaggagtctgggggacgattggtgcagccaaggggctctctgagactctcctgtgcaggctctggacgcactttcagtacctatggtatggcctggttccgccaggctccagggaaggagcgtgagttcgtagcgtctaaagcatcgatgaattacagcggtagaacatactatgcagactccgtgaagggccgattcaccatcgccagagacaacgccaagaacatggtgtttctgcaaatgaacaacctgaagcctgaggacacggccgtttattactgtgcagcgggcactggatgctcaacatatgggtgttttgacgcccagataatagactactggggcaaagggaccctggtcaccgtctcctca

SEQ ID NO: 155 - DNA, 354 bp, Artificial Sequence
  Synthetic Construct
gaggtgcagctggtggagtctgggggaggcttggtgcaggctggggggtctctgagactctcctgtgcagcctctggacgcaccttcaccatggggtggttccgtcaggctccagggaaggagcgtgagtttgtagcagctattagtttgagtcctactttagcatattatgcagagtccgtgaagggccgattcaccatcagccgagacaacgccaagaacacggtggttttgcaaatgaacagcctgaaacctgaggacacggccctttattactgtgcagcagaccggaaatcagtaatgtctattcggcccgactactggggccaggggacccaggtcaccgtctcctca

SEQ ID NO: 156 - DNA, 360 bp, Artificial Sequence
  Synthetic Construct
gccgtgcagctggtggattctgggggaggcttggtgcagcctggggggtctctgagactctcctgtgtagcctctggaggtatcttcgtcatcaatgccatgggctggtaccgccaggctccaggaaagcagcgcgagttggtcgcatctattcgtggactaggcagaacaaactatgacgactccgtgaagggccgattcaccatctccagagacaacgccaacaacacggtgtatctgcagatgaacagcctggaacctgaggacacggccgtctactactgtacagtctacgttacactacttggtggggttaatagggactactggggccaggggacccaggtcaccgtctcctca

SEQ ID NO: 157 - DNA, 357 bp, Artificial Sequence
  Synthetic Construct
gaggtgcagctggtggagtctgggggaggattggtgcaggctgggggctctctgagactctcctgtgcagcctctggacggaccttcagtagcattgtcatgggctggttccgccaggctccagggaaggagcgtgagtttgtaggagcgattatgtggaatgatggtattacatacttgcaagactccgtgaagggccgatttaccatcttcagagacaatgccaagaacacggtgtatctgcaaatgaacagcctgaaacttgaggatacggccgtttattactgtgcagcatccaagggtagatactcggaatatgagtactggggccaggggacccaggtcaccgtctcctca

SEQ ID NO: 158 - DNA, 384 bp, Artificial Sequence
  Synthetic Construct
gaggtgcagctggtggagtctgggggaggcgtggtgcaggctggggggtctctgacagtctcctgtacagcctctggattcactttcgaccgtgctgtcatagtctggttccgccaggcccccgggaagggccgtgagggggtctcatttattaaacctagtgatggcaccatatactacattgactccctgaagggccgattcacgatctccagtgacatcgccaagaatacggtatatctgcaaatgaaaagtctggaatcggaggactcggccgtttattactgtgcggcctcgcctgaggactggtacacggattggatcgactggagtatatatcggtggcagcactggggccaggggacccaggtcactgtctcctca

SEQ ID NO: 159 - DNA, 357 bp, Artificial Sequence
  Synthetic Construct
gaggtgcagctggtggagtctgggggaggaatggtgcaggctggggactctctgagactatcctgtgtgcagtctacttacaccgtcaatagcgatgtcatgggctggttccgccaggctccagggaaggagcgtgagtttgtaggagcgattatgtggaatgatggtattacatacttgcaagactccgtgaagggccgatttaccatcttcagagacaacgccaagaacacggtgtatctgcaaatgaacagcctgaaacttgaggatacggccgtttattactgtgcagcatccaagggtagatactcggaatatgagtactggggccaggggacccaggtcaccgtctcctca

SEQ ID NO: 160 - DNA, 360 bp, Artificial Sequence
  Synthetic Construct
gcggtgcagctggtggagtctgggggaggattggtgcaggctggggactctctgagactctcctgtacagcctctggtgcaaccttgactaacgatcacatggcatggttccgccaggctccagggaaggggcgtgaatttgtagcagctattgactggagtggtcgtaccacaaattacgcagaccccgtagagggccgattcaccatctccagaaacaacgccaagaacacggtgtatctggaaatgaacagcctgaaacttgaggacacggccgtttattactgtgcggtcctccgcgcttggatctcatatgacaatgactactggggccaggggacccaggtcaccgtctcctca

SEQ ID NO: 161 - DNA, 360 bp, Artificial Sequence
  Synthetic Construct
caggtgcagctggtggagtctgggggaggattggtgcaggctgggggctctctgagactctcctgtgcagcctctggaggcaccttaagtaaaaataccgtggcttggttccgccaggctccagggaaggagcgtgggtttgtagcgtctattacctgggatggtcgtacgacatactatgcagactccgtgaagggccgattcaccatctccagagacaacgccaagaacacagtgtatctgcaaatgaacagcctgaaacctgaggatacggccgtttatgtctgtgcagacttagggaaatggcctgcgggcccggcggactactggggccaggggacccaggtcaccgtctcctca

SEQ ID NO: 162 - DNA, 357 bp, Artificial Sequence
  Synthetic Construct
caggtaaagctggaggagtctgggggaggcttggtgcaggctgggcggtctctgagactctcctgtgcagcctctgaacacaccttcagtagccatgtcatgggctggttccgccaggctccagggaaggagcgtgagtctgttgcagttattggctggagagatattagcacaagctatgcagactccgtgaagggccgattcaccatctccagagacaacgccaagaagacgctgtatctgcaaatgaatagcctgaaacctgaggacacggccgtttactactgtgcagcacgtcggatcgacgcagctgactttgattcctgggggcaggggacccaggtcaccgtctcctcg

SEQ ID NO: 163 - DNA, 357 bp, Artificial Sequence
  Synthetic Construct
gcggtgcagctggtggagtctgggggaggattggtgcaggctggggactctctgagactcacctgtacagcctctggacgcgccttcagtacctatttcatggcctggttccgccaggctccagggaaggagcgtgagtttgtagcaggaattgcatggagtggtggtagcacggcgtatgcagactccgtgaagggccgattcaccatctccagagacaacgccaagaacacggtgtatctgcaaatgaacagcctgaaatctgaggacacggccgtttattactgtgccagcagggggattgaggtcgaagagtttggtgcctggggccaggggacccaggtcaccgtctcgtcg

SEQ ID NO: 164 - DNA, 372 bp, Artificial Sequence
  Synthetic Construct
gaggtgcagctggtggagtctgggggaggcttggtgccgcctggggggtctctgagactctcctgtacagcctctggaagcacagtcagcatcaatgtcatggcctggtaccgccaggtttcagggaagcagcgcgagttggtcgcggccgttactagggatggtaggaaaagttgtggagactccgtgaagggccgattcaccatttccagagacggcgccaagaatgcggtatatttgcaaatgaacagtctgaaacctgaggacacagcggtctatttatgtggagccgatggttggggtgctactaccttagattatacctacggcatggactattggggcaaagggacccaggtcaccgtctcctca

SEQ ID NO: 165 - DNA, 354 bp, Artificial Sequence
  Synthetic Construct
gcggtgcagctggtggagtctgggggaggattggtgcaggctgggggctctctgagactctcctgtgcagcctctggacgcaccttcaccatggggtggttccgtcaggctccagggaaggagcgtgggtttgtagcgtctattacctgggatggtcgttcggcatactatgcagagtccgtgaagggccgattcaccatcagccgagacaacgccaagaacacggtggttttgcaaatgaacagcctgaaacctgaggacacggccctttattactgtgcagcagaccggaaatcagtaatgtctattcggcccgactactggggccaggggacccaggtcaccgtctcctca

SEQ ID NO: 166 - DNA, 366 bp, Artificial Sequence
  Synthetic Construct
caggtacagctggtggagtctgggggaggattggtgcagcctggggggtctctaagactcgcatgtgaagcgcctggaagcggcaatagtatcaatgccatgggctggtaccggcagactccggggaagcggcgcgagttggtcgcaactattactcggggtggtagcacgaactatggaccctccgtgaagggccgattcacgatcaccagagacaatgtcaagaatacggtgcatctgcagatgaacagcctgaaacctgacgacacggccgtctattattgcaatgcggagaggctggacggctcggggtacggatatgagtatgattactggggccaggggacccaggtcaccgtctcctca

SEQ ID NO: 167 - DNA, 363 bp, Artificial Sequence
  Synthetic Construct
caggtaaagctggaggagtctgggggaggattggtgcaggctgggggctctctgagactctcctgtgcagcctctggaggcaccttaagtaagaataccgtggcttgggtccgccaggctccagggaaggagcgtgggtttgtaacgtctattacctgtgatggtcgtacgacatactatgcgaactccgtaaacggccgattccccatcaaccgaaacaacgccgagaatttggtggttttgcaaatgaacagcctgaaacctgacgacacggccctttattactgtgcagcataccggaagtcaataatgtctattcagcccgactactggggccaggggacccaggtcaccgtctcctca

SEQ ID NO: 168 - DNA, 363 bp, Artificial Sequence
  Synthetic Construct
gatgtgcagctggtggagtctgggggaggattggtgcaggctgggggctctctgagactctcctgtgcagcctctggacggaccttcagtagcattgtcatgggctggttccgccaggctccagggaaggagcgtgagtttgtaggagcgattatgtggaatgatggtctgacatacttgcaagggtccgtgaagggccgattcaccatttccagagacaacgccaagaacacggtggttttgcaaatgaacagcctgaaacctgaggacacggccctttattactgtgcagcagaccggaaatcagtaatgtctattcggcccgactactggggccaggggacccaggtcaccgtctcctca

SEQ ID NO: 169 - DNA, 348 bp, Artificial Sequence
  Synthetic Construct
caggtacagctggtggagtctgggggaggattggtgcaggctgggggctctctgagactctcctgtgcagcctctggacgcaccttcaccatggggtggttccgtcaggctccagggaaggagcgtgagtttgtagcagctattagtttgagtcctactttagcatattatgcagagtccgtgaagggccgattcaccatcagccgagacaacgccaagaacacggtggttttgcaaatgaacagcctgaaacctgaggacacggccgtttactactgtgcagcacgtcggatcgacgcagctgactttgattcctgggggcaggggacccaggtcaccgtctcctca

SEQ ID NO: 170 - DNA, 360 bp, Artificial Sequence
  Synthetic Construct
caggtacagctggtggagtctgggggaggattggtgcaggctgggggctctctgagactctcctgtgcagcctctggaggcaccttaagtaaaaataccgtggcttggttccgccaggctccagggaaggagcgtgggtttgtagcgtctattacctgggatggtcgtacgacatactatgcagactccgtgaagggccgattcaccatctccagagacaacgccaagaacacagtgtatctgcaaatgaacagcctgaaacctgaggatacggccgtttatgtctgtgcagacttagggaaatggcctgcgggcccggcggactactggggccaggggacccaggtcaccgtctcctca

SEQ ID NO: 171 - DNA, 363 bp, Artificial Sequence
  Synthetic Construct
caggtgcagctggtggagtctgggggaggcttggtgcagcctggggggtctctgacactctcctgtgcagcctctggaagcatcgacagtatcaataccatggactggttccgtcaggctccagggaaggagcgtgagtttgtagcagctattagtttgagtcccactttagcatattatgcagagtccgtgaagggccgattcaccatcagccgagacaacgccaagaacacggtggttttgcaaatgaacagcctgaaacctgaggacacggccctttattactgtgcagcagaccggaaatcagtaatgtctattcggcccgactactggggccaggggacccaggtcaccgtctcctca

SEQ ID NO: 172 - DNA, 360 bp, Artificial Sequence
  Synthetic Construct
gatgtgcagctggtggagtctgggggaggattggtgcaggctgggggctctctgagactctcctgtgcagcctctggaggcaccttaagtaagaataccgtggcttgggtccgccaggctccagggaaggagcgtgggtttgtaacgtctattacctgtgatggtcgtacgacatactatgcgaactccgtgaagggccgattccccatctccagagacaacgccgagaacacagtgtatctgcaaatgaacagcctgaaacctgaggatacggccggttatgtctgtgcagacttagggaagtggcctgcgggttcggcggactactggggccaggggacccacgtcaccgtctcctcc

SEQ ID NO: 173 - DNA, 363 bp, Artificial Sequence
  Synthetic Construct
caggtaaagctggaggagtctgggggaggcttggtgcagcctggggggtctctgagactctcctgtacagcctcggaattcacattcagtgactactggatgcattgggtccgtcaggctccggggaaggggctcgagtgggtcgcatctatagatactagtggacagaccacatactatgcagactccctgaagggccgattcaccatctccagagacaacgccaagagcacgttgtatctgcaaatgaacagtctgaaatctgaagacacgggcgtgtatttctgtgcaaaacgatataggggtggtacctggtatggcatggccaactggggcaaagggacccaggtcaccgtctcctca

SEQ ID NO: 174 - DNA, 360 bp, Artificial Sequence
  Synthetic Construct
caggtgcagctggtggagtctgggggaggattggtgcaggctgggggctctctgagactctcctgtgcagcctctggacgcaccttaagtagtaataccatggcttggttccgccaggctccagggaaggagcgtgagtttgtagcgtctactacctggaatggtcgtagcacatactatgcagactccgtgaagggccgattcaccatctccagagacaacgccaagaacacgatgtatctgcaaatgaacagcctgaaacctgaggatacggccgtttatgtctgtgcagacttagggaaatggcctgcgggcccggcggactactggggccaggggacccaggtcaccgtctcctca

SEQ ID NO: 175 - DNA, 348 bp, Artificial Sequence
  Synthetic Construct
caggtgcagctggtggagtctgggggaggattggtgcaggctgggggctctctgagactctcctgtgcagcctctggacgcaccttcaccatggggtggttccgtcaggctccagggaagcagcgcgaattggtcgcagatattagtggtggtcgcacaaactatgcagattccgtgaagggacgattcaccatctccagagacaacgccaagaacacggtatatctgcaaatgaacagcctgaaacctgaggacacggccgtttattactgtgcagcagaccggaaatcagtaatgtctattcggcccgactactggggccaggggacccaggtcaccgtctcctca

SEQ ID NO: 176 - DNA, 312 bp, Artificial Sequence
  Synthetic Construct
caggtgcagctggtggagtctgggggaggcttggtgcaggctggggcctctctgagactctcctgtgcagcctctggacgcaccttcaccgtggcagctattagtttgagtcctactttagcatattatgcagagtccgtgaagggccgattcaccatcagccgagacaacgccaagaacacggtggttttgcaaatgaacagcctgaaacctgaggacacggccctttattactgtgcagcagaccggaaatcagtaatgtctattcggcccgactactggggccaggggacccaggtcaccgtctcctca

SEQ ID NO: 177 - DNA, 375 bp, Artificial Sequence
  Synthetic Construct
gatgtgcagctggtggagtctgggggaggattggagcaggctgggggctctctgagactctcctgtgcagcctctggaggcaccttaagtaaaaataccgtggcttggttccgccaggctccagggaaggagcgtgggtttgtagcgtctattacctgggatggtcgtacgacatactatgcagactccgtgaagggccgattcaccatctccagagacaacgccaagaacacagtgtatctgcaaatgaacagcctgaaacctgaggatacggccgtttattactgtgcgtcgacggcatcgtgccacctcttcggattggggtccggggcctttgtgtcctggggccgggggacccaggtcaccgtctcctca

SEQ ID NO: 178 - DNA, 348 bp, Artificial Sequence
  Synthetic Construct
gcggtgcagctggtggagtctgggggaggattggtgcaggctgggggctctctgagactctcctgtgcagcctctggacgcaccttcaccatggggtggttccatcaggctccagggaaggagcgtgagtttgtagcagctattagtttgagtcctactttagcatattatgcagagtccgtgaagggccgattcaccatcagccgagacaacgccaagaacacggtggttttgcaaatgaacagcctgaaacctgaggacacggccctttattactgtgcagcatccaaggatagatattcggaatatgagtactggggccaggggacccaggtcaccgtctcctca

SEQ ID NO: 179 - DNA, 342 bp, Artificial Sequence
  Synthetic Construct
caggtaaagctggaggagtctgggggaggattggtgcaggctgggggctctctgagactctcctgtgcagcctctggacgcaccttcaccatggggtggttccgtcaggctccagggaaggagcgtgagtttgtagcagctattagtttgagtcctactttagcatattatgcagagtccgtgaagggccgattcaccatcagccgagacaacgccaagaacacggtggttttgcaaatgaacagcctgaaacctgaggacacggccctttattactgtgcaaaaaaaaacggggggcctgtggactactggggcaaagggacccaggtcaccgtctcctca

SEQ ID NO: 180 - DNA, 357 bp, Artificial Sequence
  Synthetic Construct
gatgtgcagctggtggagtctgggggaggcttggtgcagcctggggggtctctgagactctcctgtgcagcctctggacggaccttcagtagcattgtcatgggctggttccgccaggctccagggaaggagcgtgagtttgtaggagcgattatgtggaatgatggtattacatacttgcaagactccgtgaagggccgatttaccatcttcagagacaacgccaagaacacggtgtatctgcaaatgaacagcctgaaacttgaggatacggccgtttattactgtgcagcatccaagggtagatactcggaatatgagtactggggccaggggacccaggtcaccgtctcctca

SEQ ID NO: 181 - DNA, 354 bp, Artificial Sequence
  Synthetic Construct
caggtaaagctggaggaatctgggggaagattggtgcaggctgggggctctctgaaactctcctgggcagcctctggacgcaccttcaccatggggtggttccgtcaggctccagggaaggaacgtgagtttgtaacagctattaatttgagtcctactttaacatattatgcagaatccgtgaagggccgattccccatcagccgaaacaacgcccagaacacggtggttttgcaaatgaacagcctgaaacctgaggacacggccctttattactgtgcagcagaacggaaatcagtaatggctattccgcccgactactggggccaggggacccaggtcaccgtctcctca

SEQ ID NO: 182 - DNA, 354 bp, Artificial Sequence
  Synthetic Construct
gaggtgcagctggtggagtctgggggaggattggtgcaggctgggggctctctgagactctcctgtgcagcctctggacgcaccttcaccatgggggggttccgtcgggttcctcgggatgagcgggagtttgtagcatctattactttgattcctacttttccttattatgcatattccgtgaagggccgattcgccctcttccgagacaaccccaacaacaccgtgattttgctgatgatcagcctgaaacctgaggacccggacctttattactgtgcttcataccggaaatacctaatgtctattctgcccgactactggggccaggggacccagggcaccgtctcctcc

SEQ ID NO: 183 - DNA, 372 bp, Artificial Sequence
  Synthetic Construct
caggtaaagctggaggagtctgggggaggattggtgcaggctgggggctctctgagactctcctgtgcagcctctggacgcaccttcaccatggggtggttccgtcaggctccagggaaggagcgtgagtttgtagcagctattagtttgagtcctactttagcatattatgcagagtccgtgaagggccgattcaccatcagccgagacaacgccaagaacacggtggatctgcaaatgaacagcctgaaacctgaggacacggccgtctatttctgtgcagcaaatcggaactcccaacgggtaattgcggcactgtcctggattggcatgaactactggggcgaatggacccaggtcaccgtctcctcc

SEQ ID NO: 184 - DNA, 348 bp, Artificial Sequence
  Synthetic Construct
caggtgcagctggtggagtctgggggaggattggtgcaggctgggggctctctgagactctcctgtgcagcctctggacgcaccttcaccatggggtggttccgtcaggctccagggaaggagcgtgagtttgtagcagctattagtttgagtcctactttagcatattatgcagagtccgtgaagggccgattcaccatctccagagacaacgccaagaagacgctgtatctgcgaatgaatagcctgaaacctgaggacacggccgtttactactgtgcagcacgtcggatcgacgcagctgactttgattcctgggggcaggggacccaggtcaccgtctcctca

SEQ ID NO: 185 - DNA, 348 bp, Artificial Sequence
  Synthetic Construct
caggtaaagctggaggagtctgggggaggattggtgcaggctgggggctctctgagactctcctgtgcagcctctggacgcaccttcaccatggggtggttccgtcgggctccagggaaggagcgtgagtctgttgcagttattggctggagagatattaacgcaagctatgcagactccgtgaagggccgattcgccatctccagagacaacgccaagaagacgctgtatctgcagatgaatagcctgaaacctgaggacacggccgtttactactgtgcagcacgtcggatcgacgcaactgactttgattcctgggggcaggggacccaggtcaccgtctcctca

SEQ ID NO: 186 - DNA, 357 bp, Artificial Sequence
  Synthetic Construct
caggtaaagctggaggagtctgggggaggattggtgcagactgggggctctctgagactctcctgtgcagcctctgaacacaccttcagtaaccatgtcatgggctggttccgccaggctccagggaaggagcgtgagtctgttgcagttattggctggagagatattagcacaagctatgcagactccgtgaagggccgattcaccatctccagagacaacgccaagaagacgctgtatctgcaaatgaatagcctgaaacctgaggacacggccgtttactactgtgcagcacgtcggatcgacgcagctgactttgattcccgggggcaggggacccaggtcaccgtctcctca

SEQ ID NO: 187 - DNA, 369 bp, Artificial Sequence
  Synthetic Construct
gccgtgcagctggtggattctgggggaggattggtgcaggctgggggctctctgagaatttcctgtgcagtctctggacgcacctccagtaactatatattggcctggttccgtcaggctccaggaaaagagcgtgactttgtagcacatattagccggagtggtggtaagtccggctatggagactccgtgaagggccgattcaccatctccagagacaacgccgagaacacggtcagggtgtatctgcaaatgaacagtctgaaacctggggacacggccgtctattactgtaatcgccccctctggtacggaagtcccacgttgattgactactggggccaggggacccaggtcaccgtctcctca

SEQ ID NO: 188 - DNA, 354 bp, Artificial Sequence
  Synthetic Construct
gcggtgcagctggtggagtctgggggaggcttggtgcagcctggggggtctctgagactctcctgtgcagcctctggacgcaccttcaccatggggtggttccgtcaggctccagggaaggagcgtgagtttgtagcagctattagtttgagtcctactttagcatattatgcagagtccgtgaagggccgattcaccatcagccgagacaacgccaagaacacggtggttttgcaaatgaacagcctgaaacctgaggacacggccctttattactgtgcagcagaccggaaatcagtaatgtctattcggcccgactactggggccaggggacccaggtcaccgtctcctca

SEQ ID NO: 189 - DNA, 354 bp, Artificial Sequence
  Synthetic Construct
gcggtgcagctggtggagtctgggggaggattggtgcaggctgggggctctctgagactctcctgtgcagcctctggacgcaccttcaccatggggtggttccgtcaggctccagggaaggagcgtgagtttgtagcagctattagtttgagtcctactttagcatattatgcagagtccgtgaagggccgattcaccatcagccgagacaacgccaagaacacggtggttttgcaaatgaacagcctgaaacctgaggacacggccctttattactgtgcagcagaccggaaatcagtaatgtctattcggcccgactactggggccaggggacccaggtcaccgtctcctca

SEQ ID NO: 190 - DNA, 363 bp, Artificial Sequence
  Synthetic Construct
gatgtgcagctggtggagtctgggggaggatcggtgcagactgggggctctctgagactctcctgtacagcctctggacgcaccctcaataactttgtcatgggctggttccgtcaggctccagggaaggagcgtgagtttgtagcagctattagtttgagtcctactttagcatattatgtagagtccgtgaagggccgattcaccatcagccgagacaacgccaagaacacggtggttttgcaaatgaacagcctgaaacctgaggacacggccctttattactgtgcagcagaccggaaatcagtaatgtctattcggcccgactactggggccaggggacccaggtcaccgtctcctca

SEQ ID NO: 191 - protein, 21 aa, Artificial Sequence
  Synthetic Construct
MALPVTALLLPLALLLHAARP

SEQ ID NO: 192 - protein, 45 aa, Artificial Sequence
  Synthetic Construct
TTTPAPRPPTPAPTIASQPLSLRPEACRPAAGGAVHTRGLDFACD

SEQ ID NO: 193 - protein, 24 aa, Artificial Sequence
  Synthetic Construct
IYIWAPLAGTCGVLLLSLVITLYC

SEQ ID NO: 194 - protein, 27 aa, Artificial Sequence
  Synthetic Construct
FWVLVVVGGVLACYSLLVTVAFIIFWV

SEQ ID NO: 195 - protein, 41 aa, Artificial Sequence
  Synthetic Construct
RSKRSRLLHSDYMNMTPRRPGPTRKHYQPYAPPRDFAAYRS

SEQ ID NO: 196 - protein, 42 aa, Artificial Sequence
  Synthetic Construct
KRGRKKLLYIFKQPFMRPVQTTQEEDGCSCRFPEEEEGGCEL

SEQ ID NO: 197 - protein, 113 aa, Artificial Sequence
  Synthetic Construct
RVKFSRSADAPAYQQGQNQLYNELNLGRREEYDVLDKRRGRDPEMGGKPQRRKNPQEGLYNELQKDKMAEAYSEIGMKGERRRGKGHDGLYQGLSTATKDTYDALHMQALPPR

SEQ ID NO: 198 - protein, 113 aa, Artificial Sequence
  Synthetic Construct
RVKFSRSADAPAYKQGQNQLYNELNLGRREEYDVLDKRRGRDPEMGGKPQRRKNPQEGLYNELQKDKMAEAYSEIGMKGERRRGKGHDGLYQGLSTATKDTYDALHMQALPPR

SEQ ID NO: 199 - DNA, 63 bp, Artificial Sequence
  Synthetic Construct
atggccttaccagtgaccgccttgctcctgccgctggccttgctgctccacgccgccaggccg

SEQ ID NO: 200 - DNA, 63 bp, Artificial Sequence
  Synthetic Construct
atggctctgcccgtcactgctctgctgctgcccctggctctgctgctgcacgccgcaagaccc

SEQ ID NO: 201 - DNA, 135 bp, Artificial Sequence
  Synthetic Construct
accacgacgccagcgccgcgaccaccaacaccggcgcccaccatcgcgtcgcagcccctgtccctgcgcccagaggcgtgccggccagcggcggggggcgcagtgcacacgagggggctggacttcgcctgtgat

SEQ ID NO: 202 - DNA, 72 bp, Artificial Sequence
  Synthetic Construct
atctacatctgggcgcccttggccgggacttgtggggtccttctcctgtcactggttatcaccctttactgc

SEQ ID NO: 203 - DNA, 81 bp, Artificial Sequence
  Synthetic Construct
ttttgggtgctggtggtggttggtggagtcctggcttgctatagcttgctagtaacagtggcctttattattttctgggtg

SEQ ID NO: 204 - DNA, 123 bp, Artificial Sequence
  Synthetic Construct
aggagtaagaggagcaggctcctgcacagtgactacatgaacatgactccccgccgccccgggcccacccgcaagcattaccagccctatgccccaccacgcgacttcgcagcctatcgctcc

SEQ ID NO: 205 - DNA, 126 bp, Artificial Sequence
  Synthetic Construct
aaacggggcagaaagaaactcctgtatatattcaaacaaccatttatgagaccagtacaaactactcaagaggaagatggctgtagctgccgatttccagaagaagaagaaggaggatgtgaactg

SEQ ID NO: 206 - DNA, 336 bp, Artificial Sequence
  Synthetic Construct
agagtgaagttcagcaggagcgcagacgcccccgcgtaccagcagggccagaaccagctctataacgagctcaatctaggacgaagagaggagtacgatgttttggacaagagacgtggccgggaccctgagatggggggaaagccgagaaggaagaaccctcaggaaggcctgtacaatgaactgcagaaagataagatggcggaggcctacagtgagattgggatgaaaggcgagcgccggaggggcaaggggcacgatggcctttaccagggtctcagtacagccaccaaggacacctacgacgcccttcacatgcaggccctgccccctcgc

SEQ ID NO: 207 - DNA, 336 bp, Artificial Sequence
  Synthetic Construct
agagtgaagttcagcaggagcgcagacgcccccgcgtacaagcagggccagaaccagctctataacgagctcaatctaggacgaagagaggagtacgatgttttggacaagagacgtggccgggaccctgagatggggggaaagccgagaaggaagaaccctcaggaaggcctgtacaatgaactgcagaaagataagatggcggaggcctacagtgagattgggatgaaaggcgagcgccggaggggcaaggggcacgatggcctttaccagggtctcagtacagccaccaaggacacctacgacgcccttcacatgcaggccctgccccctcgc

SEQ ID NO: 208 - protein, 5 aa, Artificial Sequence
  Synthetic Construct
GGGGS

SEQ ID NO: 209 - protein, 10 aa, Artificial Sequence
  Synthetic Construct
GGGGSGGGGS

SEQ ID NO: 210 - protein, 16 aa, Artificial Sequence
  Synthetic Construct
GGGSGGGSGGGSGGGS

SEQ ID NO: 211 - protein, 24 aa, Artificial Sequence
  Synthetic Construct
GGGGSGGGGSGGGGGGSGSGGGGS

SEQ ID NO: 212 - protein, 34 aa, Artificial Sequence
  Synthetic Construct
GGGGSGGGGSGGGGGGSGSGGGGSGGGGSGGGGS

SEQ ID NO: 213 - protein, 15 aa, Artificial Sequence
  Synthetic Construct
GGGGSGGGGSGGGGS

SEQ ID NO: 214 - protein, 20 aa, Artificial Sequence
  Synthetic Construct
GGGGSGGGGSGGGGSGGGGS

SEQ ID NO: 215 - protein, 25 aa, Artificial Sequence
  Synthetic Construct
GGGGSGGGGSGGGGSGGGGSGGGGS

SEQ ID NO: 216 - protein, 420 aa, Artificial Sequence
  Synthetic Construct
MALPVTALLLPLALLLHAARPVNRTRRMHQVQLVESGGGLVQPGGSLRLSCEASGFTLDYYAIGWFRQAPGKEREGVICISRSDGSTYYADSVKGRFTISRDNAKKTVYLQMISLKPEDTAAYYCAAGADCSGYLRDYEFRGQGTQVTVSSTSTTTPAPRPPTPAPTIASQPLSLRPEACRPAAGGAVHTRGLDFACDFWVLVVVGGVLACYSLLVTVAFIIFWVRSKRSRLLHSDYMNMTPRRPGPTRKHYQPYAPPRDFAAYRSKRGRKKLLYIFKQPFMRPVQTTQEEDGCSCRFPEEEEGGCELRVKFSRSADAPAYKQGQNQLYNELNLGRREEYDVLDKRRGRDPEMGGKPRRKNPQEGLYNELQKDKMAEAYSEIGMKGERRRGKGHDGLYQGLSTATKDTYDALHMQALPPR

SEQ ID NO: 217 - protein, 426 aa, Artificial Sequence
  Synthetic Construct
MALPVTALLLPLALLLHAARPVNRTRRMHQVKLEESGGRLVQPRGSLRLSCAGSGRTFSTYGMAWFRQAPGKEREFVASKASMNYSGRTYYADSVKGRFTIARDNAKNMVFLQMNNLKPEDTAVYYCAAGTGCSTYGCFDAQIIDYWGKGTLVTVSSTSTTTPAPRPPTPAPTIASQPLSLRPEACRPAAGGAVHTRGLDFACDFWVLVVVGGVLACYSLLVTVAFIIFWVRSKRSRLLHSDYMNMTPRRPGPTRKHYQPYAPPRDFAAYRSKRGRKKLLYIFKQPFMRPVQTTQEEDGCSCRFPEEEEGGCELRVKFSRSADAPAYKQGQNQLYNELNLGRREEYDVLDKRRGRDPEMGGKPRRKNPQEGLYNELQKDKMAEAYSEIGMKGERRRGKGHDGLYQGLSTATKDTYDALHMQALPPR

SEQ ID NO: 218 - protein, 416 aa, Artificial Sequence
  Synthetic Construct
MALPVTALLLPLALLLHAARPVNRTRRMHEVQLVESGGGLVQAGGSLRLSCAASGRTFTMGWFRQAPGKEREFVAAISLSPTLAYYAESVKGRFTISRDNAKNTVVLQMNSLKPEDTALYYCAADRKSVMSIRPDYWGQGTQVTVSSTSTTTPAPRPPTPAPTIASQPLSLRPEACRPAAGGAVHTRGLDFACDFWVLVVVGGVLACYSLLVTVAFIIFWVRSKRSRLLHSDYMNMTPRRPGPTRKHYQPYAPPRDFAAYRSKRGRKKLLYIFKQPFMRPVQTTQEEDGCSCRFPEEEEGGCELRVKFSRSADAPAYKQGQNQLYNELNLGRREEYDVLDKRRGRDPEMGGKPRRKNPQEGLYNELQKDKMAEAYSEIGMKGERRRGKGHDGLYQGLSTATKDTYDALHMQALPPR

SEQ ID NO: 219 - protein, 418 aa, Artificial Sequence
  Synthetic Construct
MALPVTALLLPLALLLHAARPVNRTRRMHAVQLVDSGGGLVQPGGSLRLSCVASGGIFVINAMGWYRQAPGKQRELVASIRGLGRTNYDDSVKGRFTISRDNANNTVYLQMNSLEPEDTAVYYCTVYVTLLGGVNRDYWGQGTQVTVSSTSTTTPAPRPPTPAPTIASQPLSLRPEACRPAAGGAVHTRGLDFACDFWVLVVVGGVLACYSLLVTVAFIIFWVRSKRSRLLHSDYMNMTPRRPGPTRKHYQPYAPPRDFAAYRSKRGRKKLLYIFKQPFMRPVQTTQEEDGCSCRFPEEEEGGCELRVKFSRSADAPAYKQGQNQLYNELNLGRREEYDVLDKRRGRDPEMGGKPRRKNPQEGLYNELQKDKMAEAYSEIGMKGERRRGKGHDGLYQGLSTATKDTYDALHMQALPPR

SEQ ID NO: 220 - protein, 417 aa, Artificial Sequence
  Synthetic Construct
MALPVTALLLPLALLLHAARPVNRTRRMHEVQLVESGGGLVQAGGSLRLSCAASGRTFSSIVMGWFRQAPGKEREFVGAIMWNDGITYLQDSVKGRFTIFRDNAKNTVYLQMNSLKLEDTAVYYCAASKGRYSEYEYWGQGTQVTVSSTSTTTPAPRPPTPAPTIASQPLSLRPEACRPAAGGAVHTRGLDFACDFWVLVVVGGVLACYSLLVTVAFIIFWVRSKRSRLLHSDYMNMTPRRPGPTRKHYQPYAPPRDFAAYRSKRGRKKLLYIFKQPFMRPVQTTQEEDGCSCRFPEEEEGGCELRVKFSRSADAPAYKQGQNQLYNELNLGRREEYDVLDKRRGRDPEMGGKPRRKNPQEGLYNELQKDKMAEAYSEIGMKGERRRGKGHDGLYQGLSTATKDTYDALHMQALPPR

SEQ ID NO: 221 - protein, 426 aa, Artificial Sequence
  Synthetic Construct
MALPVTALLLPLALLLHAARPVNRTRRMHEVQLVESGGGVVQAGGSLTVSCTASGFTFDRAVIVWFRQAPGKGREGVSFIKPSDGTIYYIDSLKGRFTISSDIAKNTVYLQMKSLESEDSAVYYCAASPEDWYTDWIDWSIYRWQHWGQGTQVTVSSTSTTTPAPRPPTPAPTIASQPLSLRPEACRPAAGGAVHTRGLDFACDFWVLVVVGGVLACYSLLVTVAFIIFWVRSKRSRLLHSDYMNMTPRRPGPTRKHYQPYAPPRDFAAYRSKRGRKKLLYIFKQPFMRPVQTTQEEDGCSCRFPEEEEGGCELRVKFSRSADAPAYKQGQNQLYNELNLGRREEYDVLDKRRGRDPEMGGKPRRKNPQEGLYNELQKDKMAEAYSEIGMKGERRRGKGHDGLYQGLSTATKDTYDALHMQALPPR

SEQ ID NO: 222 - protein, 417 aa, Artificial Sequence
  Synthetic Construct
MALPVTALLLPLALLLHAARPVNRTRRMHEVQLVESGGGMVQAGDSLRLSCVQSTYTVNSDVMGWFRQAPGKEREFVGAIMWNDGITYLQDSVKGRFTIFRDNAKNTVYLQMNSLKLEDTAVYYCAASKGRYSEYEYWGQGTQVTVSSTSTTTPAPRPPTPAPTIASQPLSLRPEACRPAAGGAVHTRGLDFACDFWVLVVVGGVLACYSLLVTVAFIIFWVRSKRSRLLHSDYMNMTPRRPGPTRKHYQPYAPPRDFAAYRSKRGRKKLLYIFKQPFMRPVQTTQEEDGCSCRFPEEEEGGCELRVKFSRSADAPAYKQGQNQLYNELNLGRREEYDVLDKRRGRDPEMGGKPRRKNPQEGLYNELQKDKMAEAYSEIGMKGERRRGKGHDGLYQGLSTATKDTYDALHMQALPPR

SEQ ID NO: 223 - protein, 418 aa, Artificial Sequence
  Synthetic Construct
MALPVTALLLPLALLLHAARPVNRTRRMHAVQLVESGGGLVQAGDSLRLSCTASGATLTNDHMAWFRQAPGKGREFVAAIDWSGRTTNYADPVEGRFTISRNNAKNTVYLEMNSLKLEDTAVYYCAVLRAWISYDNDYWGQGTQVTVSSTSTTTPAPRPPTPAPTIASQPLSLRPEACRPAAGGAVHTRGLDFACDFWVLVVVGGVLACYSLLVTVAFIIFWVRSKRSRLLHSDYMNMTPRRPGPTRKHYQPYAPPRDFAAYRSKRGRKKLLYIFKQPFMRPVQTTQEEDGCSCRFPEEEEGGCELRVKFSRSADAPAYKQGQNQLYNELNLGRREEYDVLDKRRGRDPEMGGKPRRKNPQEGLYNELQKDKMAEAYSEIGMKGERRRGKGHDGLYQGLSTATKDTYDALHMQALPPR

SEQ ID NO: 224 - protein, 418 aa, Artificial Sequence
  Synthetic Construct
MALPVTALLLPLALLLHAARPVNRTRRMHQVQLVESGGGLVQAGGSLRLSCAASGGTLSKNTVAWFRQAPGKERGFVASITWDGRTTYYADSVKGRFTISRDNAKNTVYLQMNSLKPEDTAVYVCADLGKWPAGPADYWGQGTQVTVSSTSTTTPAPRPPTPAPTIASQPLSLRPEACRPAAGGAVHTRGLDFACDFWVLVVVGGVLACYSLLVTVAFIIFWVRSKRSRLLHSDYMNMTPRRPGPTRKHYQPYAPPRDFAAYRSKRGRKKLLYIFKQPFMRPVQTTQEEDGCSCRFPEEEEGGCELRVKFSRSADAPAYKQGQNQLYNELNLGRREEYDVLDKRRGRDPEMGGKPRRKNPQEGLYNELQKDKMAEAYSEIGMKGERRRGKGHDGLYQGLSTATKDTYDALHMQALPPR

SEQ ID NO: 225 - protein, 417 aa, Artificial Sequence
  Synthetic Construct
MALPVTALLLPLALLLHAARPVNRTRRMHQVKLEESGGGLVQAGRSLRLSCAASEHTFSSHVMGWFRQAPGKERESVAVIGWRDISTSYADSVKGRFTISRDNAKKTLYLQMNSLKPEDTAVYYCAARRIDAADFDSWGQGTQVTVSSTSTTTPAPRPPTPAPTIASQPLSLRPEACRPAAGGAVHTRGLDFACDFWVLVVVGGVLACYSLLVTVAFIIFWVRSKRSRLLHSDYMNMTPRRPGPTRKHYQPYAPPRDFAAYRSKRGRKKLLYIFKQPFMRPVQTTQEEDGCSCRFPEEEEGGCELRVKFSRSADAPAYKQGQNQLYNELNLGRREEYDVLDKRRGRDPEMGGKPRRKNPQEGLYNELQKDKMAEAYSEIGMKGERRRGKGHDGLYQGLSTATKDTYDALHMQALPPR

SEQ ID NO: 226 - protein, 417 aa, Artificial Sequence
  Synthetic Construct
MALPVTALLLPLALLLHAARPVNRTRRMHAVQLVESGGGLVQAGDSLRLTCTASGRAFSTYFMAWFRQAPGKEREFVAGIAWSGGSTAYADSVKGRFTISRDNAKNTVYLQMNSLKSEDTAVYYCASRGIEVEEFGAWGQGTQVTVSSTSTTTPAPRPPTPAPTIASQPLSLRPEACRPAAGGAVHTRGLDFACDFWVLVVVGGVLACYSLLVTVAFIIFWVRSKRSRLLHSDYMNMTPRRPGPTRKHYQPYAPPRDFAAYRSKRGRKKLLYIFKQPFMRPVQTTQEEDGCSCRFPEEEEGGCELRVKFSRSADAPAYKQGQNQLYNELNLGRREEYDVLDKRRGRDPEMGGKPRRKNPQEGLYNELQKDKMAEAYSEIGMKGERRRGKGHDGLYQGLSTATKDTYDALHMQALPPR

SEQ ID NO: 227 - protein, 376 aa, Artificial Sequence
  Synthetic Construct
MALPVTALLLPLALLLHAARPVNRTRRMHQVQLVESGGGLVQPGGSLRLSCEASGFTLDYYAIGWFRQAPGKEREGVICISRSDGSTYYADSVKGRFTISRDNAKKTVYLQMISLKPEDTAAYYCAAGADCSGYLRDYEFRGQGTQVTVSSTSTTTPAPRPPTPAPTIASQPLSLRPEACRPAAGGAVHTRGLDFACDIYIWAPLAGTCGVLLLSLVITLYCKRGRKKLLYIFKQPFMRPVQTTQEEDGCSCRFPEEEEGGCELRVKFSRSADAPAYQQGQNQLYNELNLGRREEYDVLDKRRGRDPEMGGKPRRKNPQEGLYNELQKDKMAEAYSEIGMKGERRRGKGHDGLYQGLSTATKDTYDALHMQALPPR

SEQ ID NO: 228 - protein, 373 aa, Artificial Sequence
  Synthetic Construct
MALPVTALLLPLALLLHAARPVNRTRRMHQVKLEESGGGLVQAGRSLRLSCAASEHTFSSHVMGWFRQAPGKERESVAVIGWRDISTSYADSVKGRFTISRDNAKKTLYLQMNSLKPEDTAVYYCAARRIDAADFDSWGQGTQVTVSSTSTTTPAPRPPTPAPTIASQPLSLRPEACRPAAGGAVHTRGLDFACDIYIWAPLAGTCGVLLLSLVITLYCKRGRKKLLYIFKQPFMRPVQTTQEEDGCSCRFPEEEEGGCELRVKFSRSADAPAYQQGQNQLYNELNLGRREEYDVLDKRRGRDPEMGGKPRRKNPQEGLYNELQKDKMAEAYSEIGMKGERRRGKGHDGLYQGLSTATKDTYDALHMQALPPR

SEQ ID NO: 229 - protein, 372 aa, Artificial Sequence
  Synthetic Construct
MALPVTALLLPLALLLHAARPVNRTRRMHEVQLVESGGGLVQAGGSLRLSCAASGRTFTMGWFRQAPGKEREFVAAISLSPTLAYYAESVKGRFTISRDNAKNTVVLQMNSLKPEDTALYYCAADRKSVMSIRPDYWGQGTQVTVSSTSTTTPAPRPPTPAPTIASQPLSLRPEACRPAAGGAVHTRGLDFACDIYIWAPLAGTCGVLLLSLVITLYCKRGRKKLLYIFKQPFMRPVQTTQEEDGCSCRFPEEEEGGCELRVKFSRSADAPAYQQGQNQLYNELNLGRREEYDVLDKRRGRDPEMGGKPRRKNPQEGLYNELQKDKMAEAYSEIGMKGERRRGKGHDGLYQGLSTATKDTYDALHMQALPPR

SEQ ID NO: 230 - protein, 372 aa, Artificial Sequence
  Synthetic Construct
MALPVTALLLPLALLLHAARPEVQLVESGGGLVPPGGSLRLSCTASGSTVSINVMAWYRQVSGKQRELVAAVTRDGRKSCGDSVKGRFTISRDGAKNAVYLQMNSLKPEDTAVYLCGADGWGATTLDYTYGMDYWGKGTQVTVSSAATSTTTPAPRPPTPAPTIASQPLSLRPEACRPAAGGAVHTRGLDFACDIYIWAPLAGTCGVLLLSLVITLYCKRGRKKLLYIFKQPFMRPVQTTQEEDGCSCRFPEEEEGGCELRVKFSRSADAPAYQQGQNQLYNELNLGRREEYDVLDKRRGRDPEMGGKPRRKNPQEGLYNELQKDKMAEAYSEIGMKGERRRGKGHDGLYQGLSTATKDTYDALHMQALPPR

SEQ ID NO: 231 - protein, 364 aa, Artificial Sequence
  Synthetic Construct
MALPVTALLLPLALLLHAARPAVQLVESGGGLVQAGGSLRLSCAASGRTFTMGWFRQAPGKERGFVASITWDGRSAYYAESVKGRFTISRDNAKNTVVLQMNSLKPEDTALYYCAADRKSVMSIRPDYWGQGTQVTVSSTSTTTPAPRPPTPAPTIASQPLSLRPEACRPAAGGAVHTRGLDFACDIYIWAPLAGTCGVLLLSLVITLYCKRGRKKLLYIFKQPFMRPVQTTQEEDGCSCRFPEEEEGGCELRVKFSRSADAPAYQQGQNQLYNELNLGRREEYDVLDKRRGRDPEMGGKPRRKNPQEGLYNELQKDKMAEAYSEIGMKGERRRGKGHDGLYQGLSTATKDTYDALHMQALPPR

SEQ ID NO: 232 - protein, 368 aa, Artificial Sequence
  Synthetic Construct
MALPVTALLLPLALLLHAARPQVQLVESGGGLVQPGGSLRLACEAPGSGNSINAMGWYRQTPGKRRELVATITRGGSTNYGPSVKGRFTITRDNVKNTVHLQMNSLKPDDTAVYYCNAERLDGSGYGYEYDYWGQGTQVTVSSTSTTTPAPRPPTPAPTIASQPLSLRPEACRPAAGGAVHTRGLDFACDIYIWAPLAGTCGVLLLSLVITLYCKRGRKKLLYIFKQPFMRPVQTTQEEDGCSCRFPEEEEGGCELRVKFSRSADAPAYQQGQNQLYNELNLGRREEYDVLDKRRGRDPEMGGKPRRKNPQEGLYNELQKDKMAEAYSEIGMKGERRRGKGHDGLYQGLSTATKDTYDALHMQALPPR

SEQ ID NO: 233 - protein, 367 aa, Artificial Sequence
  Synthetic Construct
MALPVTALLLPLALLLHAARPQVKLEESGGGLVQAGGSLRLSCAASGGTLSKNTVAWVRQAPGKERGFVTSITCDGRTTYYANSVNGRFPINRNNAENLVVLQMNSLKPDDTALYYCAAYRKSIMSIQPDYWGQGTQVTVSSTSTTTPAPRPPTPAPTIASQPLSLRPEACRPAAGGAVHTRGLDFACDIYIWAPLAGTCGVLLLSLVITLYCKRGRKKLLYIFKQPFMRPVQTTQEEDGCSCRFPEEEEGGCELRVKFSRSADAPAYQQGQNQLYNELNLGRREEYDVLDKRRGRDPEMGGKPRRKNPQEGLYNELQKDKMAEAYSEIGMKGERRRGKGHDGLYQGLSTATKDTYDALHMQALPPR

SEQ ID NO: 234 - protein, 367 aa, Artificial Sequence
  Synthetic Construct
MALPVTALLLPLALLLHAARPDVQLVESGGGLVQAGGSLRLSCAASGRTFSSIVMGWFRQAPGKEREFVGAIMWNDGLTYLQGSVKGRFTISRDNAKNTVVLQMNSLKPEDTALYYCAADRKSVMSIRPDYWGQGTQVTVSSTSTTTPAPRPPTPAPTIASQPLSLRPEACRPAAGGAVHTRGLDFACDIYIWAPLAGTCGVLLLSLVITLYCKRGRKKLLYIFKQPFMRPVQTTQEEDGCSCRFPEEEEGGCELRVKFSRSADAPAYQQGQNQLYNELNLGRREEYDVLDKRRGRDPEMGGKPRRKNPQEGLYNELQKDKMAEAYSEIGMKGERRRGKGHDGLYQGLSTATKDTYDALHMQALPPR

SEQ ID NO: 235 - protein, 362 aa, Artificial Sequence
  Synthetic Construct
MALPVTALLLPLALLLHAARPQVQLVESGGGLVQAGGSLRLSCAASGRTFTMGWFRQAPGKEREFVAAISLSPTLAYYAESVKGRFTISRDNAKNTVVLQMNSLKPEDTAVYYCAARRIDAADFDSWGQGTQVTVSSTSTTTPAPRPPTPAPTIASQPLSLRPEACRPAAGGAVHTRGLDFACDIYIWAPLAGTCGVLLLSLVITLYCKRGRKKLLYIFKQPFMRPVQTTQEEDGCSCRFPEEEEGGCELRVKFSRSADAPAYQQGQNQLYNELNLGRREEYDVLDKRRGRDPEMGGKPRRKNPQEGLYNELQKDKMAEAYSEIGMKGERRRGKGHDGLYQGLSTATKDTYDALHMQALPPR

SEQ ID NO: 236 - protein, 366 aa, Artificial Sequence
  Synthetic Construct
MALPVTALLLPLALLLHAARPQVQLVESGGGLVQAGGSLRLSCAASGGTLSKNTVAWFRQAPGKERGFVASITWDGRTTYYADSVKGRFTISRDNAKNTVYLQMNSLKPEDTAVYVCADLGKWPAGPADYWGQGTQVTVSSTSTTTPAPRPPTPAPTIASQPLSLRPEACRPAAGGAVHTRGLDFACDIYIWAPLAGTCGVLLLSLVITLYCKRGRKKLLYIFKQPFMRPVQTTQEEDGCSCRFPEEEEGGCELRVKFSRSADAPAYQQGQNQLYNELNLGRREEYDVLDKRRGRDPEMGGKPRRKNPQEGLYNELQKDKMAEAYSEIGMKGERRRGKGHDGLYQGLSTATKDTYDALHMQALPPR

SEQ ID NO: 237 - protein, 367 aa, Artificial Sequence
  Synthetic Construct
MALPVTALLLPLALLLHAARPQVQLVESGGGLVQPGGSLTLSCAASGSIDSINTMDWFRQAPGKEREFVAAISLSPTLAYYAESVKGRFTISRDNAKNTVVLQMNSLKPEDTALYYCAADRKSVMSIRPDYWGQGTQVTVSSTSTTTPAPRPPTPAPTIASQPLSLRPEACRPAAGGAVHTRGLDFACDIYIWAPLAGTCGVLLLSLVITLYCKRGRKKLLYIFKQPFMRPVQTTQEEDGCSCRFPEEEEGGCELRVKFSRSADAPAYQQGQNQLYNELNLGRREEYDVLDKRRGRDPEMGGKPRRKNPQEGLYNELQKDKMAEAYSEIGMKGERRRGKGHDGLYQGLSTATKDTYDALHMQALPPR

SEQ ID NO: 238 - protein, 366 aa, Artificial Sequence
  Synthetic Construct
MALPVTALLLPLALLLHAARPDVQLVESGGGLVQAGGSLRLSCAASGGTLSKNTVAWVRQAPGKERGFVTSITCDGRTTYYANSVKGRFPISRDNAENTVYLQMNSLKPEDTAGYVCADLGKWPAGSADYWGQGTHVTVSSTSTTTPAPRPPTPAPTIASQPLSLRPEACRPAAGGAVHTRGLDFACDIYIWAPLAGTCGVLLLSLVITLYCKRGRKKLLYIFKQPFMRPVQTTQEEDGCSCRFPEEEEGGCELRVKFSRSADAPAYQQGQNQLYNELNLGRREEYDVLDKRRGRDPEMGGKPRRKNPQEGLYNELQKDKMAEAYSEIGMKGERRRGKGHDGLYQGLSTATKDTYDALHMQALPPR

SEQ ID NO: 239 - protein, 367 aa, Artificial Sequence
  Synthetic Construct
MALPVTALLLPLALLLHAARPQVKLEESGGGLVQPGGSLRLSCTASEFTFSDYWMHWVRQAPGKGLEWVASIDTSGQTTYYADSLKGRFTISRDNAKSTLYLQMNSLKSEDTGVYFCAKRYRGGTWYGMANWGKGTQVTVSSTSTTTPAPRPPTPAPTIASQPLSLRPEACRPAAGGAVHTRGLDFACDIYIWAPLAGTCGVLLLSLVITLYCKRGRKKLLYIFKQPFMRPVQTTQEEDGCSCRFPEEEEGGCELRVKFSRSADAPAYQQGQNQLYNELNLGRREEYDVLDKRRGRDPEMGGKPRRKNPQEGLYNELQKDKMAEAYSEIGMKGERRRGKGHDGLYQGLSTATKDTYDALHMQALPPR

SEQ ID NO: 240 - protein, 366 aa, Artificial Sequence
  Synthetic Construct
MALPVTALLLPLALLLHAARPQVQLVESGGGLVQAGGSLRLSCAASGRTLSSNTMAWFRQAPGKEREFVASTTWNGRSTYYADSVKGRFTISRDNAKNTMYLQMNSLKPEDTAVYVCADLGKWPAGPADYWGQGTQVTVSSTSTTTPAPRPPTPAPTIASQPLSLRPEACRPAAGGAVHTRGLDFACDIYIWAPLAGTCGVLLLSLVITLYCKRGRKKLLYIFKQPFMRPVQTTQEEDGCSCRFPEEEEGGCELRVKFSRSADAPAYQQGQNQLYNELNLGRREEYDVLDKRRGRDPEMGGKPRRKNPQEGLYNELQKDKMAEAYSEIGMKGERRRGKGHDGLYQGLSTATKDTYDALHMQALPPR

SEQ ID NO: 241 - protein, 362 aa, Artificial Sequence
  Synthetic Construct
MALPVTALLLPLALLLHAARPQVQLVESGGGLVQAGGSLRLSCAASGRTFTMGWFRQAPGKQRELVADISGGRTNYADSVKGRFTISRDNAKNTVYLQMNSLKPEDTAVYYCAADRKSVMSIRPDYWGQGTQVTVSSTSTTTPAPRPPTPAPTIASQPLSLRPEACRPAAGGAVHTRGLDFACDIYIWAPLAGTCGVLLLSLVITLYCKRGRKKLLYIFKQPFMRPVQTTQEEDGCSCRFPEEEEGGCELRVKFSRSADAPAYQQGQNQLYNELNLGRREEYDVLDKRRGRDPEMGGKPRRKNPQEGLYNELQKDKMAEAYSEIGMKGERRRGKGHDGLYQGLSTATKDTYDALHMQALPPR

SEQ ID NO: 242 - protein, 350 aa, Artificial Sequence
  Synthetic Construct
MALPVTALLLPLALLLHAARPQVQLVESGGGLVQAGASLRLSCAASGRTFTVAAISLSPTLAYYAESVKGRFTISRDNAKNTVVLQMNSLKPEDTALYYCAADRKSVMSIRPDYWGQGTQVTVSSTSTTTPAPRPPTPAPTIASQPLSLRPEACRPAAGGAVHTRGLDFACDIYIWAPLAGTCGVLLLSLVITLYCKRGRKKLLYIFKQPFMRPVQTTQEEDGCSCRFPEEEEGGCELRVKFSRSADAPAYQQGQNQLYNELNLGRREEYDVLDKRRGRDPEMGGKPRRKNPQEGLYNELQKDKMAEAYSEIGMKGERRRGKGHDGLYQGLSTATKDTYDALHMQALPPR

SEQ ID NO: 243 - protein, 371 aa, Artificial Sequence
  Synthetic Construct
MALPVTALLLPLALLLHAARPDVQLVESGGGLEQAGGSLRLSCAASGGTLSKNTVAWFRQAPGKERGFVASITWDGRTTYYADSVKGRFTISRDNAKNTVYLQMNSLKPEDTAVYYCASTASCHLFGLGSGAFVSWGRGTQVTVSSTSTTTPAPRPPTPAPTIASQPLSLRPEACRPAAGGAVHTRGLDFACDIYIWAPLAGTCGVLLLSLVITLYCKRGRKKLLYIFKQPFMRPVQTTQEEDGCSCRFPEEEEGGCELRVKFSRSADAPAYQQGQNQLYNELNLGRREEYDVLDKRRGRDPEMGGKPRRKNPQEGLYNELQKDKMAEAYSEIGMKGERRRGKGHDGLYQGLSTATKDTYDALHMQALPPR

SEQ ID NO: 244 - protein, 362 aa, Artificial Sequence
  Synthetic Construct
MALPVTALLLPLALLLHAARPAVQLVESGGGLVQAGGSLRLSCAASGRTFTMGWFHQAPGKEREFVAAISLSPTLAYYAESVKGRFTISRDNAKNTVVLQMNSLKPEDTALYYCAASKDRYSEYEYWGQGTQVTVSSTSTTTPAPRPPTPAPTIASQPLSLRPEACRPAAGGAVHTRGLDFACDIYIWAPLAGTCGVLLLSLVITLYCKRGRKKLLYIFKQPFMRPVQTTQEEDGCSCRFPEEEEGGCELRVKFSRSADAPAYQQGQNQLYNELNLGRREEYDVLDKRRGRDPEMGGKPRRKNPQEGLYNELQKDKMAEAYSEIGMKGERRRGKGHDGLYQGLSTATKDTYDALHMQALPPR

SEQ ID NO: 245 - protein, 360 aa, Artificial Sequence
  Synthetic Construct
MALPVTALLLPLALLLHAARPQVKLEESGGGLVQAGGSLRLSCAASGRTFTMGWFRQAPGKEREFVAAISLSPTLAYYAESVKGRFTISRDNAKNTVVLQMNSLKPEDTALYYCAKKNGGPVDYWGKGTQVTVSSTSTTTPAPRPPTPAPTIASQPLSLRPEACRPAAGGAVHTRGLDFACDIYIWAPLAGTCGVLLLSLVITLYCKRGRKKLLYIFKQPFMRPVQTTQEEDGCSCRFPEEEEGGCELRVKFSRSADAPAYQQGQNQLYNELNLGRREEYDVLDKRRGRDPEMGGKPRRKNPQEGLYNELQKDKMAEAYSEIGMKGERRRGKGHDGLYQGLSTATKDTYDALHMQALPPR

SEQ ID NO: 246 - protein, 365 aa, Artificial Sequence
  Synthetic Construct
MALPVTALLLPLALLLHAARPDVQLVESGGGLVQPGGSLRLSCAASGRTFSSIVMGWFRQAPGKEREFVGAIMWNDGITYLQDSVKGRFTIFRDNAKNTVYLQMNSLKLEDTAVYYCAASKGRYSEYEYWGQGTQVTVSSTSTTTPAPRPPTPAPTIASQPLSLRPEACRPAAGGAVHTRGLDFACDIYIWAPLAGTCGVLLLSLVITLYCKRGRKKLLYIFKQPFMRPVQTTQEEDGCSCRFPEEEEGGCELRVKFSRSADAPAYQQGQNQLYNELNLGRREEYDVLDKRRGRDPEMGGKPRRKNPQEGLYNELQKDKMAEAYSEIGMKGERRRGKGHDGLYQGLSTATKDTYDALHMQALPPR

SEQ ID NO: 247 - protein, 364 aa, Artificial Sequence
  Synthetic Construct
MALPVTALLLPLALLLHAARPQVKLEESGGRLVQAGGSLKLSWAASGRTFTMGWFRQAPGKEREFVTAINLSPTLTYYAESVKGRFPISRNNAQNTVVLQMNSLKPEDTALYYCAAERKSVMAIPPDYWGQGTQVTVSSTSTTTPAPRPPTPAPTIASQPLSLRPEACRPAAGGAVHTRGLDFACDIYIWAPLAGTCGVLLLSLVITLYCKRGRKKLLYIFKQPFMRPVQTTQEEDGCSCRFPEEEEGGCELRVKFSRSADAPAYQQGQNQLYNELNLGRREEYDVLDKRRGRDPEMGGKPRRKNPQEGLYNELQKDKMAEAYSEIGMKGERRRGKGHDGLYQGLSTATKDTYDALHMQALPPR

SEQ ID NO: 248 - protein, 364 aa, Artificial Sequence
  Synthetic Construct
MALPVTALLLPLALLLHAARPEVQLVESGGGLVQAGGSLRLSCAASGRTFTMGGFRRVPRDEREFVASITLIPTFPYYAYSVKGRFALFRDNPNNTVILLMISLKPEDPDLYYCASYRKYLMSILPDYWGQGTQGTVSSTSTTTPAPRPPTPAPTIASQPLSLRPEACRPAAGGAVHTRGLDFACDIYIWAPLAGTCGVLLLSLVITLYCKRGRKKLLYIFKQPFMRPVQTTQEEDGCSCRFPEEEEGGCELRVKFSRSADAPAYQQGQNQLYNELNLGRREEYDVLDKRRGRDPEMGGKPRRKNPQEGLYNELQKDKMAEAYSEIGMKGERRRGKGHDGLYQGLSTATKDTYDALHMQALPPR

SEQ ID NO: 249 - protein, 370 aa, Artificial Sequence
  Synthetic Construct
MALPVTALLLPLALLLHAARPQVKLEESGGGLVQAGGSLRLSCAASGRTFTMGWFRQAPGKEREFVAAISLSPTLAYYAESVKGRFTISRDNAKNTVDLQMNSLKPEDTAVYFCAANRNSQRVIAALSWIGMNYWGEWTQVTVSSTSTTTPAPRPPTPAPTIASQPLSLRPEACRPAAGGAVHTRGLDFACDIYIWAPLAGTCGVLLLSLVITLYCKRGRKKLLYIFKQPFMRPVQTTQEEDGCSCRFPEEEEGGCELRVKFSRSADAPAYQQGQNQLYNELNLGRREEYDVLDKRRGRDPEMGGKPRRKNPQEGLYNELQKDKMAEAYSEIGMKGERRRGKGHDGLYQGLSTATKDTYDALHMQALPPR

SEQ ID NO: 250 - protein, 362 aa, Artificial Sequence
  Synthetic Construct
MALPVTALLLPLALLLHAARPQVQLVESGGGLVQAGGSLRLSCAASGRTFTMGWFRQAPGKEREFVAAISLSPTLAYYAESVKGRFTISRDNAKKTLYLRMNSLKPEDTAVYYCAARRIDAADFDSWGQGTQVTVSSTSTTTPAPRPPTPAPTIASQPLSLRPEACRPAAGGAVHTRGLDFACDIYIWAPLAGTCGVLLLSLVITLYCKRGRKKLLYIFKQPFMRPVQTTQEEDGCSCRFPEEEEGGCELRVKFSRSADAPAYQQGQNQLYNELNLGRREEYDVLDKRRGRDPEMGGKPRRKNPQEGLYNELQKDKMAEAYSEIGMKGERRRGKGHDGLYQGLSTATKDTYDALHMQALPPR

SEQ ID NO: 251 - protein, 362 aa, Artificial Sequence
  Synthetic Construct
MALPVTALLLPLALLLHAARPQVKLEESGGGLVQAGGSLRLSCAASGRTFTMGWFRRAPGKERESVAVIGWRDINASYADSVKGRFAISRDNAKKTLYLQMNSLKPEDTAVYYCAARRIDATDFDSWGQGTQVTVSSTSTTTPAPRPPTPAPTIASQPLSLRPEACRPAAGGAVHTRGLDFACDIYIWAPLAGTCGVLLLSLVITLYCKRGRKKLLYIFKQPFMRPVQTTQEEDGCSCRFPEEEEGGCELRVKFSRSADAPAYQQGQNQLYNELNLGRREEYDVLDKRRGRDPEMGGKPRRKNPQEGLYNELQKDKMAEAYSEIGMKGERRRGKGHDGLYQGLSTATKDTYDALHMQALPPR

SEQ ID NO: 252 - protein, 365 aa, Artificial Sequence
  Synthetic Construct
MALPVTALLLPLALLLHAARPQVKLEESGGGLVQTGGSLRLSCAASEHTFSNHVMGWFRQAPGKERESVAVIGWRDISTSYADSVKGRFTISRDNAKKTLYLQMNSLKPEDTAVYYCAARRIDAADFDSRGQGTQVTVSSTSTTTPAPRPPTPAPTIASQPLSLRPEACRPAAGGAVHTRGLDFACDIYIWAPLAGTCGVLLLSLVITLYCKRGRKKLLYIFKQPFMRPVQTTQEEDGCSCRFPEEEEGGCELRVKFSRSADAPAYQQGQNQLYNELNLGRREEYDVLDKRRGRDPEMGGKPRRKNPQEGLYNELQKDKMAEAYSEIGMKGERRRGKGHDGLYQGLSTATKDTYDALHMQALPPR

SEQ ID NO: 253 - protein, 369 aa, Artificial Sequence
  Synthetic Construct
MALPVTALLLPLALLLHAARPAVQLVDSGGGLVQAGGSLRISCAVSGRTSSNYILAWFRQAPGKERDFVAHISRSGGKSGYGDSVKGRFTISRDNAENTVRVYLQMNSLKPGDTAVYYCNRPLWYGSPTLIDYWGQGTQVTVSSTSTTTPAPRPPTPAPTIASQPLSLRPEACRPAAGGAVHTRGLDFACDIYIWAPLAGTCGVLLLSLVITLYCKRGRKKLLYIFKQPFMRPVQTTQEEDGCSCRFPEEEEGGCELRVKFSRSADAPAYQQGQNQLYNELNLGRREEYDVLDKRRGRDPEMGGKPRRKNPQEGLYNELQKDKMAEAYSEIGMKGERRRGKGHDGLYQGLSTATKDTYDALHMQALPPR

SEQ ID NO: 254 - protein, 364 aa, Artificial Sequence
  Synthetic Construct
MALPVTALLLPLALLLHAARPQVQLVESGGGLVQAGGSLRLSCAASGRTFTMGWFRQAPGKEREFVAAISLSPTLAYYAESVKGRFTISRDNAKNTVVLQMNSLKPEDTALYYCAADRKSVMSIRPDYWGQGTQVTVSSTSTTTPAPRPPTPAPTIASQPLSLRPEACRPAAGGAVHTRGLDFACDIYIWAPLAGTCGVLLLSLVITLYCKRGRKKLLYIFKQPFMRPVQTTQEEDGCSCRFPEEEEGGCELRVKFSRSADAPAYQQGQNQLYNELNLGRREEYDVLDKRRGRDPEMGGKPRRKNPQEGLYNELQKDKMAEAYSEIGMKGERRRGKGHDGLYQGLSTATKDTYDALHMQALPPR

SEQ ID NO: 255 - protein, 364 aa, Artificial Sequence
  Synthetic Construct
MALPVTALLLPLALLLHAARPAVQLVDSGGGLVQAGGSLRLSCAASGRTFTMGWFRQAPGKEREFVAAISLSPTLAYYAEPVKGRFTISRDNAKNTVVLQMNSLKPEDTALYYCAADRKSVMSIRPDYWGQGTQVTVSSTSTTTPAPRPPTPAPTIASQPLSLRPEACRPAAGGAVHTRGLDFACDIYIWAPLAGTCGVLLLSLVITLYCKRGRKKLLYIFKQPFMRPVQTTQEEDGCSCRFPEEEEGGCELRVKFSRSADAPAYQQGQNQLYNELNLGRREEYDVLDKRRGRDPEMGGKPRRKNPQEGLYNELQKDKMAEAYSEIGMKGERRRGKGHDGLYQGLSTATKDTYDALHMQALPPR

SEQ ID NO: 256 - protein, 367 aa, Artificial Sequence
  Synthetic Construct
MALPVTALLLPLALLLHAARPDVQLVESGGGSVQTGGSLRLSCTASGRTLNNFVMGWFRQAPGKEREFVAAISLSPTLAYYVESVKGRFTISRDNAKNTVVLQMNSLKPEDTALYYCAADRKSVMSIRPDYWGQGTQVTVSSTSTTTPAPRPPTPAPTIASQPLSLRPEACRPAAGGAVHTRGLDFACDIYIWAPLAGTCGVLLLSLVITLYCKRGRKKLLYIFKQPFMRPVQTTQEEDGCSCRFPEEEEGGCELRVKFSRSADAPAYQQGQNQLYNELNLGRREEYDVLDKRRGRDPEMGGKPRRKNPQEGLYNELQKDKMAEAYSEIGMKGERRRGKGHDGLYQGLSTATKDTYDALHMQALPPR

SEQ ID NO: 257 - DNA, 1263 bp, Artificial Sequence
  Synthetic Construct
atggccttaccagtgaccgccttgctcctgccgctggccttgctgctccacgccgccaggccggttaaccgcacgcgtcgcatgcatcaggtgcagctggtggagtctgggggaggcttggtgcagcctgggggttctctgaggctctcctgtgaagcctctggattcactttggattattatgccataggctggttccgccaggccccagggaaggagcgcgagggggtcatatgtattagtagaagtgatggtagcacatactatgcagactccgtgaagggccgattcaccatctccagagacaacgccaagaaaacggtgtatctgcaaatgatcagcctgaaacctgaggacacggccgcttattactgtgcagcaggggccgattgttcggggtacctacgagattatgagttccgggggcaggggacccaggtcaccgtctcctcaactagtaccacgacgccagcgccgcgaccaccaacaccggcgcccaccatcgcgtcgcagcccctgtccctgcgcccagaggcgtgccggccagcggcggggggcgcagtgcacacgagggggctggacttcgcctgtgatttttgggtgctggtggtggttggtggagtcctggcttgctatagcttgctagtaacagtggcctttattattttctgggtgaggagtaagaggagcaggctcctgcacagtgactacatgaacatgactccccgccgccccgggcccacccgcaagcattaccagccctatgccccaccacgcgacttcgcagcctatcgctccaaacggggcagaaagaaactcctgtatatattcaaacaaccatttatgagaccagtacaaactactcaagaggaagatggctgtagctgccgatttccagaagaagaagaaggaggatgtgaactgagagtgaagttcagcaggagcgcagacgcccccgcgtacaagcagggccagaaccagctctataacgagctcaatctaggacgaagagaggagtacgatgttttggacaagagacgtggccgggaccctgagatggggggaaagccgagaaggaagaaccctcaggaaggcctgtacaatgaactgcagaaagataagatggcggaggcctacagtgagattgggatgaaaggcgagcgccggaggggcaaggggcacgatggcctttaccagggtctcagtacagccaccaaggacacctacgacgcccttcacatgcaggccctgccccctcgctga

SEQ ID NO: 258 - DNA, 1281 bp, Artificial Sequence
  Synthetic Construct
atggccttaccagtgaccgccttgctcctgccgctggccttgctgctccacgccgccaggccggttaaccgcacgcgtcgcatgcatcaggtaaagctggaggagtctgggggacgattggtgcagccaaggggctctctgagactctcctgtgcaggctctggacgcactttcagtacctatggtatggcctggttccgccaggctccagggaaggagcgtgagttcgtagcgtctaaagcatcgatgaattacagcggtagaacatactatgcagactccgtgaagggccgattcaccatcgccagagacaacgccaagaacatggtgtttctgcaaatgaacaacctgaagcctgaggacacggccgtttattactgtgcagcgggcactggatgctcaacatatgggtgttttgacgcccagataatagactactggggcaaagggaccctggtcaccgtctcctcaactagtaccacgacgccagcgccgcgaccaccaacaccggcgcccaccatcgcgtcgcagcccctgtccctgcgcccagaggcgtgccggccagcggcggggggcgcagtgcacacgagggggctggacttcgcctgtgatttttgggtgctggtggtggttggtggagtcctggcttgctatagcttgctagtaacagtggcctttattattttctgggtgaggagtaagaggagcaggctcctgcacagtgactacatgaacatgactccccgccgccccgggcccacccgcaagcattaccagccctatgccccaccacgcgacttcgcagcctatcgctccaaacggggcagaaagaaactcctgtatatattcaaacaaccatttatgagaccagtacaaactactcaagaggaagatggctgtagctgccgatttccagaagaagaagaaggaggatgtgaactgagagtgaagttcagcaggagcgcagacgcccccgcgtacaagcagggccagaaccagctctataacgagctcaatctaggacgaagagaggagtacgatgttttggacaagagacgtggccgggaccctgagatggggggaaagccgagaaggaagaaccctcaggaaggcctgtacaatgaactgcagaaagataagatggcggaggcctacagtgagattgggatgaaaggcgagcgccggaggggcaaggggcacgatggcctttaccagggtctcagtacagccaccaaggacacctacgacgcccttcacatgcaggccctgccccctcgctga

SEQ ID NO: 259 - DNA, 1251 bp, Artificial Sequence
  Synthetic Construct
atggccttaccagtgaccgccttgctcctgccgctggccttgctgctccacgccgccaggccggttaaccgcacgcgtcgcatgcatgaggtgcagctggtggagtctgggggaggcttggtgcaggctggggggtctctgagactctcctgtgcagcctctggacgcaccttcaccatggggtggttccgtcaggctccagggaaggagcgtgagtttgtagcagctattagtttgagtcctactttagcatattatgcagagtccgtgaagggccgattcaccatcagccgagacaacgccaagaacacggtggttttgcaaatgaacagcctgaaacctgaggacacggccctttattactgtgcagcagaccggaaatcagtaatgtctattcggcccgactactggggccaggggacccaggtcaccgtctcctcaactagtaccacgacgccagcgccgcgaccaccaacaccggcgcccaccatcgcgtcgcagcccctgtccctgcgcccagaggcgtgccggccagcggcggggggcgcagtgcacacgagggggctggacttcgcctgtgatttttgggtgctggtggtggttggtggagtcctggcttgctatagcttgctagtaacagtggcctttattattttctgggtgaggagtaagaggagcaggctcctgcacagtgactacatgaacatgactccccgccgccccgggcccacccgcaagcattaccagccctatgccccaccacgcgacttcgcagcctatcgctccaaacggggcagaaagaaactcctgtatatattcaaacaaccatttatgagaccagtacaaactactcaagaggaagatggctgtagctgccgatttccagaagaagaagaaggaggatgtgaactgagagtgaagttcagcaggagcgcagacgcccccgcgtacaagcagggccagaaccagctctataacgagctcaatctaggacgaagagaggagtacgatgttttggacaagagacgtggccgggaccctgagatggggggaaagccgagaaggaagaaccctcaggaaggcctgtacaatgaactgcagaaagataagatggcggaggcctacagtgagattgggatgaaaggcgagcgccggaggggcaaggggcacgatggcctttaccagggtctcagtacagccaccaaggacacctacgacgcccttcacatgcaggccctgccccctcgctga

SEQ ID NO: 260 - DNA, 1257 bp, Artificial Sequence
  Synthetic Construct
atggccttaccagtgaccgccttgctcctgccgctggccttgctgctccacgccgccaggccggttaaccgcacgcgtcgcatgcatgccgtgcagctggtggattctgggggaggcttggtgcagcctggggggtctctgagactctcctgtgtagcctctggaggtatcttcgtcatcaatgccatgggctggtaccgccaggctccaggaaagcagcgcgagttggtcgcatctattcgtggactaggcagaacaaactatgacgactccgtgaagggccgattcaccatctccagagacaacgccaacaacacggtgtatctgcagatgaacagcctggaacctgaggacacggccgtctactactgtacagtctacgttacactacttggtggggttaatagggactactggggccaggggacccaggtcaccgtctcctcaactagtaccacgacgccagcgccgcgaccaccaacaccggcgcccaccatcgcgtcgcagcccctgtccctgcgcccagaggcgtgccggccagcggcggggggcgcagtgcacacgagggggctggacttcgcctgtgatttttgggtgctggtggtggttggtggagtcctggcttgctatagcttgctagtaacagtggcctttattattttctgggtgaggagtaagaggagcaggctcctgcacagtgactacatgaacatgactccccgccgccccgggcccacccgcaagcattaccagccctatgccccaccacgcgacttcgcagcctatcgctccaaacggggcagaaagaaactcctgtatatattcaaacaaccatttatgagaccagtacaaactactcaagaggaagatggctgtagctgccgatttccagaagaagaagaaggaggatgtgaactgagagtgaagttcagcaggagcgcagacgcccccgcgtacaagcagggccagaaccagctctataacgagctcaatctaggacgaagagaggagtacgatgttttggacaagagacgtggccgggaccctgagatggggggaaagccgagaaggaagaaccctcaggaaggcctgtacaatgaactgcagaaagataagatggcggaggcctacagtgagattgggatgaaaggcgagcgccggaggggcaaggggcacgatggcctttaccagggtctcagtacagccaccaaggacacctacgacgcccttcacatgcaggccctgccccctcgctga

SEQ ID NO: 261 - DNA, 1254 bp, Artificial Sequence
  Synthetic Construct
atggccttaccagtgaccgccttgctcctgccgctggccttgctgctccacgccgccaggccggttaaccgcacgcgtcgcatgcatgaggtgcagctggtggagtctgggggaggattggtgcaggctgggggctctctgagactctcctgtgcagcctctggacggaccttcagtagcattgtcatgggctggttccgccaggctccagggaaggagcgtgagtttgtaggagcgattatgtggaatgatggtattacatacttgcaagactccgtgaagggccgatttaccatcttcagagacaatgccaagaacacggtgtatctgcaaatgaacagcctgaaacttgaggatacggccgtttattactgtgcagcatccaagggtagatactcggaatatgagtactggggccaggggacccaggtcaccgtctcctcaactagtaccacgacgccagcgccgcgaccaccaacaccggcgcccaccatcgcgtcgcagcccctgtccctgcgcccagaggcgtgccggccagcggcggggggcgcagtgcacacgagggggctggacttcgcctgtgatttttgggtgctggtggtggttggtggagtcctggcttgctatagcttgctagtaacagtggcctttattattttctgggtgaggagtaagaggagcaggctcctgcacagtgactacatgaacatgactccccgccgccccgggcccacccgcaagcattaccagccctatgccccaccacgcgacttcgcagcctatcgctccaaacggggcagaaagaaactcctgtatatattcaaacaaccatttatgagaccagtacaaactactcaagaggaagatggctgtagctgccgatttccagaagaagaagaaggaggatgtgaactgagagtgaagttcagcaggagcgcagacgcccccgcgtacaagcagggccagaaccagctctataacgagctcaatctaggacgaagagaggagtacgatgttttggacaagagacgtggccgggaccctgagatggggggaaagccgagaaggaagaaccctcaggaaggcctgtacaatgaactgcagaaagataagatggcggaggcctacagtgagattgggatgaaaggcgagcgccggaggggcaaggggcacgatggcctttaccagggtctcagtacagccaccaaggacacctacgacgcccttcacatgcaggccctgccccctcgctga

SEQ ID NO: 262 - DNA, 1281 bp, Artificial Sequence
  Synthetic Construct
atggccttaccagtgaccgccttgctcctgccgctggccttgctgctccacgccgccaggccggttaaccgcacgcgtcgcatgcatgaggtgcagctggtggagtctgggggaggcgtggtgcaggctggggggtctctgacagtctcctgtacagcctctggattcactttcgaccgtgctgtcatagtctggttccgccaggcccccgggaagggccgtgagggggtctcatttattaaacctagtgatggcaccatatactacattgactccctgaagggccgattcacgatctccagtgacatcgccaagaatacggtatatctgcaaatgaaaagtctggaatcggaggactcggccgtttattactgtgcggcctcgcctgaggactggtacacggattggatcgactggagtatatatcggtggcagcactggggccaggggacccaggtcactgtctcctcaactagtaccacgacgccagcgccgcgaccaccaacaccggcgcccaccatcgcgtcgcagcccctgtccctgcgcccagaggcgtgccggccagcggcggggggcgcagtgcacacgagggggctggacttcgcctgtgatttttgggtgctggtggtggttggtggagtcctggcttgctatagcttgctagtaacagtggcctttattattttctgggtgaggagtaagaggagcaggctcctgcacagtgactacatgaacatgactccccgccgccccgggcccacccgcaagcattaccagccctatgccccaccacgcgacttcgcagcctatcgctccaaacggggcagaaagaaactcctgtatatattcaaacaaccatttatgagaccagtacaaactactcaagaggaagatggctgtagctgccgatttccagaagaagaagaaggaggatgtgaactgagagtgaagttcagcaggagcgcagacgcccccgcgtacaagcagggccagaaccagctctataacgagctcaatctaggacgaagagaggagtacgatgttttggacaagagacgtggccgggaccctgagatggggggaaagccgagaaggaagaaccctcaggaaggcctgtacaatgaactgcagaaagataagatggcggaggcctacagtgagattgggatgaaaggcgagcgccggaggggcaaggggcacgatggcctttaccagggtctcagtacagccaccaaggacacctacgacgcccttcacatgcaggccctgccccctcgctga

SEQ ID NO: 263 - DNA, 1254 bp, Artificial Sequence
  Synthetic Construct
atggccttaccagtgaccgccttgctcctgccgctggccttgctgctccacgccgccaggccggttaaccgcacgcgtcgcatgcatgaggtgcagctggtggagtctgggggaggaatggtgcaggctggggactctctgagactatcctgtgtgcagtctacttacaccgtcaatagcgatgtcatgggctggttccgccaggctccagggaaggagcgtgagtttgtaggagcgattatgtggaatgatggtattacatacttgcaagactccgtgaagggccgatttaccatcttcagagacaacgccaagaacacggtgtatctgcaaatgaacagcctgaaacttgaggatacggccgtttattactgtgcagcatccaagggtagatactcggaatatgagtactggggccaggggacccaggtcaccgtctcctcaactagtaccacgacgccagcgccgcgaccaccaacaccggcgcccaccatcgcgtcgcagcccctgtccctgcgcccagaggcgtgccggccagcggcggggggcgcagtgcacacgagggggctggacttcgcctgtgatttttgggtgctggtggtggttggtggagtcctggcttgctatagcttgctagtaacagtggcctttattattttctgggtgaggagtaagaggagcaggctcctgcacagtgactacatgaacatgactccccgccgccccgggcccacccgcaagcattaccagccctatgccccaccacgcgacttcgcagcctatcgctccaaacggggcagaaagaaactcctgtatatattcaaacaaccatttatgagaccagtacaaactactcaagaggaagatggctgtagctgccgatttccagaagaagaagaaggaggatgtgaactgagagtgaagttcagcaggagcgcagacgcccccgcgtacaagcagggccagaaccagctctataacgagctcaatctaggacgaagagaggagtacgatgttttggacaagagacgtggccgggaccctgagatggggggaaagccgagaaggaagaaccctcaggaaggcctgtacaatgaactgcagaaagataagatggcggaggcctacagtgagattgggatgaaaggcgagcgccggaggggcaaggggcacgatggcctttaccagggtctcagtacagccaccaaggacacctacgacgcccttcacatgcaggccctgccccctcgctga

SEQ ID NO: 264 - DNA, 1257 bp, Artificial Sequence
  Synthetic Construct
atggccttaccagtgaccgccttgctcctgccgctggccttgctgctccacgccgccaggccggttaaccgcacgcgtcgcatgcatgcggtgcagctggtggagtctgggggaggattggtgcaggctggggactctctgagactctcctgtacagcctctggtgcaaccttgactaacgatcacatggcatggttccgccaggctccagggaaggggcgtgaatttgtagcagctattgactggagtggtcgtaccacaaattacgcagaccccgtagagggccgattcaccatctccagaaacaacgccaagaacacggtgtatctggaaatgaacagcctgaaacttgaggacacggccgtttattactgtgcggtcctccgcgcttggatctcatatgacaatgactactggggccaggggacccaggtcaccgtctcctcaactagtaccacgacgccagcgccgcgaccaccaacaccggcgcccaccatcgcgtcgcagcccctgtccctgcgcccagaggcgtgccggccagcggcggggggcgcagtgcacacgagggggctggacttcgcctgtgatttttgggtgctggtggtggttggtggagtcctggcttgctatagcttgctagtaacagtggcctttattattttctgggtgaggagtaagaggagcaggctcctgcacagtgactacatgaacatgactccccgccgccccgggcccacccgcaagcattaccagccctatgccccaccacgcgacttcgcagcctatcgctccaaacggggcagaaagaaactcctgtatatattcaaacaaccatttatgagaccagtacaaactactcaagaggaagatggctgtagctgccgatttccagaagaagaagaaggaggatgtgaactgagagtgaagttcagcaggagcgcagacgcccccgcgtacaagcagggccagaaccagctctataacgagctcaatctaggacgaagagaggagtacgatgttttggacaagagacgtggccgggaccctgagatggggggaaagccgagaaggaagaaccctcaggaaggcctgtacaatgaactgcagaaagataagatggcggaggcctacagtgagattgggatgaaaggcgagcgccggaggggcaaggggcacgatggcctttaccagggtctcagtacagccaccaaggacacctacgacgcccttcacatgcaggccctgccccctcgctga

SEQ ID NO: 265 - DNA, 1257 bp, Artificial Sequence
  Synthetic Construct
atggccttaccagtgaccgccttgctcctgccgctggccttgctgctccacgccgccaggccggttaaccgcacgcgtcgcatgcatcaggtgcagctggtggagtctgggggaggattggtgcaggctgggggctctctgagactctcctgtgcagcctctggaggcaccttaagtaaaaataccgtggcttggttccgccaggctccagggaaggagcgtgggtttgtagcgtctattacctgggatggtcgtacgacatactatgcagactccgtgaagggccgattcaccatctccagagacaacgccaagaacacagtgtatctgcaaatgaacagcctgaaacctgaggatacggccgtttatgtctgtgcagacttagggaaatggcctgcgggcccggcggactactggggccaggggacccaggtcaccgtctcctcaactagtaccacgacgccagcgccgcgaccaccaacaccggcgcccaccatcgcgtcgcagcccctgtccctgcgcccagaggcgtgccggccagcggcggggggcgcagtgcacacgagggggctggacttcgcctgtgatttttgggtgctggtggtggttggtggagtcctggcttgctatagcttgctagtaacagtggcctttattattttctgggtgaggagtaagaggagcaggctcctgcacagtgactacatgaacatgactccccgccgccccgggcccacccgcaagcattaccagccctatgccccaccacgcgacttcgcagcctatcgctccaaacggggcagaaagaaactcctgtatatattcaaacaaccatttatgagaccagtacaaactactcaagaggaagatggctgtagctgccgatttccagaagaagaagaaggaggatgtgaactgagagtgaagttcagcaggagcgcagacgcccccgcgtacaagcagggccagaaccagctctataacgagctcaatctaggacgaagagaggagtacgatgttttggacaagagacgtggccgggaccctgagatggggggaaagccgagaaggaagaaccctcaggaaggcctgtacaatgaactgcagaaagataagatggcggaggcctacagtgagattgggatgaaaggcgagcgccggaggggcaaggggcacgatggcctttaccagggtctcagtacagccaccaaggacacctacgacgcccttcacatgcaggccctgccccctcgctga

SEQ ID NO: 266 - DNA, 1254 bp, Artificial Sequence
  Synthetic Construct
atggccttaccagtgaccgccttgctcctgccgctggccttgctgctccacgccgccaggccggttaaccgcacgcgtcgcatgcatcaggtaaagctggaggagtctgggggaggcttggtgcaggctgggcggtctctgagactctcctgtgcagcctctgaacacaccttcagtagccatgtcatgggctggttccgccaggctccagggaaggagcgtgagtctgttgcagttattggctggagagatattagcacaagctatgcagactccgtgaagggccgattcaccatctccagagacaacgccaagaagacgctgtatctgcaaatgaatagcctgaaacctgaggacacggccgtttactactgtgcagcacgtcggatcgacgcagctgactttgattcctgggggcaggggacccaggtcaccgtctcctcgactagtaccacgacgccagcgccgcgaccaccaacaccggcgcccaccatcgcgtcgcagcccctgtccctgcgcccagaggcgtgccggccagcggcggggggcgcagtgcacacgagggggctggacttcgcctgtgatttttgggtgctggtggtggttggtggagtcctggcttgctatagcttgctagtaacagtggcctttattattttctgggtgaggagtaagaggagcaggctcctgcacagtgactacatgaacatgactccccgccgccccgggcccacccgcaagcattaccagccctatgccccaccacgcgacttcgcagcctatcgctccaaacggggcagaaagaaactcctgtatatattcaaacaaccatttatgagaccagtacaaactactcaagaggaagatggctgtagctgccgatttccagaagaagaagaaggaggatgtgaactgagagtgaagttcagcaggagcgcagacgcccccgcgtacaagcagggccagaaccagctctataacgagctcaatctaggacgaagagaggagtacgatgttttggacaagagacgtggccgggaccctgagatggggggaaagccgagaaggaagaaccctcaggaaggcctgtacaatgaactgcagaaagataagatggcggaggcctacagtgagattgggatgaaaggcgagcgccggaggggcaaggggcacgatggcctttaccagggtctcagtacagccaccaaggacacctacgacgcccttcacatgcaggccctgccccctcgctga

SEQ ID NO: 267 - DNA, 1254 bp, Artificial Sequence
  Synthetic Construct
atggccttaccagtgaccgccttgctcctgccgctggccttgctgctccacgccgccaggccggttaaccgcacgcgtcgcatgcatgcggtgcagctggtggagtctgggggaggattggtgcaggctggggactctctgagactcacctgtacagcctctggacgcgccttcagtacctatttcatggcctggttccgccaggctccagggaaggagcgtgagtttgtagcaggaattgcatggagtggtggtagcacggcgtatgcagactccgtgaagggccgattcaccatctccagagacaacgccaagaacacggtgtatctgcaaatgaacagcctgaaatctgaggacacggccgtttattactgtgccagcagggggattgaggtcgaagagtttggtgcctggggccaggggacccaggtcaccgtctcgtcgactagtaccacgacgccagcgccgcgaccaccaacaccggcgcccaccatcgcgtcgcagcccctgtccctgcgcccagaggcgtgccggccagcggcggggggcgcagtgcacacgagggggctggacttcgcctgtgatttttgggtgctggtggtggttggtggagtcctggcttgctatagcttgctagtaacagtggcctttattattttctgggtgaggagtaagaggagcaggctcctgcacagtgactacatgaacatgactccccgccgccccgggcccacccgcaagcattaccagccctatgccccaccacgcgacttcgcagcctatcgctccaaacggggcagaaagaaactcctgtatatattcaaacaaccatttatgagaccagtacaaactactcaagaggaagatggctgtagctgccgatttccagaagaagaagaaggaggatgtgaactgagagtgaagttcagcaggagcgcagacgcccccgcgtacaagcagggccagaaccagctctataacgagctcaatctaggacgaagagaggagtacgatgttttggacaagagacgtggccgggaccctgagatggggggaaagccgagaaggaagaaccctcaggaaggcctgtacaatgaactgcagaaagataagatggcggaggcctacagtgagattgggatgaaaggcgagcgccggaggggcaaggggcacgatggcctttaccagggtctcagtacagccaccaaggacacctacgacgcccttcacatgcaggccctgccccctcgctga

SEQ ID NO: 268 - DNA, 1131 bp, Artificial Sequence
  Synthetic Construct
atggccttaccagtgaccgccttgctcctgccgctggccttgctgctccacgccgccaggccggttaaccgcacgcgtcgcatgcatcaggtgcagctggtggagtctgggggaggcttggtgcagcctgggggttctctgaggctctcctgtgaagcctctggattcactttggattattatgccataggctggttccgccaggccccagggaaggagcgcgagggggtcatatgtattagtagaagtgatggtagcacatactatgcagactccgtgaagggccgattcaccatctccagagacaacgccaagaaaacggtgtatctgcaaatgatcagcctgaaacctgaggacacggccgcttattactgtgcagcaggggccgattgttcggggtacctacgagattatgagttccgggggcaggggacccaggtcaccgtctcctcaactagtaccacgacgccagcgccgcgaccaccaacaccggcgcccaccatcgcgtcgcagcccctgtccctgcgcccagaggcgtgccggccagcggcggggggcgcagtgcacacgagggggctggacttcgcctgtgatatctacatctgggcgcccttggccgggacttgtggggtccttctcctgtcactggttatcaccctttactgcaaacggggcagaaagaaactcctgtatatattcaaacaaccatttatgagaccagtacaaactactcaagaggaagatggctgtagctgccgatttccagaagaagaagaaggaggatgtgaactgagagtgaagttcagcaggagcgcagacgcccccgcgtaccagcagggccagaaccagctctataacgagctcaatctaggacgaagagaggagtacgatgttttggacaagagacgtggccgggaccctgagatggggggaaagccgagaaggaagaaccctcaggaaggcctgtacaatgaactgcagaaagataagatggcggaggcctacagtgagattgggatgaaaggcgagcgccggaggggcaaggggcacgatggcctttaccagggtctcagtacagccaccaaggacacctacgacgcccttcacatgcaggccctgccccctcgctaa

SEQ ID NO: 269 - DNA, 1122 bp, Artificial Sequence
  Synthetic Construct
atggccttaccagtgaccgccttgctcctgccgctggccttgctgctccacgccgccaggccggttaaccgcacgcgtcgcatgcatcaggtaaagctggaggagtctgggggaggcttggtgcaggctgggcggtctctgagactctcctgtgcagcctctgaacacaccttcagtagccatgtcatgggctggttccgccaggctccagggaaggagcgtgagtctgttgcagttattggctggagagatattagcacaagctatgcagactccgtgaagggccgattcaccatctccagagacaacgccaagaagacgctgtatctgcaaatgaatagcctgaaacctgaggacacggccgtttactactgtgcagcacgtcggatcgacgcagctgactttgattcctgggggcaggggacccaggtcaccgtctcctcgactagtaccacgacgccagcgccgcgaccaccaacaccggcgcccaccatcgcgtcgcagcccctgtccctgcgcccagaggcgtgccggccagcggcggggggcgcagtgcacacgagggggctggacttcgcctgtgatatctacatctgggcgcccttggccgggacttgtggggtccttctcctgtcactggttatcaccctttactgcaaacggggcagaaagaaactcctgtatatattcaaacaaccatttatgagaccagtacaaactactcaagaggaagatggctgtagctgccgatttccagaagaagaagaaggaggatgtgaactgagagtgaagttcagcaggagcgcagacgcccccgcgtaccagcagggccagaaccagctctataacgagctcaatctaggacgaagagaggagtacgatgttttggacaagagacgtggccgggaccctgagatggggggaaagccgagaaggaagaaccctcaggaaggcctgtacaatgaactgcagaaagataagatggcggaggcctacagtgagattgggatgaaaggcgagcgccggaggggcaaggggcacgatggcctttaccagggtctcagtacagccaccaaggacacctacgacgcccttcacatgcaggccctgccccctcgctaa

SEQ ID NO: 270 - DNA, 1119 bp, Artificial Sequence
  Synthetic Construct
atggccttaccagtgaccgccttgctcctgccgctggccttgctgctccacgccgccaggccggttaaccgcacgcgtcgcatgcatgaggtgcagctggtggagtctgggggaggcttggtgcaggctggggggtctctgagactctcctgtgcagcctctggacgcaccttcaccatggggtggttccgtcaggctccagggaaggagcgtgagtttgtagcagctattagtttgagtcctactttagcatattatgcagagtccgtgaagggccgattcaccatcagccgagacaacgccaagaacacggtggttttgcaaatgaacagcctgaaacctgaggacacggccctttattactgtgcagcagaccggaaatcagtaatgtctattcggcccgactactggggccaggggacccaggtcaccgtctcctcaactagtaccacgacgccagcgccgcgaccaccaacaccggcgcccaccatcgcgtcgcagcccctgtccctgcgcccagaggcgtgccggccagcggcggggggcgcagtgcacacgagggggctggacttcgcctgtgatatctacatctgggcgcccttggccgggacttgtggggtccttctcctgtcactggttatcaccctttactgcaaacggggcagaaagaaactcctgtatatattcaaacaaccatttatgagaccagtacaaactactcaagaggaagatggctgtagctgccgatttccagaagaagaagaaggaggatgtgaactgagagtgaagttcagcaggagcgcagacgcccccgcgtaccagcagggccagaaccagctctataacgagctcaatctaggacgaagagaggagtacgatgttttggacaagagacgtggccgggaccctgagatggggggaaagccgagaaggaagaaccctcaggaaggcctgtacaatgaactgcagaaagataagatggcggaggcctacagtgagattgggatgaaaggcgagcgccggaggggcaaggggcacgatggcctttaccagggtctcagtacagccaccaaggacacctacgacgcccttcacatgcaggccctgccccctcgctaa

SEQ ID NO: 271 - DNA, 1113 bp, Artificial Sequence
  Synthetic Construct
atggctctgcccgtcaccgctctgctgctgcctctggctctgctgctgcacgctgctcgccctgaggtgcagctggtggagtctgggggaggcttggtgccgcctggggggtctctgagactctcctgtacagcctctggaagcacagtcagcatcaatgtcatggcctggtaccgccaggtttcagggaagcagcgcgagttggtcgcggccgttactagggatggtaggaaaagttgtggagactccgtgaagggccgattcaccatttccagagacggcgccaagaatgcggtatatttgcaaatgaacagtctgaaacctgaggacacagcggtctatttatgtggagccgatggttggggtgctactaccttagattatacctacggcatggactattggggcaaagggacccaggtcaccgtctcctcaactagtaccacgacgccagcgccgcgaccaccaacaccggcgcccaccatcgcgtcgcagcccctgtccctgcgcccagaggcgtgccggccagcggcggggggcgcagtgcacacgagggggctggacttcgcctgtgatatctacatctgggcgcccttggccgggacttgtggggtccttctcctgtcactggttatcaccctttactgcaaacggggcagaaagaaactcctgtatatattcaaacaaccatttatgagaccagtacaaactactcaagaggaagatggctgtagctgccgatttccagaagaagaagaaggaggatgtgaactgagagtgaagttcagcaggagcgcagacgcccccgcgtaccagcagggccagaaccagctctataacgagctcaatctaggacgaagagaggagtacgatgttttggacaagagacgtggccgggaccctgagatggggggaaagccgagaaggaagaaccctcaggaaggcctgtacaatgaactgcagaaagataagatggcggaggcctacagtgagattgggatgaaaggcgagcgccggaggggcaaggggcacgatggcctttaccagggtctcagtacagccaccaaggacacctacgacgcccttcacatgcaggccctgccccctcgctaa

SEQ ID NO: 272 - DNA, 1095 bp, Artificial Sequence
  Synthetic Construct
atggctctgcccgtcaccgctctgctgctgcctctggctctgctgctgcacgctgctcgccctgcggtgcagctggtggagtctgggggaggattggtgcaggctgggggctctctgagactctcctgtgcagcctctggacgcaccttcaccatggggtggttccgtcaggctccagggaaggagcgtgggtttgtagcgtctattacctgggatggtcgttcggcatactatgcagagtccgtgaagggccgattcaccatcagccgagacaacgccaagaacacggtggttttgcaaatgaacagcctgaaacctgaggacacggccctttattactgtgcagcagaccggaaatcagtaatgtctattcggcccgactactggggccaggggacccaggtcaccgtctcctcaactagtaccacgacgccagcgccgcgaccaccaacaccggcgcccaccatcgcgtcgcagcccctgtccctgcgcccagaggcgtgccggccagcggcggggggcgcagtgcacacgagggggctggacttcgcctgtgatatctacatctgggcgcccttggccgggacttgtggggtccttctcctgtcactggttatcaccctttactgcaaacggggcagaaagaaactcctgtatatattcaaacaaccatttatgagaccagtacaaactactcaagaggaagatggctgtagctgccgatttccagaagaagaagaaggaggatgtgaactgagagtgaagttcagcaggagcgcagacgcccccgcgtaccagcagggccagaaccagctctataacgagctcaatctaggacgaagagaggagtacgatgttttggacaagagacgtggccgggaccctgagatggggggaaagccgagaaggaagaaccctcaggaaggcctgtacaatgaactgcagaaagataagatggcggaggcctacagtgagattgggatgaaaggcgagcgccggaggggcaaggggcacgatggcctttaccagggtctcagtacagccaccaaggacacctacgacgcccttcacatgcaggccctgccccctcgctaa

SEQ ID NO: 273 - DNA, 1107 bp, Artificial Sequence
  Synthetic Construct
atggctctgcccgtcaccgctctgctgctgcctctggctctgctgctgcacgctgctcgccctcaggtacagctggtggagtctgggggaggattggtgcagcctggggggtctctaagactcgcatgtgaagcgcctggaagcggcaatagtatcaatgccatgggctggtaccggcagactccggggaagcggcgcgagttggtcgcaactattactcggggtggtagcacgaactatggaccctccgtgaagggccgattcacgatcaccagagacaatgtcaagaatacggtgcatctgcagatgaacagcctgaaacctgacgacacggccgtctattattgcaatgcggagaggctggacggctcggggtacggatatgagtatgattactggggccaggggacccaggtcaccgtctcctcaactagtaccacgacgccagcgccgcgaccaccaacaccggcgcccaccatcgcgtcgcagcccctgtccctgcgcccagaggcgtgccggccagcggcggggggcgcagtgcacacgagggggctggacttcgcctgtgatatctacatctgggcgcccttggccgggacttgtggggtccttctcctgtcactggttatcaccctttactgcaaacggggcagaaagaaactcctgtatatattcaaacaaccatttatgagaccagtacaaactactcaagaggaagatggctgtagctgccgatttccagaagaagaagaaggaggatgtgaactgagagtgaagttcagcaggagcgcagacgcccccgcgtaccagcagggccagaaccagctctataacgagctcaatctaggacgaagagaggagtacgatgttttggacaagagacgtggccgggaccctgagatggggggaaagccgagaaggaagaaccctcaggaaggcctgtacaatgaactgcagaaagataagatggcggaggcctacagtgagattgggatgaaaggcgagcgccggaggggcaaggggcacgatggcctttaccagggtctcagtacagccaccaaggacacctacgacgcccttcacatgcaggccctgccccctcgctaa

SEQ ID NO: 274 - DNA, 1104 bp, Artificial Sequence
  Synthetic Construct
atggctctgcccgtcaccgctctgctgctgcctctggctctgctgctgcacgctgctcgccctcaggtaaagctggaggagtctgggggaggattggtgcaggctgggggctctctgagactctcctgtgcagcctctggaggcaccttaagtaagaataccgtggcttgggtccgccaggctccagggaaggagcgtgggtttgtaacgtctattacctgtgatggtcgtacgacatactatgcgaactccgtaaacggccgattccccatcaaccgaaacaacgccgagaatttggtggttttgcaaatgaacagcctgaaacctgacgacacggccctttattactgtgcagcataccggaagtcaataatgtctattcagcccgactactggggccaggggacccaggtcaccgtctcctcaactagtaccacgacgccagcgccgcgaccaccaacaccggcgcccaccatcgcgtcgcagcccctgtccctgcgcccagaggcgtgccggccagcggcggggggcgcagtgcacacgagggggctggacttcgcctgtgatatctacatctgggcgcccttggccgggacttgtggggtccttctcctgtcactggttatcaccctttactgcaaacggggcagaaagaaactcctgtatatattcaaacaaccatttatgagaccagtacaaactactcaagaggaagatggctgtagctgccgatttccagaagaagaagaaggaggatgtgaactgagagtgaagttcagcaggagcgcagacgcccccgcgtaccagcagggccagaaccagctctataacgagctcaatctaggacgaagagaggagtacgatgttttggacaagagacgtggccgggaccctgagatggggggaaagccgagaaggaagaaccctcaggaaggcctgtacaatgaactgcagaaagataagatggcggaggcctacagtgagattgggatgaaaggcgagcgccggaggggcaaggggcacgatggcctttaccagggtctcagtacagccaccaaggacacctacgacgcccttcacatgcaggccctgccccctcgctaa

SEQ ID NO: 275 - DNA, 1104 bp, Artificial Sequence
  Synthetic Construct
atggctctgcccgtcaccgctctgctgctgcctctggctctgctgctgcacgctgctcgccctgatgtgcagctggtggagtctgggggaggattggtgcaggctgggggctctctgagactctcctgtgcagcctctggacggaccttcagtagcattgtcatgggctggttccgccaggctccagggaaggagcgtgagtttgtaggagcgattatgtggaatgatggtctgacatacttgcaagggtccgtgaagggccgattcaccatttccagagacaacgccaagaacacggtggttttgcaaatgaacagcctgaaacctgaggacacggccctttattactgtgcagcagaccggaaatcagtaatgtctattcggcccgactactggggccaggggacccaggtcaccgtctcctcaactagtaccacgacgccagcgccgcgaccaccaacaccggcgcccaccatcgcgtcgcagcccctgtccctgcgcccagaggcgtgccggccagcggcggggggcgcagtgcacacgagggggctggacttcgcctgtgatatctacatctgggcgcccttggccgggacttgtggggtccttctcctgtcactggttatcaccctttactgcaaacggggcagaaagaaactcctgtatatattcaaacaaccatttatgagaccagtacaaactactcaagaggaagatggctgtagctgccgatttccagaagaagaagaaggaggatgtgaactgagagtgaagttcagcaggagcgcagacgcccccgcgtaccagcagggccagaaccagctctataacgagctcaatctaggacgaagagaggagtacgatgttttggacaagagacgtggccgggaccctgagatggggggaaagccgagaaggaagaaccctcaggaaggcctgtacaatgaactgcagaaagataagatggcggaggcctacagtgagattgggatgaaaggcgagcgccggaggggcaaggggcacgatggcctttaccagggtctcagtacagccaccaaggacacctacgacgcccttcacatgcaggccctgccccctcgctaa

SEQ ID NO: 276 - DNA, 1089 bp, Artificial Sequence
  Synthetic Construct
atggctctgcccgtcaccgctctgctgctgcctctggctctgctgctgcacgctgctcgccctcaggtacagctggtggagtctgggggaggattggtgcaggctgggggctctctgagactctcctgtgcagcctctggacgcaccttcaccatggggtggttccgtcaggctccagggaaggagcgtgagtttgtagcagctattagtttgagtcctactttagcatattatgcagagtccgtgaagggccgattcaccatcagccgagacaacgccaagaacacggtggttttgcaaatgaacagcctgaaacctgaggacacggccgtttactactgtgcagcacgtcggatcgacgcagctgactttgattcctgggggcaggggacccaggtcaccgtctcctcaactagtaccacgacgccagcgccgcgaccaccaacaccggcgcccaccatcgcgtcgcagcccctgtccctgcgcccagaggcgtgccggccagcggcggggggcgcagtgcacacgagggggctggacttcgcctgtgatatctacatctgggcgcccttggccgggacttgtggggtccttctcctgtcactggttatcaccctttactgcaaacggggcagaaagaaactcctgtatatattcaaacaaccatttatgagaccagtacaaactactcaagaggaagatggctgtagctgccgatttccagaagaagaagaaggaggatgtgaactgagagtgaagttcagcaggagcgcagacgcccccgcgtaccagcagggccagaaccagctctataacgagctcaatctaggacgaagagaggagtacgatgttttggacaagagacgtggccgggaccctgagatggggggaaagccgagaaggaagaaccctcaggaaggcctgtacaatgaactgcagaaagataagatggcggaggcctacagtgagattgggatgaaaggcgagcgccggaggggcaaggggcacgatggcctttaccagggtctcagtacagccaccaaggacacctacgacgcccttcacatgcaggccctgccccctcgctaa

SEQ ID NO: 277 - DNA, 1101 bp, Artificial Sequence
  Synthetic Construct
atggctctgcccgtcaccgctctgctgctgcctctggctctgctgctgcacgctgctcgccctcaggtacagctggtggagtctgggggaggattggtgcaggctgggggctctctgagactctcctgtgcagcctctggaggcaccttaagtaaaaataccgtggcttggttccgccaggctccagggaaggagcgtgggtttgtagcgtctattacctgggatggtcgtacgacatactatgcagactccgtgaagggccgattcaccatctccagagacaacgccaagaacacagtgtatctgcaaatgaacagcctgaaacctgaggatacggccgtttatgtctgtgcagacttagggaaatggcctgcgggcccggcggactactggggccaggggacccaggtcaccgtctcctcaactagtaccacgacgccagcgccgcgaccaccaacaccggcgcccaccatcgcgtcgcagcccctgtccctgcgcccagaggcgtgccggccagcggcggggggcgcagtgcacacgagggggctggacttcgcctgtgatatctacatctgggcgcccttggccgggacttgtggggtccttctcctgtcactggttatcaccctttactgcaaacggggcagaaagaaactcctgtatatattcaaacaaccatttatgagaccagtacaaactactcaagaggaagatggctgtagctgccgatttccagaagaagaagaaggaggatgtgaactgagagtgaagttcagcaggagcgcagacgcccccgcgtaccagcagggccagaaccagctctataacgagctcaatctaggacgaagagaggagtacgatgttttggacaagagacgtggccgggaccctgagatggggggaaagccgagaaggaagaaccctcaggaaggcctgtacaatgaactgcagaaagataagatggcggaggcctacagtgagattgggatgaaaggcgagcgccggaggggcaaggggcacgatggcctttaccagggtctcagtacagccaccaaggacacctacgacgcccttcacatgcaggccctgccccctcgctaa

SEQ ID NO: 278 - DNA, 1104 bp, Artificial Sequence
  Synthetic Construct
atggctctgcccgtcaccgctctgctgctgcctctggctctgctgctgcacgctgctcgccctcaggtgcagctggtggagtctgggggaggcttggtgcagcctggggggtctctgacactctcctgtgcagcctctggaagcatcgacagtatcaataccatggactggttccgtcaggctccagggaaggagcgtgagtttgtagcagctattagtttgagtcccactttagcatattatgcagagtccgtgaagggccgattcaccatcagccgagacaacgccaagaacacggtggttttgcaaatgaacagcctgaaacctgaggacacggccctttattactgtgcagcagaccggaaatcagtaatgtctattcggcccgactactggggccaggggacccaggtcaccgtctcctcaactagtaccacgacgccagcgccgcgaccaccaacaccggcgcccaccatcgcgtcgcagcccctgtccctgcgcccagaggcgtgccggccagcggcggggggcgcagtgcacacgagggggctggacttcgcctgtgatatctacatctgggcgcccttggccgggacttgtggggtccttctcctgtcactggttatcaccctttactgcaaacggggcagaaagaaactcctgtatatattcaaacaaccatttatgagaccagtacaaactactcaagaggaagatggctgtagctgccgatttccagaagaagaagaaggaggatgtgaactgagagtgaagttcagcaggagcgcagacgcccccgcgtaccagcagggccagaaccagctctataacgagctcaatctaggacgaagagaggagtacgatgttttggacaagagacgtggccgggaccctgagatggggggaaagccgagaaggaagaaccctcaggaaggcctgtacaatgaactgcagaaagataagatggcggaggcctacagtgagattgggatgaaaggcgagcgccggaggggcaaggggcacgatggcctttaccagggtctcagtacagccaccaaggacacctacgacgcccttcacatgcaggccctgccccctcgctaa

SEQ ID NO: 279 - DNA, 1101 bp, Artificial Sequence
  Synthetic Construct
atggctctgcccgtcaccgctctgctgctgcctctggctctgctgctgcacgctgctcgccctgatgtgcagctggtggagtctgggggaggattggtgcaggctgggggctctctgagactctcctgtgcagcctctggaggcaccttaagtaagaataccgtggcttgggtccgccaggctccagggaaggagcgtgggtttgtaacgtctattacctgtgatggtcgtacgacatactatgcgaactccgtgaagggccgattccccatctccagagacaacgccgagaacacagtgtatctgcaaatgaacagcctgaaacctgaggatacggccggttatgtctgtgcagacttagggaagtggcctgcgggttcggcggactactggggccaggggacccacgtcaccgtctcctccactagtaccacgacgccagcgccgcgaccaccaacaccggcgcccaccatcgcgtcgcagcccctgtccctgcgcccagaggcgtgccggccagcggcggggggcgcagtgcacacgagggggctggacttcgcctgtgatatctacatctgggcgcccttggccgggacttgtggggtccttctcctgtcactggttatcaccctttactgcaaacggggcagaaagaaactcctgtatatattcaaacaaccatttatgagaccagtacaaactactcaagaggaagatggctgtagctgccgatttccagaagaagaagaaggaggatgtgaactgagagtgaagttcagcaggagcgcagacgcccccgcgtaccagcagggccagaaccagctctataacgagctcaatctaggacgaagagaggagtacgatgttttggacaagagacgtggccgggaccctgagatggggggaaagccgagaaggaagaaccctcaggaaggcctgtacaatgaactgcagaaagataagatggcggaggcctacagtgagattgggatgaaaggcgagcgccggaggggcaaggggcacgatggcctttaccagggtctcagtacagccaccaaggacacctacgacgcccttcacatgcaggccctgccccctcgctaa

SEQ ID NO: 280 - DNA, 1104 bp, Artificial Sequence
  Synthetic Construct
atggctctgcccgtcaccgctctgctgctgcctctggctctgctgctgcacgctgctcgccctcaggtaaagctggaggagtctgggggaggcttggtgcagcctggggggtctctgagactctcctgtacagcctcggaattcacattcagtgactactggatgcattgggtccgtcaggctccggggaaggggctcgagtgggtcgcatctatagatactagtggacagaccacatactatgcagactccctgaagggccgattcaccatctccagagacaacgccaagagcacgttgtatctgcaaatgaacagtctgaaatctgaagacacgggcgtgtatttctgtgcaaaacgatataggggtggtacctggtatggcatggccaactggggcaaagggacccaggtcaccgtctcctcaactagtaccacgacgccagcgccgcgaccaccaacaccggcgcccaccatcgcgtcgcagcccctgtccctgcgcccagaggcgtgccggccagcggcggggggcgcagtgcacacgagggggctggacttcgcctgtgatatctacatctgggcgcccttggccgggacttgtggggtccttctcctgtcactggttatcaccctttactgcaaacggggcagaaagaaactcctgtatatattcaaacaaccatttatgagaccagtacaaactactcaagaggaagatggctgtagctgccgatttccagaagaagaagaaggaggatgtgaactgagagtgaagttcagcaggagcgcagacgcccccgcgtaccagcagggccagaaccagctctataacgagctcaatctaggacgaagagaggagtacgatgttttggacaagagacgtggccgggaccctgagatggggggaaagccgagaaggaagaaccctcaggaaggcctgtacaatgaactgcagaaagataagatggcggaggcctacagtgagattgggatgaaaggcgagcgccggaggggcaaggggcacgatggcctttaccagggtctcagtacagccaccaaggacacctacgacgcccttcacatgcaggccctgccccctcgctaa

SEQ ID NO: 281 - DNA, 1101 bp, Artificial Sequence
  Synthetic Construct
atggctctgcccgtcaccgctctgctgctgcctctggctctgctgctgcacgctgctcgccctcaggtgcagctggtggagtctgggggaggattggtgcaggctgggggctctctgagactctcctgtgcagcctctggacgcaccttaagtagtaataccatggcttggttccgccaggctccagggaaggagcgtgagtttgtagcgtctactacctggaatggtcgtagcacatactatgcagactccgtgaagggccgattcaccatctccagagacaacgccaagaacacgatgtatctgcaaatgaacagcctgaaacctgaggatacggccgtttatgtctgtgcagacttagggaaatggcctgcgggcccggcggactactggggccaggggacccaggtcaccgtctcctcaactagtaccacgacgccagcgccgcgaccaccaacaccggcgcccaccatcgcgtcgcagcccctgtccctgcgcccagaggcgtgccggccagcggcggggggcgcagtgcacacgagggggctggacttcgcctgtgatatctacatctgggcgcccttggccgggacttgtggggtccttctcctgtcactggttatcaccctttactgcaaacggggcagaaagaaactcctgtatatattcaaacaaccatttatgagaccagtacaaactactcaagaggaagatggctgtagctgccgatttccagaagaagaagaaggaggatgtgaactgagagtgaagttcagcaggagcgcagacgcccccgcgtaccagcagggccagaaccagctctataacgagctcaatctaggacgaagagaggagtacgatgttttggacaagagacgtggccgggaccctgagatggggggaaagccgagaaggaagaaccctcaggaaggcctgtacaatgaactgcagaaagataagatggcggaggcctacagtgagattgggatgaaaggcgagcgccggaggggcaaggggcacgatggcctttaccagggtctcagtacagccaccaaggacacctacgacgcccttcacatgcaggccctgccccctcgctaa

SEQ ID NO: 282 - DNA, 1089 bp, Artificial Sequence
  Synthetic Construct
atggctctgcccgtcaccgctctgctgctgcctctggctctgctgctgcacgctgctcgccctcaggtgcagctggtggagtctgggggaggattggtgcaggctgggggctctctgagactctcctgtgcagcctctggacgcaccttcaccatggggtggttccgtcaggctccagggaagcagcgcgaattggtcgcagatattagtggtggtcgcacaaactatgcagattccgtgaagggacgattcaccatctccagagacaacgccaagaacacggtatatctgcaaatgaacagcctgaaacctgaggacacggccgtttattactgtgcagcagaccggaaatcagtaatgtctattcggcccgactactggggccaggggacccaggtcaccgtctcctcaactagtaccacgacgccagcgccgcgaccaccaacaccggcgcccaccatcgcgtcgcagcccctgtccctgcgcccagaggcgtgccggccagcggcggggggcgcagtgcacacgagggggctggacttcgcctgtgatatctacatctgggcgcccttggccgggacttgtggggtccttctcctgtcactggttatcaccctttactgcaaacggggcagaaagaaactcctgtatatattcaaacaaccatttatgagaccagtacaaactactcaagaggaagatggctgtagctgccgatttccagaagaagaagaaggaggatgtgaactgagagtgaagttcagcaggagcgcagacgcccccgcgtaccagcagggccagaaccagctctataacgagctcaatctaggacgaagagaggagtacgatgttttggacaagagacgtggccgggaccctgagatggggggaaagccgagaaggaagaaccctcaggaaggcctgtacaatgaactgcagaaagataagatggcggaggcctacagtgagattgggatgaaaggcgagcgccggaggggcaaggggcacgatggcctttaccagggtctcagtacagccaccaaggacacctacgacgcccttcacatgcaggccctgccccctcgctaa

SEQ ID NO: 283 - DNA, 1053 bp, Artificial Sequence
  Synthetic Construct
atggctctgcccgtcaccgctctgctgctgcctctggctctgctgctgcacgctgctcgccctcaggtgcagctggtggagtctgggggaggcttggtgcaggctggggcctctctgagactctcctgtgcagcctctggacgcaccttcaccgtggcagctattagtttgagtcctactttagcatattatgcagagtccgtgaagggccgattcaccatcagccgagacaacgccaagaacacggtggttttgcaaatgaacagcctgaaacctgaggacacggccctttattactgtgcagcagaccggaaatcagtaatgtctattcggcccgactactggggccaggggacccaggtcaccgtctcctcaactagtaccacgacgccagcgccgcgaccaccaacaccggcgcccaccatcgcgtcgcagcccctgtccctgcgcccagaggcgtgccggccagcggcggggggcgcagtgcacacgagggggctggacttcgcctgtgatatctacatctgggcgcccttggccgggacttgtggggtccttctcctgtcactggttatcaccctttactgcaaacggggcagaaagaaactcctgtatatattcaaacaaccatttatgagaccagtacaaactactcaagaggaagatggctgtagctgccgatttccagaagaagaagaaggaggatgtgaactgagagtgaagttcagcaggagcgcagacgcccccgcgtaccagcagggccagaaccagctctataacgagctcaatctaggacgaagagaggagtacgatgttttggacaagagacgtggccgggaccctgagatggggggaaagccgagaaggaagaaccctcaggaaggcctgtacaatgaactgcagaaagataagatggcggaggcctacagtgagattgggatgaaaggcgagcgccggaggggcaaggggcacgatggcctttaccagggtctcagtacagccaccaaggacacctacgacgcccttcacatgcaggccctgccccctcgctaa

SEQ ID NO: 284 - DNA, 1116 bp, Artificial Sequence
  Synthetic Construct
atggctctgcccgtcaccgctctgctgctgcctctggctctgctgctgcacgctgctcgccctgatgtgcagctggtggagtctgggggaggattggagcaggctgggggctctctgagactctcctgtgcagcctctggaggcaccttaagtaaaaataccgtggcttggttccgccaggctccagggaaggagcgtgggtttgtagcgtctattacctgggatggtcgtacgacatactatgcagactccgtgaagggccgattcaccatctccagagacaacgccaagaacacagtgtatctgcaaatgaacagcctgaaacctgaggatacggccgtttattactgtgcgtcgacggcatcgtgccacctcttcggattggggtccggggcctttgtgtcctggggccgggggacccaggtcaccgtctcctcaactagtaccacgacgccagcgccgcgaccaccaacaccggcgcccaccatcgcgtcgcagcccctgtccctgcgcccagaggcgtgccggccagcggcggggggcgcagtgcacacgagggggctggacttcgcctgtgatatctacatctgggcgcccttggccgggacttgtggggtccttctcctgtcactggttatcaccctttactgcaaacggggcagaaagaaactcctgtatatattcaaacaaccatttatgagaccagtacaaactactcaagaggaagatggctgtagctgccgatttccagaagaagaagaaggaggatgtgaactgagagtgaagttcagcaggagcgcagacgcccccgcgtaccagcagggccagaaccagctctataacgagctcaatctaggacgaagagaggagtacgatgttttggacaagagacgtggccgggaccctgagatggggggaaagccgagaaggaagaaccctcaggaaggcctgtacaatgaactgcagaaagataagatggcggaggcctacagtgagattgggatgaaaggcgagcgccggaggggcaaggggcacgatggcctttaccagggtctcagtacagccaccaaggacacctacgacgcccttcacatgcaggccctgccccctcgctaa

SEQ ID NO: 285 - DNA, 1089 bp, Artificial Sequence
  Synthetic Construct
atggctctgcccgtcaccgctctgctgctgcctctggctctgctgctgcacgctgctcgccctgcggtgcagctggtggagtctgggggaggattggtgcaggctgggggctctctgagactctcctgtgcagcctctggacgcaccttcaccatggggtggttccatcaggctccagggaaggagcgtgagtttgtagcagctattagtttgagtcctactttagcatattatgcagagtccgtgaagggccgattcaccatcagccgagacaacgccaagaacacggtggttttgcaaatgaacagcctgaaacctgaggacacggccctttattactgtgcagcatccaaggatagatattcggaatatgagtactggggccaggggacccaggtcaccgtctcctcaactagtaccacgacgccagcgccgcgaccaccaacaccggcgcccaccatcgcgtcgcagcccctgtccctgcgcccagaggcgtgccggccagcggcggggggcgcagtgcacacgagggggctggacttcgcctgtgatatctacatctgggcgcccttggccgggacttgtggggtccttctcctgtcactggttatcaccctttactgcaaacggggcagaaagaaactcctgtatatattcaaacaaccatttatgagaccagtacaaactactcaagaggaagatggctgtagctgccgatttccagaagaagaagaaggaggatgtgaactgagagtgaagttcagcaggagcgcagacgcccccgcgtaccagcagggccagaaccagctctataacgagctcaatctaggacgaagagaggagtacgatgttttggacaagagacgtggccgggaccctgagatggggggaaagccgagaaggaagaaccctcaggaaggcctgtacaatgaactgcagaaagataagatggcggaggcctacagtgagattgggatgaaaggcgagcgccggaggggcaaggggcacgatggcctttaccagggtctcagtacagccaccaaggacacctacgacgcccttcacatgcaggccctgccccctcgctaa

SEQ ID NO: 286 - DNA, 1083 bp, Artificial Sequence
  Synthetic Construct
atggctctgcccgtcaccgctctgctgctgcctctggctctgctgctgcacgctgctcgccctcaggtaaagctggaggagtctgggggaggattggtgcaggctgggggctctctgagactctcctgtgcagcctctggacgcaccttcaccatggggtggttccgtcaggctccagggaaggagcgtgagtttgtagcagctattagtttgagtcctactttagcatattatgcagagtccgtgaagggccgattcaccatcagccgagacaacgccaagaacacggtggttttgcaaatgaacagcctgaaacctgaggacacggccctttattactgtgcaaaaaaaaacggggggcctgtggactactggggcaaagggacccaggtcaccgtctcctcaactagtaccacgacgccagcgccgcgaccaccaacaccggcgcccaccatcgcgtcgcagcccctgtccctgcgcccagaggcgtgccggccagcggcggggggcgcagtgcacacgagggggctggacttcgcctgtgatatctacatctgggcgcccttggccgggacttgtggggtccttctcctgtcactggttatcaccctttactgcaaacggggcagaaagaaactcctgtatatattcaaacaaccatttatgagaccagtacaaactactcaagaggaagatggctgtagctgccgatttccagaagaagaagaaggaggatgtgaactgagagtgaagttcagcaggagcgcagacgcccccgcgtaccagcagggccagaaccagctctataacgagctcaatctaggacgaagagaggagtacgatgttttggacaagagacgtggccgggaccctgagatggggggaaagccgagaaggaagaaccctcaggaaggcctgtacaatgaactgcagaaagataagatggcggaggcctacagtgagattgggatgaaaggcgagcgccggaggggcaaggggcacgatggcctttaccagggtctcagtacagccaccaaggacacctacgacgcccttcacatgcaggccctgccccctcgctaa

SEQ ID NO: 287 - DNA, 1098 bp, Artificial Sequence
  Synthetic Construct
atggctctgcccgtcaccgctctgctgctgcctctggctctgctgctgcacgctgctcgccctgatgtgcagctggtggagtctgggggaggcttggtgcagcctggggggtctctgagactctcctgtgcagcctctggacggaccttcagtagcattgtcatgggctggttccgccaggctccagggaaggagcgtgagtttgtaggagcgattatgtggaatgatggtattacatacttgcaagactccgtgaagggccgatttaccatcttcagagacaacgccaagaacacggtgtatctgcaaatgaacagcctgaaacttgaggatacggccgtttattactgtgcagcatccaagggtagatactcggaatatgagtactggggccaggggacccaggtcaccgtctcctcaactagtaccacgacgccagcgccgcgaccaccaacaccggcgcccaccatcgcgtcgcagcccctgtccctgcgcccagaggcgtgccggccagcggcggggggcgcagtgcacacgagggggctggacttcgcctgtgatatctacatctgggcgcccttggccgggacttgtggggtccttctcctgtcactggttatcaccctttactgcaaacggggcagaaagaaactcctgtatatattcaaacaaccatttatgagaccagtacaaactactcaagaggaagatggctgtagctgccgatttccagaagaagaagaaggaggatgtgaactgagagtgaagttcagcaggagcgcagacgcccccgcgtaccagcagggccagaaccagctctataacgagctcaatctaggacgaagagaggagtacgatgttttggacaagagacgtggccgggaccctgagatggggggaaagccgagaaggaagaaccctcaggaaggcctgtacaatgaactgcagaaagataagatggcggaggcctacagtgagattgggatgaaaggcgagcgccggaggggcaaggggcacgatggcctttaccagggtctcagtacagccaccaaggacacctacgacgcccttcacatgcaggccctgccccctcgctaa

SEQ ID NO: 288 - DNA, 1095 bp, Artificial Sequence
  Synthetic Construct
atggctctgcccgtcaccgctctgctgctgcctctggctctgctgctgcacgctgctcgccctcaggtaaagctggaggaatctgggggaagattggtgcaggctgggggctctctgaaactctcctgggcagcctctggacgcaccttcaccatggggtggttccgtcaggctccagggaaggaacgtgagtttgtaacagctattaatttgagtcctactttaacatattatgcagaatccgtgaagggccgattccccatcagccgaaacaacgcccagaacacggtggttttgcaaatgaacagcctgaaacctgaggacacggccctttattactgtgcagcagaacggaaatcagtaatggctattccgcccgactactggggccaggggacccaggtcaccgtctcctcaactagtaccacgacgccagcgccgcgaccaccaacaccggcgcccaccatcgcgtcgcagcccctgtccctgcgcccagaggcgtgccggccagcggcggggggcgcagtgcacacgagggggctggacttcgcctgtgatatctacatctgggcgcccttggccgggacttgtggggtccttctcctgtcactggttatcaccctttactgcaaacggggcagaaagaaactcctgtatatattcaaacaaccatttatgagaccagtacaaactactcaagaggaagatggctgtagctgccgatttccagaagaagaagaaggaggatgtgaactgagagtgaagttcagcaggagcgcagacgcccccgcgtaccagcagggccagaaccagctctataacgagctcaatctaggacgaagagaggagtacgatgttttggacaagagacgtggccgggaccctgagatggggggaaagccgagaaggaagaaccctcaggaaggcctgtacaatgaactgcagaaagataagatggcggaggcctacagtgagattgggatgaaaggcgagcgccggaggggcaaggggcacgatggcctttaccagggtctcagtacagccaccaaggacacctacgacgcccttcacatgcaggccctgccccctcgctaa

SEQ ID NO: 289 - DNA, 1095 bp, Artificial Sequence
  Synthetic Construct
atggctctgcccgtcaccgctctgctgctgcctctggctctgctgctgcacgctgctcgccctgaggtgcagctggtggagtctgggggaggattggtgcaggctgggggctctctgagactctcctgtgcagcctctggacgcaccttcaccatgggggggttccgtcgggttcctcgggatgagcgggagtttgtagcatctattactttgattcctacttttccttattatgcatattccgtgaagggccgattcgccctcttccgagacaaccccaacaacaccgtgattttgctgatgatcagcctgaaacctgaggacccggacctttattactgtgcttcataccggaaatacctaatgtctattctgcccgactactggggccaggggacccagggcaccgtctcctccactagtaccacgacgccagcgccgcgaccaccaacaccggcgcccaccatcgcgtcgcagcccctgtccctgcgcccagaggcgtgccggccagcggcggggggcgcagtgcacacgagggggctggacttcgcctgtgatatctacatctgggcgcccttggccgggacttgtggggtccttctcctgtcactggttatcaccctttactgcaaacggggcagaaagaaactcctgtatatattcaaacaaccatttatgagaccagtacaaactactcaagaggaagatggctgtagctgccgatttccagaagaagaagaaggaggatgtgaactgagagtgaagttcagcaggagcgcagacgcccccgcgtaccagcagggccagaaccagctctataacgagctcaatctaggacgaagagaggagtacgatgttttggacaagagacgtggccgggaccctgagatggggggaaagccgagaaggaagaaccctcaggaaggcctgtacaatgaactgcagaaagataagatggcggaggcctacagtgagattgggatgaaaggcgagcgccggaggggcaaggggcacgatggcctttaccagggtctcagtacagccaccaaggacacctacgacgcccttcacatgcaggccctgccccctcgctaa

SEQ ID NO: 290 - DNA, 1113 bp, Artificial Sequence
  Synthetic Construct
atggctctgcccgtcaccgctctgctgctgcctctggctctgctgctgcacgctgctcgccctcaggtaaagctggaggagtctgggggaggattggtgcaggctgggggctctctgagactctcctgtgcagcctctggacgcaccttcaccatggggtggttccgtcaggctccagggaaggagcgtgagtttgtagcagctattagtttgagtcctactttagcatattatgcagagtccgtgaagggccgattcaccatcagccgagacaacgccaagaacacggtggatctgcaaatgaacagcctgaaacctgaggacacggccgtctatttctgtgcagcaaatcggaactcccaacgggtaattgcggcactgtcctggattggcatgaactactggggcgaatggacccaggtcaccgtctcctccactagtaccacgacgccagcgccgcgaccaccaacaccggcgcccaccatcgcgtcgcagcccctgtccctgcgcccagaggcgtgccggccagcggcggggggcgcagtgcacacgagggggctggacttcgcctgtgatatctacatctgggcgcccttggccgggacttgtggggtccttctcctgtcactggttatcaccctttactgcaaacggggcagaaagaaactcctgtatatattcaaacaaccatttatgagaccagtacaaactactcaagaggaagatggctgtagctgccgatttccagaagaagaagaaggaggatgtgaactgagagtgaagttcagcaggagcgcagacgcccccgcgtaccagcagggccagaaccagctctataacgagctcaatctaggacgaagagaggagtacgatgttttggacaagagacgtggccgggaccctgagatggggggaaagccgagaaggaagaaccctcaggaaggcctgtacaatgaactgcagaaagataagatggcggaggcctacagtgagattgggatgaaaggcgagcgccggaggggcaaggggcacgatggcctttaccagggtctcagtacagccaccaaggacacctacgacgcccttcacatgcaggccctgccccctcgctaa

SEQ ID NO: 291 - DNA, 1089 bp, Artificial Sequence
  Synthetic Construct
atggctctgcccgtcaccgctctgctgctgcctctggctctgctgctgcacgctgctcgccctcaggtgcagctggtggagtctgggggaggattggtgcaggctgggggctctctgagactctcctgtgcagcctctggacgcaccttcaccatggggtggttccgtcaggctccagggaaggagcgtgagtttgtagcagctattagtttgagtcctactttagcatattatgcagagtccgtgaagggccgattcaccatctccagagacaacgccaagaagacgctgtatctgcgaatgaatagcctgaaacctgaggacacggccgtttactactgtgcagcacgtcggatcgacgcagctgactttgattcctgggggcaggggacccaggtcaccgtctcctcaactagtaccacgacgccagcgccgcgaccaccaacaccggcgcccaccatcgcgtcgcagcccctgtccctgcgcccagaggcgtgccggccagcggcggggggcgcagtgcacacgagggggctggacttcgcctgtgatatctacatctgggcgcccttggccgggacttgtggggtccttctcctgtcactggttatcaccctttactgcaaacggggcagaaagaaactcctgtatatattcaaacaaccatttatgagaccagtacaaactactcaagaggaagatggctgtagctgccgatttccagaagaagaagaaggaggatgtgaactgagagtgaagttcagcaggagcgcagacgcccccgcgtaccagcagggccagaaccagctctataacgagctcaatctaggacgaagagaggagtacgatgttttggacaagagacgtggccgggaccctgagatggggggaaagccgagaaggaagaaccctcaggaaggcctgtacaatgaactgcagaaagataagatggcggaggcctacagtgagattgggatgaaaggcgagcgccggaggggcaaggggcacgatggcctttaccagggtctcagtacagccaccaaggacacctacgacgcccttcacatgcaggccctgccccctcgctaa

SEQ ID NO: 292 - DNA, 1089 bp, Artificial Sequence
  Synthetic Construct
atggctctgcccgtcaccgctctgctgctgcctctggctctgctgctgcacgctgctcgccctcaggtaaagctggaggagtctgggggaggattggtgcaggctgggggctctctgagactctcctgtgcagcctctggacgcaccttcaccatggggtggttccgtcgggctccagggaaggagcgtgagtctgttgcagttattggctggagagatattaacgcaagctatgcagactccgtgaagggccgattcgccatctccagagacaacgccaagaagacgctgtatctgcagatgaatagcctgaaacctgaggacacggccgtttactactgtgcagcacgtcggatcgacgcaactgactttgattcctgggggcaggggacccaggtcaccgtctcctcaactagtaccacgacgccagcgccgcgaccaccaacaccggcgcccaccatcgcgtcgcagcccctgtccctgcgcccagaggcgtgccggccagcggcggggggcgcagtgcacacgagggggctggacttcgcctgtgatatctacatctgggcgcccttggccgggacttgtggggtccttctcctgtcactggttatcaccctttactgcaaacggggcagaaagaaactcctgtatatattcaaacaaccatttatgagaccagtacaaactactcaagaggaagatggctgtagctgccgatttccagaagaagaagaaggaggatgtgaactgagagtgaagttcagcaggagcgcagacgcccccgcgtaccagcagggccagaaccagctctataacgagctcaatctaggacgaagagaggagtacgatgttttggacaagagacgtggccgggaccctgagatggggggaaagccgagaaggaagaaccctcaggaaggcctgtacaatgaactgcagaaagataagatggcggaggcctacagtgagattgggatgaaaggcgagcgccggaggggcaaggggcacgatggcctttaccagggtctcagtacagccaccaaggacacctacgacgcccttcacatgcaggccctgccccctcgctaa

SEQ ID NO: 293 - DNA, 1098 bp, Artificial Sequence
  Synthetic Construct
atggctctgcccgtcaccgctctgctgctgcctctggctctgctgctgcacgctgctcgccctcaggtaaagctggaggagtctgggggaggattggtgcagactgggggctctctgagactctcctgtgcagcctctgaacacaccttcagtaaccatgtcatgggctggttccgccaggctccagggaaggagcgtgagtctgttgcagttattggctggagagatattagcacaagctatgcagactccgtgaagggccgattcaccatctccagagacaacgccaagaagacgctgtatctgcaaatgaatagcctgaaacctgaggacacggccgtttactactgtgcagcacgtcggatcgacgcagctgactttgattcccgggggcaggggacccaggtcaccgtctcctcaactagtaccacgacgccagcgccgcgaccaccaacaccggcgcccaccatcgcgtcgcagcccctgtccctgcgcccagaggcgtgccggccagcggcggggggcgcagtgcacacgagggggctggacttcgcctgtgatatctacatctgggcgcccttggccgggacttgtggggtccttctcctgtcactggttatcaccctttactgcaaacggggcagaaagaaactcctgtatatattcaaacaaccatttatgagaccagtacaaactactcaagaggaagatggctgtagctgccgatttccagaagaagaagaaggaggatgtgaactgagagtgaagttcagcaggagcgcagacgcccccgcgtaccagcagggccagaaccagctctataacgagctcaatctaggacgaagagaggagtacgatgttttggacaagagacgtggccgggaccctgagatggggggaaagccgagaaggaagaaccctcaggaaggcctgtacaatgaactgcagaaagataagatggcggaggcctacagtgagattgggatgaaaggcgagcgccggaggggcaaggggcacgatggcctttaccagggtctcagtacagccaccaaggacacctacgacgcccttcacatgcaggccctgccccctcgctaa

SEQ ID NO: 294 - DNA, 1110 bp, Artificial Sequence
  Synthetic Construct
atggctctgcccgtcaccgctctgctgctgcctctggctctgctgctgcacgctgctcgccctgccgtgcagctggtggattctgggggaggattggtgcaggctgggggctctctgagaatttcctgtgcagtctctggacgcacctccagtaactatatattggcctggttccgtcaggctccaggaaaagagcgtgactttgtagcacatattagccggagtggtggtaagtccggctatggagactccgtgaagggccgattcaccatctccagagacaacgccgagaacacggtcagggtgtatctgcaaatgaacagtctgaaacctggggacacggccgtctattactgtaatcgccccctctggtacggaagtcccacgttgattgactactggggccaggggacccaggtcaccgtctcctcaactagtaccacgacgccagcgccgcgaccaccaacaccggcgcccaccatcgcgtcgcagcccctgtccctgcgcccagaggcgtgccggccagcggcggggggcgcagtgcacacgagggggctggacttcgcctgtgatatctacatctgggcgcccttggccgggacttgtggggtccttctcctgtcactggttatcaccctttactgcaaacggggcagaaagaaactcctgtatatattcaaacaaccatttatgagaccagtacaaactactcaagaggaagatggctgtagctgccgatttccagaagaagaagaaggaggatgtgaactgagagtgaagttcagcaggagcgcagacgcccccgcgtaccagcagggccagaaccagctctataacgagctcaatctaggacgaagagaggagtacgatgttttggacaagagacgtggccgggaccctgagatggggggaaagccgagaaggaagaaccctcaggaaggcctgtacaatgaactgcagaaagataagatggcggaggcctacagtgagattgggatgaaaggcgagcgccggaggggcaaggggcacgatggcctttaccagggtctcagtacagccaccaaggacacctacgacgcccttcacatgcaggccctgccccctcgctaa

SEQ ID NO: 295 - DNA, 1095 bp, Artificial Sequence
  Synthetic Construct
atggctctgcccgtcaccgctctgctgctgcctctggctctgctgctgcacgctgctcgccctgcggtgcagctggtggagtctgggggaggcttggtgcagcctggggggtctctgagactctcctgtgcagcctctggacgcaccttcaccatggggtggttccgtcaggctccagggaaggagcgtgagtttgtagcagctattagtttgagtcctactttagcatattatgcagagtccgtgaagggccgattcaccatcagccgagacaacgccaagaacacggtggttttgcaaatgaacagcctgaaacctgaggacacggccctttattactgtgcagcagaccggaaatcagtaatgtctattcggcccgactactggggccaggggacccaggtcaccgtctcctcaactagtaccacgacgccagcgccgcgaccaccaacaccggcgcccaccatcgcgtcgcagcccctgtccctgcgcccagaggcgtgccggccagcggcggggggcgcagtgcacacgagggggctggacttcgcctgtgatatctacatctgggcgcccttggccgggacttgtggggtccttctcctgtcactggttatcaccctttactgcaaacggggcagaaagaaactcctgtatatattcaaacaaccatttatgagaccagtacaaactactcaagaggaagatggctgtagctgccgatttccagaagaagaagaaggaggatgtgaactgagagtgaagttcagcaggagcgcagacgcccccgcgtaccagcagggccagaaccagctctataacgagctcaatctaggacgaagagaggagtacgatgttttggacaagagacgtggccgggaccctgagatggggggaaagccgagaaggaagaaccctcaggaaggcctgtacaatgaactgcagaaagataagatggcggaggcctacagtgagattgggatgaaaggcgagcgccggaggggcaaggggcacgatggcctttaccagggtctcagtacagccaccaaggacacctacgacgcccttcacatgcaggccctgccccctcgctaa

SEQ ID NO: 296 - DNA, 1095 bp, Artificial Sequence
  Synthetic Construct
atggctctgcccgtcaccgctctgctgctgcctctggctctgctgctgcacgctgctcgccctgcggtgcagctggtggagtctgggggaggattggtgcaggctgggggctctctgagactctcctgtgcagcctctggacgcaccttcaccatggggtggttccgtcaggctccagggaaggagcgtgagtttgtagcagctattagtttgagtcctactttagcatattatgcagagtccgtgaagggccgattcaccatcagccgagacaacgccaagaacacggtggttttgcaaatgaacagcctgaaacctgaggacacggccctttattactgtgcagcagaccggaaatcagtaatgtctattcggcccgactactggggccaggggacccaggtcaccgtctcctcaactagtaccacgacgccagcgccgcgaccaccaacaccggcgcccaccatcgcgtcgcagcccctgtccctgcgcccagaggcgtgccggccagcggcggggggcgcagtgcacacgagggggctggacttcgcctgtgatatctacatctgggcgcccttggccgggacttgtggggtccttctcctgtcactggttatcaccctttactgcaaacggggcagaaagaaactcctgtatatattcaaacaaccatttatgagaccagtacaaactactcaagaggaagatggctgtagctgccgatttccagaagaagaagaaggaggatgtgaactgagagtgaagttcagcaggagcgcagacgcccccgcgtaccagcagggccagaaccagctctataacgagctcaatctaggacgaagagaggagtacgatgttttggacaagagacgtggccgggaccctgagatggggggaaagccgagaaggaagaaccctcaggaaggcctgtacaatgaactgcagaaagataagatggcggaggcctacagtgagattgggatgaaaggcgagcgccggaggggcaaggggcacgatggcctttaccagggtctcagtacagccaccaaggacacctacgacgcccttcacatgcaggccctgccccctcgctaa

SEQ ID NO: 297 - DNA, 1104 bp, Artificial Sequence
  Synthetic Construct
atggctctgcccgtcaccgctctgctgctgcctctggctctgctgctgcacgctgctcgccctgatgtgcagctggtggagtctgggggaggatcggtgcagactgggggctctctgagactctcctgtacagcctctggacgcaccctcaataactttgtcatgggctggttccgtcaggctccagggaaggagcgtgagtttgtagcagctattagtttgagtcctactttagcatattatgtagagtccgtgaagggccgattcaccatcagccgagacaacgccaagaacacggtggttttgcaaatgaacagcctgaaacctgaggacacggccctttattactgtgcagcagaccggaaatcagtaatgtctattcggcccgactactggggccaggggacccaggtcaccgtctcctcaactagtaccacgacgccagcgccgcgaccaccaacaccggcgcccaccatcgcgtcgcagcccctgtccctgcgcccagaggcgtgccggccagcggcggggggcgcagtgcacacgagggggctggacttcgcctgtgatatctacatctgggcgcccttggccgggacttgtggggtccttctcctgtcactggttatcaccctttactgcaaacggggcagaaagaaactcctgtatatattcaaacaaccatttatgagaccagtacaaactactcaagaggaagatggctgtagctgccgatttccagaagaagaagaaggaggatgtgaactgagagtgaagttcagcaggagcgcagacgcccccgcgtaccagcagggccagaaccagctctataacgagctcaatctaggacgaagagaggagtacgatgttttggacaagagacgtggccgggaccctgagatggggggaaagccgagaaggaagaaccctcaggaaggcctgtacaatgaactgcagaaagataagatggcggaggcctacagtgagattgggatgaaaggcgagcgccggaggggcaaggggcacgatggcctttaccagggtctcagtacagccaccaaggacacctacgacgcccttcacatgcaggccctgccccctcgctaa

SEQ ID NO: 298 - protein, 495 aa, Artificial Sequence
  Synthetic Construct
MALPVTALLLPLALLLHAARPQVQLVESGGGLVQPGGSLRLSCEASGFTLDYYAIGWFRQAPGKEREGVICISRSDGSTYYADSVKGRFTISRDNAKKTVYLQMISLKPEDTAAYYCAAGADCSGYLRDYEFRGQGTQVTVSSGGGGSQVQLVESGGGLVQPGGSLRLSCEASGFTLDYYAIGWFRQAPGKEREGVICISRSDGSTYYADSVKGRFTISRDNAKKTVYLQMISLKPEDTAAYYCAAGADCSGYLRDYEFRGQGTQVTVSSTSTTTPAPRPPTPAPTIASQPLSLRPEACRPAAGGAVHTRGLDFACDIYIWAPLAGTCGVLLLSLVITLYCKRGRKKLLYIFKQPFMRPVQTTQEEDGCSCRFPEEEEGGCELRVKFSRSADAPAYQQGQNQLYNELNLGRREEYDVLDKRRGRDPEMGGKPRRKNPQEGLYNELQKDKMAEAYSEIGMKGERRRGKGHDGLYQGLSTATKDTYDALHMQALPPR

SEQ ID NO: 299 - protein, 622 aa, Artificial Sequence
  Synthetic Construct
MALPVTALLLPLALLLHAARPQVQLVESGGGLVQPGGSLRLSCEASGFTLDYYAIGWFRQAPGKEREGVICISRSDGSTYYADSVKGRFTISRDNAKKTVYLQMISLKPEDTAAYYCAAGADCSGYLRDYEFRGQGTQVTVSSGGGGSQVQLVESGGGLVQPGGSLRLSCEASGFTLDYYAIGWFRQAPGKEREGVICISRSDGSTYYADSVKGRFTISRDNAKKTVYLQMISLKPEDTAAYYCAAGADCSGYLRDYEFRGQGTQVTVSSGGGGSQVQLVESGGGLVQPGGSLRLSCEASGFTLDYYAIGWFRQAPGKEREGVICISRSDGSTYYADSVKGRFTISRDNAKKTVYLQMISLKPEDTAAYYCAAGADCSGYLRDYEFRGQGTQVTVSSTSTTTPAPRPPTPAPTIASQPLSLRPEACRPAAGGAVHTRGLDFACDIYIWAPLAGTCGVLLLSLVITLYCKRGRKKLLYIFKQPFMRPVQTTQEEDGCSCRFPEEEEGGCELRVKFSRSADAPAYQQGQNQLYNELNLGRREEYDVLDKRRGRDPEMGGKPRRKNPQEGLYNELQKDKMAEAYSEIGMKGERRRGKGHDGLYQGLSTATKDTYDALHMQALPPR

SEQ ID NO: 300 - protein, 488 aa, Artificial Sequence
  Synthetic Construct
MALPVTALLLPLALLLHAARPQVKLEESGGGLVQAGRSLRLSCAASEHTFSSHVMGWFRQAPGKERESVAVIGWRDISTSYADSVKGRFTISRDNAKKTLYLQMNSLKPEDTAVYYCAARRIDAADFDSWGQGTQVTVSSGGGGSEVQLVESGGGLVQAGGSLRLSCAASGRTFTMGWFRQAPGKEREFVAAISLSPTLAYYAESVKGRFTISRDNAKNTVVLQMNSLKPEDTALYYCAADRKSVMSIRPDYWGQGTQVTVSSTSTTTPAPRPPTPAPTIASQPLSLRPEACRPAAGGAVHTRGLDFACDIYIWAPLAGTCGVLLLSLVITLYCKRGRKKLLYIFKQPFMRPVQTTQEEDGCSCRFPEEEEGGCELRVKFSRSADAPAYQQGQNQLYNELNLGRREEYDVLDKRRGRDPEMGGKPRRKNPQEGLYNELQKDKMAEAYSEIGMKGERRRGKGHDGLYQGLSTATKDTYDALHMQALPPR

SEQ ID NO: 301 - protein, 498 aa, Artificial Sequence
  Synthetic Construct
MALPVTALLLPLALLLHAARPQVKLEESGGGLVQAGRSLRLSCAASEHTFSSHVMGWFRQAPGKERESVAVIGWRDISTSYADSVKGRFTISRDNAKKTLYLQMNSLKPEDTAVYYCAARRIDAADFDSWGQGTQVTVSSGGGGSGGGGSGGGGSEVQLVESGGGLVQAGGSLRLSCAASGRTFTMGWFRQAPGKEREFVAAISLSPTLAYYAESVKGRFTISRDNAKNTVVLQMNSLKPEDTALYYCAADRKSVMSIRPDYWGQGTQVTVSSTSTTTPAPRPPTPAPTIASQPLSLRPEACRPAAGGAVHTRGLDFACDIYIWAPLAGTCGVLLLSLVITLYCKRGRKKLLYIFKQPFMRPVQTTQEEDGCSCRFPEEEEGGCELRVKFSRSADAPAYQQGQNQLYNELNLGRREEYDVLDKRRGRDPEMGGKPRRKNPQEGLYNELQKDKMAEAYSEIGMKGERRRGKGHDGLYQGLSTATKDTYDALHMQALPPR

SEQ ID NO: 302 - protein, 508 aa, Artificial Sequence
  Synthetic Construct
MALPVTALLLPLALLLHAARPQVKLEESGGGLVQAGRSLRLSCAASEHTFSSHVMGWFRQAPGKERESVAVIGWRDISTSYADSVKGRFTISRDNAKKTLYLQMNSLKPEDTAVYYCAARRIDAADFDSWGQGTQVTVSSGGGGSGGGGSGGGGSGGGGSGGGGSEVQLVESGGGLVQAGGSLRLSCAASGRTFTMGWFRQAPGKEREFVAAISLSPTLAYYAESVKGRFTISRDNAKNTVVLQMNSLKPEDTALYYCAADRKSVMSIRPDYWGQGTQVTVSSTSTTTPAPRPPTPAPTIASQPLSLRPEACRPAAGGAVHTRGLDFACDIYIWAPLAGTCGVLLLSLVITLYCKRGRKKLLYIFKQPFMRPVQTTQEEDGCSCRFPEEEEGGCELRVKFSRSADAPAYQQGQNQLYNELNLGRREEYDVLDKRRGRDPEMGGKPRRKNPQEGLYNELQKDKMAEAYSEIGMKGERRRGKGHDGLYQGLSTATKDTYDALHMQALPPR

SEQ ID NO: 303 - protein, 493 aa, Artificial Sequence
  Synthetic Construct
MALPVTALLLPLALLLHAARPEVQLVESGGGLVQAGGSLRLSCAASGRTFTMGWFRQAPGKEREFVAAISLSPTLAYYAESVKGRFTISRDNAKNTVVLQMNSLKPEDTALYYCAADRKSVMSIRPDYWGQGTQVTVSSGGGGSGGGGSQVKLEESGGGLVQAGRSLRLSCAASEHTFSSHVMGWFRQAPGKERESVAVIGWRDISTSYADSVKGRFTISRDNAKKTLYLQMNSLKPEDTAVYYCAARRIDAADFDSWGQGTQVTVSSTSTTTPAPRPPTPAPTIASQPLSLRPEACRPAAGGAVHTRGLDFACDIYIWAPLAGTCGVLLLSLVITLYCKRGRKKLLYIFKQPFMRPVQTTQEEDGCSCRFPEEEEGGCELRVKFSRSADAPAYQQGQNQLYNELNLGRREEYDVLDKRRGRDPEMGGKPRRKNPQEGLYNELQKDKMAEAYSEIGMKGERRRGKGHDGLYQGLSTATKDTYDALHMQALPPR

SEQ ID NO: 304 - protein, 498 aa, Artificial Sequence
  Synthetic Construct
MALPVTALLLPLALLLHAARPEVQLVESGGGLVQAGGSLRLSCAASGRTFTMGWFRQAPGKEREFVAAISLSPTLAYYAESVKGRFTISRDNAKNTVVLQMNSLKPEDTALYYCAADRKSVMSIRPDYWGQGTQVTVSSGGGGSGGGGSGGGGSQVKLEESGGGLVQAGRSLRLSCAASEHTFSSHVMGWFRQAPGKERESVAVIGWRDISTSYADSVKGRFTISRDNAKKTLYLQMNSLKPEDTAVYYCAARRIDAADFDSWGQGTQVTVSSTSTTTPAPRPPTPAPTIASQPLSLRPEACRPAAGGAVHTRGLDFACDIYIWAPLAGTCGVLLLSLVITLYCKRGRKKLLYIFKQPFMRPVQTTQEEDGCSCRFPEEEEGGCELRVKFSRSADAPAYQQGQNQLYNELNLGRREEYDVLDKRRGRDPEMGGKPRRKNPQEGLYNELQKDKMAEAYSEIGMKGERRRGKGHDGLYQGLSTATKDTYDALHMQALPPR

SEQ ID NO: 305 - protein, 503 aa, Artificial Sequence
  Synthetic Construct
MALPVTALLLPLALLLHAARPEVQLVESGGGLVQAGGSLRLSCAASGRTFTMGWFRQAPGKEREFVAAISLSPTLAYYAESVKGRFTISRDNAKNTVVLQMNSLKPEDTALYYCAADRKSVMSIRPDYWGQGTQVTVSSGGGGSGGGGSGGGGSGGGGSQVKLEESGGGLVQAGRSLRLSCAASEHTFSSHVMGWFRQAPGKERESVAVIGWRDISTSYADSVKGRFTISRDNAKKTLYLQMNSLKPEDTAVYYCAARRIDAADFDSWGQGTQVTVSSTSTTTPAPRPPTPAPTIASQPLSLRPEACRPAAGGAVHTRGLDFACDIYIWAPLAGTCGVLLLSLVITLYCKRGRKKLLYIFKQPFMRPVQTTQEEDGCSCRFPEEEEGGCELRVKFSRSADAPAYQQGQNQLYNELNLGRREEYDVLDKRRGRDPEMGGKPRRKNPQEGLYNELQKDKMAEAYSEIGMKGERRRGKGHDGLYQGLSTATKDTYDALHMQALPPR

SEQ ID NO: 306 - protein, 489 aa, Artificial Sequence
  Synthetic Construct
MALPVTALLLPLALLLHAARPQVKLEESGGGLVQAGRSLRLSCAASEHTFSSHVMGWFRQAPGKERESVAVIGWRDISTSYADSVKGRFTISRDNAKKTLYLQMNSLKPEDTAVYYCAARRIDAADFDSWGQGTQVTVSSGGGGSAVQLVESGGGLVQAGDSLRLTCTASGRAFSTYFMAWFRQAPGKEREFVAGIAWSGGSTAYADSVKGRFTISRDNAKNTVYLQMNSLKSEDTAVYYCASRGIEVEEFGAWGQGTQVTVSSTSTTTPAPRPPTPAPTIASQPLSLRPEACRPAAGGAVHTRGLDFACDIYIWAPLAGTCGVLLLSLVITLYCKRGRKKLLYIFKQPFMRPVQTTQEEDGCSCRFPEEEEGGCELRVKFSRSADAPAYQQGQNQLYNELNLGRREEYDVLDKRRGRDPEMGGKPRRKNPQEGLYNELQKDKMAEAYSEIGMKGERRRGKGHDGLYQGLSTATKDTYDALHMQALPPR

SEQ ID NO: 307 - protein, 499 aa, Artificial Sequence
  Synthetic Construct
MALPVTALLLPLALLLHAARPQVKLEESGGGLVQAGRSLRLSCAASEHTFSSHVMGWFRQAPGKERESVAVIGWRDISTSYADSVKGRFTISRDNAKKTLYLQMNSLKPEDTAVYYCAARRIDAADFDSWGQGTQVTVSSGGGGSGGGGSGGGGSAVQLVESGGGLVQAGDSLRLTCTASGRAFSTYFMAWFRQAPGKEREFVAGIAWSGGSTAYADSVKGRFTISRDNAKNTVYLQMNSLKSEDTAVYYCASRGIEVEEFGAWGQGTQVTVSSTSTTTPAPRPPTPAPTIASQPLSLRPEACRPAAGGAVHTRGLDFACDIYIWAPLAGTCGVLLLSLVITLYCKRGRKKLLYIFKQPFMRPVQTTQEEDGCSCRFPEEEEGGCELRVKFSRSADAPAYQQGQNQLYNELNLGRREEYDVLDKRRGRDPEMGGKPRRKNPQEGLYNELQKDKMAEAYSEIGMKGERRRGKGHDGLYQGLSTATKDTYDALHMQALPPR

SEQ ID NO: 308 - protein, 509 aa, Artificial Sequence
  Synthetic Construct
MALPVTALLLPLALLLHAARPQVKLEESGGGLVQAGRSLRLSCAASEHTFSSHVMGWFRQAPGKERESVAVIGWRDISTSYADSVKGRFTISRDNAKKTLYLQMNSLKPEDTAVYYCAARRIDAADFDSWGQGTQVTVSSGGGGSGGGGSGGGGSGGGGSGGGGSAVQLVESGGGLVQAGDSLRLTCTASGRAFSTYFMAWFRQAPGKEREFVAGIAWSGGSTAYADSVKGRFTISRDNAKNTVYLQMNSLKSEDTAVYYCASRGIEVEEFGAWGQGTQVTVSSTSTTTPAPRPPTPAPTIASQPLSLRPEACRPAAGGAVHTRGLDFACDIYIWAPLAGTCGVLLLSLVITLYCKRGRKKLLYIFKQPFMRPVQTTQEEDGCSCRFPEEEEGGCELRVKFSRSADAPAYQQGQNQLYNELNLGRREEYDVLDKRRGRDPEMGGKPRRKNPQEGLYNELQKDKMAEAYSEIGMKGERRRGKGHDGLYQGLSTATKDTYDALHMQALPPR

SEQ ID NO: 309 - protein, 494 aa, Artificial Sequence
  Synthetic Construct
MALPVTALLLPLALLLHAARPAVQLVESGGGLVQAGDSLRLTCTASGRAFSTYFMAWFRQAPGKEREFVAGIAWSGGSTAYADSVKGRFTISRDNAKNTVYLQMNSLKSEDTAVYYCASRGIEVEEFGAWGQGTQVTVSSGGGGSGGGGSQVKLEESGGGLVQAGRSLRLSCAASEHTFSSHVMGWFRQAPGKERESVAVIGWRDISTSYADSVKGRFTISRDNAKKTLYLQMNSLKPEDTAVYYCAARRIDAADFDSWGQGTQVTVSSTSTTTPAPRPPTPAPTIASQPLSLRPEACRPAAGGAVHTRGLDFACDIYIWAPLAGTCGVLLLSLVITLYCKRGRKKLLYIFKQPFMRPVQTTQEEDGCSCRFPEEEEGGCELRVKFSRSADAPAYQQGQNQLYNELNLGRREEYDVLDKRRGRDPEMGGKPRRKNPQEGLYNELQKDKMAEAYSEIGMKGERRRGKGHDGLYQGLSTATKDTYDALHMQALPPR

SEQ ID NO: 310 - protein, 499 aa, Artificial Sequence
  Synthetic Construct
MALPVTALLLPLALLLHAARPAVQLVESGGGLVQAGDSLRLTCTASGRAFSTYFMAWFRQAPGKEREFVAGIAWSGGSTAYADSVKGRFTISRDNAKNTVYLQMNSLKSEDTAVYYCASRGIEVEEFGAWGQGTQVTVSSGGGGSGGGGSGGGGSQVKLEESGGGLVQAGRSLRLSCAASEHTFSSHVMGWFRQAPGKERESVAVIGWRDISTSYADSVKGRFTISRDNAKKTLYLQMNSLKPEDTAVYYCAARRIDAADFDSWGQGTQVTVSSTSTTTPAPRPPTPAPTIASQPLSLRPEACRPAAGGAVHTRGLDFACDIYIWAPLAGTCGVLLLSLVITLYCKRGRKKLLYIFKQPFMRPVQTTQEEDGCSCRFPEEEEGGCELRVKFSRSADAPAYQQGQNQLYNELNLGRREEYDVLDKRRGRDPEMGGKPRRKNPQEGLYNELQKDKMAEAYSEIGMKGERRRGKGHDGLYQGLSTATKDTYDALHMQALPPR

SEQ ID NO: 311 - protein, 504 aa, Artificial Sequence
  Synthetic Construct
MALPVTALLLPLALLLHAARPAVQLVESGGGLVQAGDSLRLTCTASGRAFSTYFMAWFRQAPGKEREFVAGIAWSGGSTAYADSVKGRFTISRDNAKNTVYLQMNSLKSEDTAVYYCASRGIEVEEFGAWGQGTQVTVSSGGGGSGGGGSGGGGSGGGGSQVKLEESGGGLVQAGRSLRLSCAASEHTFSSHVMGWFRQAPGKERESVAVIGWRDISTSYADSVKGRFTISRDNAKKTLYLQMNSLKPEDTAVYYCAARRIDAADFDSWGQGTQVTVSSTSTTTPAPRPPTPAPTIASQPLSLRPEACRPAAGGAVHTRGLDFACDIYIWAPLAGTCGVLLLSLVITLYCKRGRKKLLYIFKQPFMRPVQTTQEEDGCSCRFPEEEEGGCELRVKFSRSADAPAYQQGQNQLYNELNLGRREEYDVLDKRRGRDPEMGGKPRRKNPQEGLYNELQKDKMAEAYSEIGMKGERRRGKGHDGLYQGLSTATKDTYDALHMQALPPR

SEQ ID NO: 312 - protein, 498 aa, Artificial Sequence
  Synthetic Construct
MALPVTALLLPLALLLHAARPEVQLVESGGGMVQAGDSLRLSCVQSTYTVNSDVMGWFRQAPGKEREFVGAIMWNDGITYLQDSVKGRFTIFRDNAKNTVYLQMNSLKLEDTAVYYCAASKGRYSEYEYWGQGTQVTVSSGGGGSQVKLEESGGRLVQPRGSLRLSCAGSGRTFSTYGMAWFRQAPGKEREFVASKASMNYSGRTYYADSVKGRFTIARDNAKNMVFLQMNNLKPEDTAVYYCAAGTGCSTYGCFDAQIIDYWGKGTLVTVSSTSTTTPAPRPPTPAPTIASQPLSLRPEACRPAAGGAVHTRGLDFACDIYIWAPLAGTCGVLLLSLVITLYCKRGRKKLLYIFKQPFMRPVQTTQEEDGCSCRFPEEEEGGCELRVKFSRSADAPAYQQGQNQLYNELNLGRREEYDVLDKRRGRDPEMGGKPRRKNPQEGLYNELQKDKMAEAYSEIGMKGERRRGKGHDGLYQGLSTATKDTYDALHMQALPPR

SEQ ID NO: 313 - protein, 508 aa, Artificial Sequence
  Synthetic Construct
MALPVTALLLPLALLLHAARPEVQLVESGGGMVQAGDSLRLSCVQSTYTVNSDVMGWFRQAPGKEREFVGAIMWNDGITYLQDSVKGRFTIFRDNAKNTVYLQMNSLKLEDTAVYYCAASKGRYSEYEYWGQGTQVTVSSGGGGSGGGGSGGGGSQVKLEESGGRLVQPRGSLRLSCAGSGRTFSTYGMAWFRQAPGKEREFVASKASMNYSGRTYYADSVKGRFTIARDNAKNMVFLQMNNLKPEDTAVYYCAAGTGCSTYGCFDAQIIDYWGKGTLVTVSSTSTTTPAPRPPTPAPTIASQPLSLRPEACRPAAGGAVHTRGLDFACDIYIWAPLAGTCGVLLLSLVITLYCKRGRKKLLYIFKQPFMRPVQTTQEEDGCSCRFPEEEEGGCELRVKFSRSADAPAYQQGQNQLYNELNLGRREEYDVLDKRRGRDPEMGGKPRRKNPQEGLYNELQKDKMAEAYSEIGMKGERRRGKGHDGLYQGLSTATKDTYDALHMQALPPR

SEQ ID NO: 314 - protein, 518 aa, Artificial Sequence
  Synthetic Construct
MALPVTALLLPLALLLHAARPEVQLVESGGGMVQAGDSLRLSCVQSTYTVNSDVMGWFRQAPGKEREFVGAIMWNDGITYLQDSVKGRFTIFRDNAKNTVYLQMNSLKLEDTAVYYCAASKGRYSEYEYWGQGTQVTVSSGGGGSGGGGSGGGGSGGGGSGGGGSQVKLEESGGRLVQPRGSLRLSCAGSGRTFSTYGMAWFRQAPGKEREFVASKASMNYSGRTYYADSVKGRFTIARDNAKNMVFLQMNNLKPEDTAVYYCAAGTGCSTYGCFDAQIIDYWGKGTLVTVSSTSTTTPAPRPPTPAPTIASQPLSLRPEACRPAAGGAVHTRGLDFACDIYIWAPLAGTCGVLLLSLVITLYCKRGRKKLLYIFKQPFMRPVQTTQEEDGCSCRFPEEEEGGCELRVKFSRSADAPAYQQGQNQLYNELNLGRREEYDVLDKRRGRDPEMGGKPRRKNPQEGLYNELQKDKMAEAYSEIGMKGERRRGKGHDGLYQGLSTATKDTYDALHMQALPPR

SEQ ID NO: 315 - protein, 503 aa, Artificial Sequence
  Synthetic Construct
MALPVTALLLPLALLLHAARPEVQLVESGGGMVQAGDSLRLSCVQSTYTVNSDVMGWFRQAPGKEREFVGAIMWNDGITYLQDSVKGRFTIFRDNAKNTVYLQMNSLKLEDTAVYYCAASKGRYSEYEYWGQGTQVTVSSGGGGSGGGGSQVKLEESGGRLVQPRGSLRLSCAGSGRTFSTYGMAWFRQAPGKEREFVASKASMNYSGRTYYADSVKGRFTIARDNAKNMVFLQMNNLKPEDTAVYYCAAGTGCSTYGCFDAQIIDYWGKGTLVTVSSTSTTTPAPRPPTPAPTIASQPLSLRPEACRPAAGGAVHTRGLDFACDIYIWAPLAGTCGVLLLSLVITLYCKRGRKKLLYIFKQPFMRPVQTTQEEDGCSCRFPEEEEGGCELRVKFSRSADAPAYQQGQNQLYNELNLGRREEYDVLDKRRGRDPEMGGKPRRKNPQEGLYNELQKDKMAEAYSEIGMKGERRRGKGHDGLYQGLSTATKDTYDALHMQALPPR

SEQ ID NO: 316 - protein, 508 aa, Artificial Sequence; identical to SEQ ID NO: 313
  Synthetic Construct

SEQ ID NO: 317 - protein, 513 aa, Artificial Sequence
  Synthetic Construct
MALPVTALLLPLALLLHAARPEVQLVESGGGMVQAGDSLRLSCVQSTYTVNSDVMGWFRQAPGKEREFVGAIMWNDGITYLQDSVKGRFTIFRDNAKNTVYLQMNSLKLEDTAVYYCAASKGRYSEYEYWGQGTQVTVSSGGGGSGGGGSGGGGSGGGGSQVKLEESGGRLVQPRGSLRLSCAGSGRTFSTYGMAWFRQAPGKEREFVASKASMNYSGRTYYADSVKGRFTIARDNAKNMVFLQMNNLKPEDTAVYYCAAGTGCSTYGCFDAQIIDYWGKGTLVTVSSTSTTTPAPRPPTPAPTIASQPLSLRPEACRPAAGGAVHTRGLDFACDIYIWAPLAGTCGVLLLSLVITLYCKRGRKKLLYIFKQPFMRPVQTTQEEDGCSCRFPEEEEGGCELRVKFSRSADAPAYQQGQNQLYNELNLGRREEYDVLDKRRGRDPEMGGKPRRKNPQEGLYNELQKDKMAEAYSEIGMKGERRRGKGHDGLYQGLSTATKDTYDALHMQALPPR

SEQ ID NO: 318 - protein, 500 aa, Artificial Sequence
  Synthetic Construct
MALPVTALLLPLALLLHAARPQVKLEESGGRLVQPRGSLRLSCAGSGRTFSTYGMAWFRQAPGKEREFVASKASMNYSGRTYYADSVKGRFTIARDNAKNMVFLQMNNLKPEDTAVYYCAAGTGCSTYGCFDAQIIDYWGKGTLVTVSSGGGGSQVKLEESGGGLVQAGGSLRLSCAASGGTLSKNTVAWVRQAPGKERGFVTSITCDGRTTYYANSVNGRFPINRNNAENLVVLQMNSLKPDDTALYYCAAYRKSIMSIQPDYWGQGTQVTVSSTSTTTPAPRPPTPAPTIASQPLSLRPEACRPAAGGAVHTRGLDFACDIYIWAPLAGTCGVLLLSLVITLYCKRGRKKLLYIFKQPFMRPVQTTQEEDGCSCRFPEEEEGGCELRVKFSRSADAPAYQQGQNQLYNELNLGRREEYDVLDKRRGRDPEMGGKPRRKNPQEGLYNELQKDKMAEAYSEIGMKGERRRGKGHDGLYQGLSTATKDTYDALHMQALPPR

SEQ ID NO: 319 - protein, 510 aa, Artificial Sequence
  Synthetic Construct
MALPVTALLLPLALLLHAARPQVKLEESGGRLVQPRGSLRLSCAGSGRTFSTYGMAWFRQAPGKEREFVASKASMNYSGRTYYADSVKGRFTIARDNAKNMVFLQMNNLKPEDTAVYYCAAGTGCSTYGCFDAQIIDYWGKGTLVTVSSGGGGSGGGGSGGGGSQVKLEESGGGLVQAGGSLRLSCAASGGTLSKNTVAWVRQAPGKERGFVTSITCDGRTTYYANSVNGRFPINRNNAENLVVLQMNSLKPDDTALYYCAAYRKSIMSIQPDYWGQGTQVTVSSTSTTTPAPRPPTPAPTIASQPLSLRPEACRPAAGGAVHTRGLDFACDIYIWAPLAGTCGVLLLSLVITLYCKRGRKKLLYIFKQPFMRPVQTTQEEDGCSCRFPEEEEGGCELRVKFSRSADAPAYQQGQNQLYNELNLGRREEYDVLDKRRGRDPEMGGKPRRKNPQEGLYNELQKDKMAEAYSEIGMKGERRRGKGHDGLYQGLSTATKDTYDALHMQALPPR

SEQ ID NO: 320 - protein, 520 aa, Artificial Sequence
  Synthetic Construct
MALPVTALLLPLALLLHAARPQVKLEESGGRLVQPRGSLRLSCAGSGRTFSTYGMAWFRQAPGKEREFVASKASMNYSGRTYYADSVKGRFTIARDNAKNMVFLQMNNLKPEDTAVYYCAAGTGCSTYGCFDAQIIDYWGKGTLVTVSSGGGGSGGGGSGGGGSGGGGSGGGGSQVKLEESGGGLVQAGGSLRLSCAASGGTLSKNTVAWVRQAPGKERGFVTSITCDGRTTYYANSVNGRFPINRNNAENLVVLQMNSLKPDDTALYYCAAYRKSIMSIQPDYWGQGTQVTVSSTSTTTPAPRPPTPAPTIASQPLSLRPEACRPAAGGAVHTRGLDFACDIYIWAPLAGTCGVLLLSLVITLYCKRGRKKLLYIFKQPFMRPVQTTQEEDGCSCRFPEEEEGGCELRVKFSRSADAPAYQQGQNQLYNELNLGRREEYDVLDKRRGRDPEMGGKPRRKNPQEGLYNELQKDKMAEAYSEIGMKGERRRGKGHDGLYQGLSTATKDTYDALHMQALPPR

SEQ ID NO: 321 - protein, 505 aa, Artificial Sequence
  Synthetic Construct
MALPVTALLLPLALLLHAARPQVKLEESGGRLVQPRGSLRLSCAGSGRTFSTYGMAWFRQAPGKEREFVASKASMNYSGRTYYADSVKGRFTIARDNAKNMVFLQMNNLKPEDTAVYYCAAGTGCSTYGCFDAQIIDYWGKGTLVTVSSGGGGSGGGGSQVKLEESGGGLVQAGGSLRLSCAASGGTLSKNTVAWVRQAPGKERGFVTSITCDGRTTYYANSVNGRFPINRNNAENLVVLQMNSLKPDDTALYYCAAYRKSIMSIQPDYWGQGTQVTVSSTSTTTPAPRPPTPAPTIASQPLSLRPEACRPAAGGAVHTRGLDFACDIYIWAPLAGTCGVLLLSLVITLYCKRGRKKLLYIFKQPFMRPVQTTQEEDGCSCRFPEEEEGGCELRVKFSRSADAPAYQQGQNQLYNELNLGRREEYDVLDKRRGRDPEMGGKPRRKNPQEGLYNELQKDKMAEAYSEIGMKGERRRGKGHDGLYQGLSTATKDTYDALHMQALPPR

SEQ ID NO: 322 - protein, 510 aa, Artificial Sequence; identical to SEQ ID NO: 319
  Synthetic Construct

SEQ ID NO: 323 - protein, 515 aa, Artificial Sequence
  Synthetic Construct
MALPVTALLLPLALLLHAARPQVKLEESGGRLVQPRGSLRLSCAGSGRTFSTYGMAWFRQAPGKEREFVASKASMNYSGRTYYADSVKGRFTIARDNAKNMVFLQMNNLKPEDTAVYYCAAGTGCSTYGCFDAQIIDYWGKGTLVTVSSGGGGSGGGGSGGGGSGGGGSQVKLEESGGGLVQAGGSLRLSCAASGGTLSKNTVAWVRQAPGKERGFVTSITCDGRTTYYANSVNGRFPINRNNAENLVVLQMNSLKPDDTALYYCAAYRKSIMSIQPDYWGQGTQVTVSSTSTTTPAPRPPTPAPTIASQPLSLRPEACRPAAGGAVHTRGLDFACDIYIWAPLAGTCGVLLLSLVITLYCKRGRKKLLYIFKQPFMRPVQTTQEEDGCSCRFPEEEEGGCELRVKFSRSADAPAYQQGQNQLYNELNLGRREEYDVLDKRRGRDPEMGGKPRRKNPQEGLYNELQKDKMAEAYSEIGMKGERRRGKGHDGLYQGLSTATKDTYDALHMQALPPR

SEQ ID NO: 324 - protein, 492 aa, Artificial Sequence
  Synthetic Construct
MALPVTALLLPLALLLHAARPQVKLEESGGGLVQAGGSLRLSCAASGGTLSKNTVAWVRQAPGKERGFVTSITCDGRTTYYANSVNGRFPINRNNAENLVVLQMNSLKPDDTALYYCAAYRKSIMSIQPDYWGQGTQVTVSSGGGGSQVQLVESGGGLVQAGGSLRLSCAASGGTLSKNTVAWFRQAPGKERGFVASITWDGRTTYYADSVKGRFTISRDNAKNTVYLQMNSLKPEDTAVYVCADLGKWPAGPADYWGQGTQVTVSSTSTTTPAPRPPTPAPTIASQPLSLRPEACRPAAGGAVHTRGLDFACDIYIWAPLAGTCGVLLLSLVITLYCKRGRKKLLYIFKQPFMRPVQTTQEEDGCSCRFPEEEEGGCELRVKFSRSADAPAYQQGQNQLYNELNLGRREEYDVLDKRRGRDPEMGGKPRRKNPQEGLYNELQKDKMAEAYSEIGMKGERRRGKGHDGLYQGLSTATKDTYDALHMQALPPR

SEQ ID NO: 325 - protein, 502 aa, Artificial Sequence
  Synthetic Construct
MALPVTALLLPLALLLHAARPQVKLEESGGGLVQAGGSLRLSCAASGGTLSKNTVAWVRQAPGKERGFVTSITCDGRTTYYANSVNGRFPINRNNAENLVVLQMNSLKPDDTALYYCAAYRKSIMSIQPDYWGQGTQVTVSSGGGGSGGGGSGGGGSQVQLVESGGGLVQAGGSLRLSCAASGGTLSKNTVAWFRQAPGKERGFVASITWDGRTTYYADSVKGRFTISRDNAKNTVYLQMNSLKPEDTAVYVCADLGKWPAGPADYWGQGTQVTVSSTSTTTPAPRPPTPAPTIASQPLSLRPEACRPAAGGAVHTRGLDFACDIYIWAPLAGTCGVLLLSLVITLYCKRGRKKLLYIFKQPFMRPVQTTQEEDGCSCRFPEEEEGGCELRVKFSRSADAPAYQQGQNQLYNELNLGRREEYDVLDKRRGRDPEMGGKPRRKNPQEGLYNELQKDKMAEAYSEIGMKGERRRGKGHDGLYQGLSTATKDTYDALHMQALPPR

SEQ ID NO: 326 - protein, 512 aa, Artificial Sequence
  Synthetic Construct
MALPVTALLLPLALLLHAARPQVKLEESGGGLVQAGGSLRLSCAASGGTLSKNTVAWVRQAPGKERGFVTSITCDGRTTYYANSVNGRFPINRNNAENLVVLQMNSLKPDDTALYYCAAYRKSIMSIQPDYWGQGTQVTVSSGGGGSGGGGSGGGGSGGGGSGGGGSQVQLVESGGGLVQAGGSLRLSCAASGGTLSKNTVAWFRQAPGKERGFVASITWDGRTTYYADSVKGRFTISRDNAKNTVYLQMNSLKPEDTAVYVCADLGKWPAGPADYWGQGTQVTVSSTSTTTPAPRPPTPAPTIASQPLSLRPEACRPAAGGAVHTRGLDFACDIYIWAPLAGTCGVLLLSLVITLYCKRGRKKLLYIFKQPFMRPVQTTQEEDGCSCRFPEEEEGGCELRVKFSRSADAPAYQQGQNQLYNELNLGRREEYDVLDKRRGRDPEMGGKPRRKNPQEGLYNELQKDKMAEAYSEIGMKGERRRGKGHDGLYQGLSTATKDTYDALHMQALPPR

SEQ ID NO: 327 - protein, 497 aa, Artificial Sequence
  Synthetic Construct
MALPVTALLLPLALLLHAARPQVKLEESGGGLVQAGGSLRLSCAASGGTLSKNTVAWVRQAPGKERGFVTSITCDGRTTYYANSVNGRFPINRNNAENLVVLQMNSLKPDDTALYYCAAYRKSIMSIQPDYWGQGTQVTVSSGGGGSGGGGSQVQLVESGGGLVQAGGSLRLSCAASGGTLSKNTVAWFRQAPGKERGFVASITWDGRTTYYADSVKGRFTISRDNAKNTVYLQMNSLKPEDTAVYVCADLGKWPAGPADYWGQGTQVTVSSTSTTTPAPRPPTPAPTIASQPLSLRPEACRPAAGGAVHTRGLDFACDIYIWAPLAGTCGVLLLSLVITLYCKRGRKKLLYIFKQPFMRPVQTTQEEDGCSCRFPEEEEGGCELRVKFSRSADAPAYQQGQNQLYNELNLGRREEYDVLDKRRGRDPEMGGKPRRKNPQEGLYNELQKDKMAEAYSEIGMKGERRRGKGHDGLYQGLSTATKDTYDALHMQALPPR

SEQ ID NO: 328 - protein, 502 aa, Artificial Sequence; identical to SEQ ID NO: 325
  Synthetic Construct

SEQ ID NO: 329 - protein, 507 aa, Artificial Sequence
  Synthetic Construct
MALPVTALLLPLALLLHAARPQVKLEESGGGLVQAGGSLRLSCAASGGTLSKNTVAWVRQAPGKERGFVTSITCDGRTTYYANSVNGRFPINRNNAENLVVLQMNSLKPDDTALYYCAAYRKSIMSIQPDYWGQGTQVTVSSGGGGSGGGGSGGGGSGGGGSQVQLVESGGGLVQAGGSLRLSCAASGGTLSKNTVAWFRQAPGKERGFVASITWDGRTTYYADSVKGRFTISRDNAKNTVYLQMNSLKPEDTAVYVCADLGKWPAGPADYWGQGTQVTVSSTSTTTPAPRPPTPAPTIASQPLSLRPEACRPAAGGAVHTRGLDFACDIYIWAPLAGTCGVLLLSLVITLYCKRGRKKLLYIFKQPFMRPVQTTQEEDGCSCRFPEEEEGGCELRVKFSRSADAPAYQQGQNQLYNELNLGRREEYDVLDKRRGRDPEMGGKPRRKNPQEGLYNELQKDKMAEAYSEIGMKGERRRGKGHDGLYQGLSTATKDTYDALHMQALPPR

SEQ ID NO: 330 - protein, 491 aa, Artificial Sequence
  Synthetic Construct
MALPVTALLLPLALLLHAARPQVQLVESGGGLVQAGGSLRLSCAASGGTLSKNTVAWFRQAPGKERGFVASITWDGRTTYYADSVKGRFTISRDNAKNTVYLQMNSLKPEDTAVYVCADLGKWPAGPADYWGQGTQVTVSSGGGGSDVQLVESGGGLVQAGGSLRLSCAASGGTLSKNTVAWVRQAPGKERGFVTSITCDGRTTYYANSVKGRFPISRDNAENTVYLQMNSLKPEDTAGYVCADLGKWPAGSADYWGQGTHVTVSSTSTTTPAPRPPTPAPTIASQPLSLRPEACRPAAGGAVHTRGLDFACDIYIWAPLAGTCGVLLLSLVITLYCKRGRKKLLYIFKQPFMRPVQTTQEEDGCSCRFPEEEEGGCELRVKFSRSADAPAYQQGQNQLYNELNLGRREEYDVLDKRRGRDPEMGGKPRRKNPQEGLYNELQKDKMAEAYSEIGMKGERRRGKGHDGLYQGLSTATKDTYDALHMQALPPR

SEQ ID NO: 331 - protein, 501 aa, Artificial Sequence
  Synthetic Construct
MALPVTALLLPLALLLHAARPQVQLVESGGGLVQAGGSLRLSCAASGGTLSKNTVAWFRQAPGKERGFVASITWDGRTTYYADSVKGRFTISRDNAKNTVYLQMNSLKPEDTAVYVCADLGKWPAGPADYWGQGTQVTVSSGGGGSGGGGSGGGGSDVQLVESGGGLVQAGGSLRLSCAASGGTLSKNTVAWVRQAPGKERGFVTSITCDGRTTYYANSVKGRFPISRDNAENTVYLQMNSLKPEDTAGYVCADLGKWPAGSADYWGQGTHVTVSSTSTTTPAPRPPTPAPTIASQPLSLRPEACRPAAGGAVHTRGLDFACDIYIWAPLAGTCGVLLLSLVITLYCKRGRKKLLYIFKQPFMRPVQTTQEEDGCSCRFPEEEEGGCELRVKFSRSADAPAYQQGQNQLYNELNLGRREEYDVLDKRRGRDPEMGGKPRRKNPQEGLYNELQKDKMAEAYSEIGMKGERRRGKGHDGLYQGLSTATKDTYDALHMQALPPR

SEQ ID NO: 332 - protein, 511 aa, Artificial Sequence
  Synthetic Construct
MALPVTALLLPLALLLHAARPQVQLVESGGGLVQAGGSLRLSCAASGGTLSKNTVAWFRQAPGKERGFVASITWDGRTTYYADSVKGRFTISRDNAKNTVYLQMNSLKPEDTAVYVCADLGKWPAGPADYWGQGTQVTVSSGGGGSGGGGSGGGGSGGGGSGGGGSDVQLVESGGGLVQAGGSLRLSCAASGGTLSKNTVAWVRQAPGKERGFVTSITCDGRTTYYANSVKGRFPISRDNAENTVYLQMNSLKPEDTAGYVCADLGKWPAGSADYWGQGTHVTVSSTSTTTPAPRPPTPAPTIASQPLSLRPEACRPAAGGAVHTRGLDFACDIYIWAPLAGTCGVLLLSLVITLYCKRGRKKLLYIFKQPFMRPVQTTQEEDGCSCRFPEEEEGGCELRVKFSRSADAPAYQQGQNQLYNELNLGRREEYDVLDKRRGRDPEMGGKPRRKNPQEGLYNELQKDKMAEAYSEIGMKGERRRGKGHDGLYQGLSTATKDTYDALHMQALPPR

SEQ ID NO: 333 - protein, 496 aa, Artificial Sequence
  Synthetic Construct
MALPVTALLLPLALLLHAARPQVQLVESGGGLVQAGGSLRLSCAASGGTLSKNTVAWFRQAPGKERGFVASITWDGRTTYYADSVKGRFTISRDNAKNTVYLQMNSLKPEDTAVYVCADLGKWPAGPADYWGQGTQVTVSSGGGGSGGGGSDVQLVESGGGLVQAGGSLRLSCAASGGTLSKNTVAWVRQAPGKERGFVTSITCDGRTTYYANSVKGRFPISRDNAENTVYLQMNSLKPEDTAGYVCADLGKWPAGSADYWGQGTHVTVSSTSTTTPAPRPPTPAPTIASQPLSLRPEACRPAAGGAVHTRGLDFACDIYIWAPLAGTCGVLLLSLVITLYCKRGRKKLLYIFKQPFMRPVQTTQEEDGCSCRFPEEEEGGCELRVKFSRSADAPAYQQGQNQLYNELNLGRREEYDVLDKRRGRDPEMGGKPRRKNPQEGLYNELQKDKMAEAYSEIGMKGERRRGKGHDGLYQGLSTATKDTYDALHMQALPPR

SEQ ID NO: 334 - protein, 501 aa, Artificial Sequence; identical to SEQ ID NO: 331
  Synthetic Construct

SEQ ID NO: 335 - protein, 506 aa, Artificial Sequence
  Synthetic Construct
MALPVTALLLPLALLLHAARPQVQLVESGGGLVQAGGSLRLSCAASGGTLSKNTVAWFRQAPGKERGFVASITWDGRTTYYADSVKGRFTISRDNAKNTVYLQMNSLKPEDTAVYVCADLGKWPAGPADYWGQGTQVTVSSGGGGSGGGGSGGGGSGGGGSDVQLVESGGGLVQAGGSLRLSCAASGGTLSKNTVAWVRQAPGKERGFVTSITCDGRTTYYANSVKGRFPISRDNAENTVYLQMNSLKPEDTAGYVCADLGKWPAGSADYWGQGTHVTVSSTSTTTPAPRPPTPAPTIASQPLSLRPEACRPAAGGAVHTRGLDFACDIYIWAPLAGTCGVLLLSLVITLYCKRGRKKLLYIFKQPFMRPVQTTQEEDGCSCRFPEEEEGGCELRVKFSRSADAPAYQQGQNQLYNELNLGRREEYDVLDKRRGRDPEMGGKPRRKNPQEGLYNELQKDKMAEAYSEIGMKGERRRGKGHDGLYQGLSTATKDTYDALHMQALPPR

SEQ ID NO: 336 - DNA, 1488 bp, Artificial Sequence
  Synthetic Construct
atggctctgcccgtcactgctctgctgctgcccctggctctgctgctgcacgctgctcgccctcaggtccagctggtggaaagcggaggaggcctggtgcagccaggaggcagcctgaggctgtcctgcgaggcctctggcttcaccctggactactatgccatcggctggtttaggcaggcacctggaaaggagagggagggagtgatctgtatctctcgcagcgacggcagcacatactatgccgattccgtgaagggccggttcaccatcagcagagacaacgccaagaagacagtgtacctgcagatgatctccctgaagcctgaggataccgcagcatactattgcgcagcaggagcagactgtagcggatacctgagggattatgagtttaggggacagggaacccaggtgacagtgagctccggaggaggaggctcccaggtgcagctggtggagtctggaggcggcctggtgcagcctggaggcagcctgagactgagctgtgaagcttccggatttaccctggactactatgcaatcggatggtttaggcaggcaccaggaaaggagagagaaggcgtgatctgtatctccagatctgacggctctacatactatgccgatagtgtcaaaggacggttcaccatctctagagataatgccaagaagacagtctatctgcagatgattagcctgaagcccgaggacacagccgcctattactgcgcagcaggagcagattgtagtgggtatctgagggactatgagtttcgggggcaggggacacaggtgacagtgagttctactagtaccacgacgccagcgccgcgaccaccaacaccggcgcccaccatcgcgtcgcagcccctgtccctgcgcccagaggcgtgccggccagcggcggggggcgcagtgcacacgagggggctggacttcgcctgtgatatctacatctgggcgcccttggccgggacttgtggggtccttctcctgtcactggttatcaccctttactgcaaacggggcagaaagaaactcctgtatatattcaaacaaccatttatgagaccagtacaaactactcaagaggaagatggctgtagctgccgatttccagaagaagaagaaggaggatgtgaactgagagtgaagttcagcaggagcgcagacgcccccgcgtaccagcagggccagaaccagctctataacgagctcaatctaggacgaagagaggagtacgatgttttggacaagagacgtggccgggaccctgagatggggggaaagccgagaaggaagaaccctcaggaaggcctgtacaatgaactgcagaaagataagatggcggaggcctacagtgagattgggatgaaaggcgagcgccggaggggcaaggggcacgatggcctttaccagggtctcagtacagccaccaaggacacctacgacgcccttcacatgcaggccctgccccctcgctaa

SEQ ID NO: 337 - DNA, 1869 bp, Artificial Sequence
  Synthetic Construct
atggctctgcccgtcactgctctgctgctgcctctggccctgctgctgcacgccgcacgccctcaggtccagctggtcgagtcaggaggaggcctggtgcagccaggaggctccctgcggctgtcttgcgaggccagcggcttcaccctggactactatgccatcggctggtttaggcaggcacctggaaaggagagggagggagtgatctgtatctccagatctgacggctccacatactatgccgattctgtgaagggccggttcaccatctctagagacaacgccaagaagacagtgtacctgcagatgatcagcctgaagcccgaggataccgcagcatactattgcgcagcaggagcagactgttccggatacctgagggattatgagtttaggggacagggaacccaggtgacagtgagctccggaggaggaggctcccaggtgcagctggtggagtctggaggcggcctggtgcagcctggaggctccctgaggctgtcttgcgaggcaagcggcttcaccctggattactatgcaatcggatggtttaggcaggcaccaggaaaggagagagaaggcgtgatctgtatcagccgctccgacggcagtacctactatgccgattccgtcaaaggccggttcaccatctccagagacaatgccaagaagacagtctatctgcagatgatctctctgaagcctgaggatacagccgcctattactgtgccgcaggagcagactgtagtggctatctgagagattatgagtttcgcggccagggcacccaggtgacagtgtctagcggaggaggaggcagccaggtccagctggtggaatccggcggaggcctggtgcagcccggcggctccctgagactgtcctgtgaagcctccggatttactctggattattacgctattggatggttcagacaggcccctggcaaagaaagagaaggggtgatctgtatctctcggagcgacggctctacatactatgccgatagcgtcaagggaagatttaccatctccagagataatgccaagaagacagtgtatctgcagatgatttccctgaagcccgaggacactgccgcctattactgtgcagcaggagcagattgtagcgggtatctgcgggattatgaatttagaggacagggcactcaggtgacagtctcaagcactagtaccacgacgccagcgccgcgaccaccaacaccggcgcccaccatcgcgtcgcagcccctgtccctgcgcccagaggcgtgccggccagcggcggggggcgcagtgcacacgagggggctggacttcgcctgtgatatctacatctgggcgcccttggccgggacttgtggggtccttctcctgtcactggttatcaccctttactgcaaacggggcagaaagaaactcctgtatatattcaaacaaccatttatgagaccagtacaaactactcaagaggaagatggctgtagctgccgatttccagaagaagaagaaggaggatgtgaactgagagtgaagttcagcaggagcgcagacgcccccgcgtaccagcagggccagaaccagctctataacgagctcaatctaggacgaagagaggagtacgatgttttggacaagagacgtggccgggaccctgagatggggggaaagccgagaaggaagaaccctcaggaaggcctgtacaatgaactgcagaaagataagatggcggaggcctacagtgagattgggatgaaaggcgagcgccggaggggcaaggggcacgatggcctttaccagggtctcagtacagccaccaaggacacctacgacgcccttcacatgcaggccctgccccctcgctaa

SEQ ID NO: 338 - DNA, 1467 bp, Artificial Sequence
  Synthetic Construct
atggctctgcccgtcaccgctctgctgctgcctctggctctgctgctgcacgctgctcgccctcaggtcaaactggaagaatctggcggaggcctggtgcaggcaggacggagcctgcgcctgagctgcgcagcatccgagcacaccttcagctcccacgtgatgggctggtttcggcaggccccaggcaaggagagagagagcgtggccgtgatcggctggagggacatctccacatcttacgccgattccgtgaagggccggttcaccatcagccgggacaacgccaagaagacactgtatctgcagatgaacagcctgaagcccgaggacaccgccgtgtactattgcgcagcaaggagaatcgacgcagcagactttgattcctggggccagggcacccaggtgacagtgtctagcggaggaggaggatctgaggtgcagctggtggagagcggaggcggcctggtgcaggccggaggctctctgaggctgagctgtgcagcatccggaagaaccttcacaatgggctggtttaggcaggcaccaggaaaggagagggagttcgtggcagcaatcagcctgtcccctaccctggcctactatgccgagagcgtgaagggcaggtttaccatctcccgcgataacgccaagaatacagtggtgctgcagatgaactccctgaaacctgaggacacagccctgtactattgtgccgccgatcggaagagcgtgatgagcattagaccagactattgggggcagggaacacaggtgaccgtgagcagcactagtaccacgacgccagcgccgcgaccaccaacaccggcgcccaccatcgcgtcgcagcccctgtccctgcgcccagaggcgtgccggccagcggcggggggcgcagtgcacacgagggggctggacttcgcctgtgatatctacatctgggcgcccttggccgggacttgtggggtccttctcctgtcactggttatcaccctttactgcaaacggggcagaaagaaactcctgtatatattcaaacaaccatttatgagaccagtacaaactactcaagaggaagatggctgtagctgccgatttccagaagaagaagaaggaggatgtgaactgagagtgaagttcagcaggagcgcagacgcccccgcgtaccagcagggccagaaccagctctataacgagctcaatctaggacgaagagaggagtacgatgttttggacaagagacgtggccgggaccctgagatggggggaaagccgagaaggaagaaccctcaggaaggcctgtacaatgaactgcagaaagataagatggcggaggcctacagtgagattgggatgaaaggcgagcgccggaggggcaaggggcacgatggcctttaccagggtctcagtacagccaccaaggacacctacgacgcccttcacatgcaggccctgccccctcgctaa

SEQ ID NO: 339 - DNA, 1497 bp, Artificial Sequence
  Synthetic Construct
atggctctgcctgtcaccgctctgctgctgcctctggctctgctgctgcacgctgctcgccctcaggtcaaactggaagaaagtgggggaggcctggtgcaggcaggacggagcctgcgcctgagctgcgcagcatccgagcacaccttcagctcccacgtgatgggctggtttcggcaggccccaggcaaggagagagagtccgtggccgtgatcggctggagggacatctccacatcttacgccgattctgtgaagggccggttcaccatcagcagagacaacgccaagaagacactgtatctgcagatgaatagcctgaagcccgaggacaccgccgtgtactattgcgcagcaaggagaatcgacgcagcagactttgattcctggggccagggcacccaggtgacagtgtctagcggaggaggaggatctggaggaggaggaagcggaggaggaggatccgaggtgcagctggtggagtctggaggcggcctggtgcaggccggaggctctctgaggctgagctgtgcagcatccggaagaaccttcacaatgggctggtttaggcaggcaccaggaaaggagagggagttcgtggcagcaatcagcctgtcccctaccctggcctactatgccgagtccgtgaagggcaggtttaccatctctcgcgataacgccaagaatacagtggtgctgcagatgaacagcctgaaacctgaggacacagccctgtactattgtgccgccgatcggaagagcgtgatgagcattagacccgattattggggacagggcacacaggtgacagtgagtagcactagtaccacgacgccagcgccgcgaccaccaacaccggcgcccaccatcgcgtcgcagcccctgtccctgcgcccagaggcgtgccggccagcggcggggggcgcagtgcacacgagggggctggacttcgcctgtgatatctacatctgggcgcccttggccgggacttgtggggtccttctcctgtcactggttatcaccctttactgcaaacggggcagaaagaaactcctgtatatattcaaacaaccatttatgagaccagtacaaactactcaagaggaagatggctgtagctgccgatttccagaagaagaagaaggaggatgtgaactgagagtgaagttcagcaggagcgcagacgcccccgcgtaccagcagggccagaaccagctctataacgagctcaatctaggacgaagagaggagtacgatgttttggacaagagacgtggccgggaccctgagatggggggaaagccgagaaggaagaaccctcaggaaggcctgtacaatgaactgcagaaagataagatggcggaggcctacagtgagattgggatgaaaggcgagcgccggaggggcaaggggcacgatggcctttaccagggtctcagtacagccaccaaggacacctacgacgcccttcacatgcaggccctgccccctcgctaa

SEQ ID NO: 340 - DNA, 1527 bp, Artificial Sequence
  Synthetic Construct
atggctctgcccgtcaccgcactgctgctgcctctggctctgctgctgcacgccgcaagaccacaggtcaaactggaagaatcaggaggaggcctggtgcaggcaggacggagcctgcgcctgagctgcgcagcatccgagcacaccttcagctcccacgtgatgggctggtttcggcaggccccaggcaaggagagagagtccgtggccgtgatcggctggagggacatctccacatcttacgccgattccgtgaagggccggttcaccatcagccgggacaacgccaagaagacactgtatctgcagatgaacagcctgaagcccgaggacaccgccgtgtactattgcgcagcaaggagaatcgacgcagcagactttgatagctggggccagggcacccaggtgacagtgtctagcggaggaggaggatctggaggaggaggaagcggaggaggaggaagcggcggcggcggctctggcggcggcggcagcgaggtgcagctggtggagagcggcggcggcctggtgcaggccggcggctctctgaggctgagctgtgcagcatccggaagaaccttcacaatgggctggtttaggcaggcaccaggaaaggagagggagttcgtggcagcaatcagcctgtcccctaccctggcctactatgccgagagcgtgaagggcaggtttaccatctcccgcgataacgccaagaatacagtggtgttacaaatgaacagcctgaaacctgaggacacagccctgtactattgtgccgccgatcggaagagcgtgatgagcattagacccgattattgggggcaggggacacaggtgaccgtgagcagcactagtaccacgacgccagcgccgcgaccaccaacaccggcgcccaccatcgcgtcgcagcccctgtccctgcgcccagaggcgtgccggccagcggcggggggcgcagtgcacacgagggggctggacttcgcctgtgatatctacatctgggcgcccttggccgggacttgtggggtccttctcctgtcactggttatcaccctttactgcaaacggggcagaaagaaactcctgtatatattcaaacaaccatttatgagaccagtacaaactactcaagaggaagatggctgtagctgccgatttccagaagaagaagaaggaggatgtgaactgagagtgaagttcagcaggagcgcagacgcccccgcgtaccagcagggccagaaccagctctataacgagctcaatctaggacgaagagaggagtacgatgttttggacaagagacgtggccgggaccctgagatggggggaaagccgagaaggaagaaccctcaggaaggcctgtacaatgaactgcagaaagataagatggcggaggcctacagtgagattgggatgaaaggcgagcgccggaggggcaaggggcacgatggcctttaccagggtctcagtacagccaccaaggacacctacgacgcccttcacatgcaggccctgccccctcgctaa

SEQ ID NO: 341 - DNA, 1482 bp, Artificial Sequence
  Synthetic Construct
atggctctgcctgtgaccgcactgctgctgcctctggctctgctgctgcacgccgcacgacctgaagtccagctggtggaatccgggggaggcctggtgcaggcaggaggctccctgaggctgtcttgcgcagcaagcggaagaaccttcacaatgggctggtttaggcaggcaccaggaaaggagagggagttcgtggccgccatctccctgtctcctaccctggcctactatgccgagagcgtgaagggcaggtttaccatctcccgcgacaacgccaagaatacagtggtgctgcagatgaacagcctgaagccagaggacacagccctgtactattgcgccgccgatcggaagtctgtgatgagcatcagacccgattactggggccagggcacccaggtgacagtgagctccggaggaggaggatccggcggaggaggctctcaggtgaagctggaggagtccggaggcggcctggtgcaggccggacggtccctgagactgtcttgtgccgccagcgagcacaccttctctagccacgtgatgggatggttcaggcaggcacctggaaaggagagggagtccgtggcagtgatcggatggagggacatcagcacatcctacgccgattctgtgaagggccggttcaccatcagcagagacaacgccaagaagacactgtatttacaaatgaacagcctgaagcccgaggataccgccgtgtactattgtgccgcccggcggattgacgccgcagactttgactcatgggggcagggaactcaggtgaccgtgtcctcaactagtaccacgacgccagcgccgcgaccaccaacaccggcgcccaccatcgcgtcgcagcccctgtccctgcgcccagaggcgtgccggccagcggcggggggcgcagtgcacacgagggggctggacttcgcctgtgatatctacatctgggcgcccttggccgggacttgtggggtccttctcctgtcactggttatcaccctttactgcaaacggggcagaaagaaactcctgtatatattcaaacaaccatttatgagaccagtacaaactactcaagaggaagatggctgtagctgccgatttccagaagaagaagaaggaggatgtgaactgagagtgaagttcagcaggagcgcagacgcccccgcgtaccagcagggccagaaccagctctataacgagctcaatctaggacgaagagaggagtacgatgttttggacaagagacgtggccgggaccctgagatggggggaaagccgagaaggaagaaccctcaggaaggcctgtacaatgaactgcagaaagataagatggcggaggcctacagtgagattgggatgaaaggcgagcgccggaggggcaaggggcacgatggcctttaccagggtctcagtacagccaccaaggacacctacgacgcccttcacatgcaggccctgccccctcgctaa

SEQ ID NO: 342 - DNA, 1497 bp, Artificial Sequence
  Synthetic Construct
atggccctgcctgtcaccgctctgctgctgcccctggccctgctgctgcacgccgcacgccctgaggtccagctggtcgagtccgggggaggcctggtgcaggcaggaggctccctgaggctgtcttgcgcagcaagcggaagaaccttcacaatgggctggtttaggcaggcaccaggaaaggagagggagttcgtggccgccatctccctgtctcctaccctggcctactatgccgagtccgtgaagggcaggtttaccatctctcgcgacaacgccaagaatacagtggtgctgcagatgaactccctgaagccagaggacacagccctgtactattgcgccgccgatcggaagtctgtgatgagcatcagacccgattactggggccagggcacccaggtgacagtgagctccggaggaggaggatccggcggaggaggctctggcggcggcggcagccaggtgaagctggaggagagcggaggcggcctggtgcaggccggacggtccctgagactgtcttgtgccgccagcgagcacaccttctctagccacgtgatgggatggttcaggcaggcacctggaaaggagagggagtctgtggccgtgatcggctggagggacatcagcacatcctacgccgatagcgtgaagggccggttcaccatctccagagacaacgccaagaagacactgtatctgcagatgaatagcctgaagcccgaggataccgccgtgtactattgtgccgcccggcggattgacgccgcagattttgattcttgggggcagggaactcaggtgaccgtgtcctcaactagtaccacgacgccagcgccgcgaccaccaacaccggcgcccaccatcgcgtcgcagcccctgtccctgcgcccagaggcgtgccggccagcggcggggggcgcagtgcacacgagggggctggacttcgcctgtgatatctacatctgggcgcccttggccgggacttgtggggtccttctcctgtcactggttatcaccctttactgcaaacggggcagaaagaaactcctgtatatattcaaacaaccatttatgagaccagtacaaactactcaagaggaagatggctgtagctgccgatttccagaagaagaagaaggaggatgtgaactgagagtgaagttcagcaggagcgcagacgcccccgcgtaccagcagggccagaaccagctctataacgagctcaatctaggacgaagagaggagtacgatgttttggacaagagacgtggccgggaccctgagatggggggaaagccgagaaggaagaaccctcaggaaggcctgtacaatgaactgcagaaagataagatggcggaggcctacagtgagattgggatgaaaggcgagcgccggaggggcaaggggcacgatggcctttaccagggtctcagtacagccaccaaggacacctacgacgcccttcacatgcaggccctgccccctcgctaa

SEQ ID NO: 343 - DNA, 1512 bp, Artificial Sequence
  Synthetic Construct
atggctctgcctgtgaccgccctgctgctgcccctggccctgctgctgcacgccgcacgacctgaagtccagctggtggaatctggcggaggcctggtgcaggcaggaggctccctgaggctgtcttgcgcagcaagcggaagaaccttcacaatgggctggtttaggcaggcaccaggaaaggagagggagttcgtggccgccatctccctgtctcctaccctggcctactatgccgagtctgtgaagggcaggtttaccatcagccgcgacaacgccaagaatacagtggtgctgcagatgaacagcctgaagccagaggacacagccctgtactattgcgccgccgatcggaagtctgtgatgagcatcagacccgattactggggccagggcacccaggtgacagtgagctccggaggaggaggatccggcggaggaggctctggcggcggcggctccggcggcggcggctcccaggtgaagctggaggagtccggaggcggcctggtgcaggccggacggtccctgagactgtcttgtgccgccagcgagcacaccttctctagccacgtgatgggatggttcaggcaggcacctggaaaggagagggagagcgtggcagtgatcggatggagggacatcagcacatcctacgccgattccgtgaagggccggttcaccatcagccgggacaacgccaagaagacactgtatttacaaatgaacagcctgaagcccgaggataccgccgtgtactattgtgccgcccggcggattgatgccgcagactttgatagttggggacaggggactcaggtcaccgtcagcagcactagtaccacgacgccagcgccgcgaccaccaacaccggcgcccaccatcgcgtcgcagcccctgtccctgcgcccagaggcgtgccggccagcggcggggggcgcagtgcacacgagggggctggacttcgcctgtgatatctacatctgggcgcccttggccgggacttgtggggtccttctcctgtcactggttatcaccctttactgcaaacggggcagaaagaaactcctgtatatattcaaacaaccatttatgagaccagtacaaactactcaagaggaagatggctgtagctgccgatttccagaagaagaagaaggaggatgtgaactgagagtgaagttcagcaggagcgcagacgcccccgcgtaccagcagggccagaaccagctctataacgagctcaatctaggacgaagagaggagtacgatgttttggacaagagacgtggccgggaccctgagatggggggaaagccgagaaggaagaaccctcaggaaggcctgtacaatgaactgcagaaagataagatggcggaggcctacagtgagattgggatgaaaggcgagcgccggaggggcaaggggcacgatggcctttaccagggtctcagtacagccaccaaggacacctacgacgcccttcacatgcaggccctgccccctcgctaa

SEQ ID NO: 344 - DNA, 1470 bp, Artificial Sequence
  Synthetic Construct
atggctctgcccgtcaccgcactgctgctgcctctggctctgctgctgcacgctgctcgccctcaggtcaaactggaagaatctggcggaggcctggtgcaggcaggcaggtccctgaggctgtcttgcgcagcaagcgagcacacctttagctcccacgtgatgggatggttcaggcaggcaccaggcaaggagagagagtccgtggccgtgatcggctggagggacatctccacatcttacgccgattctgtgaagggccggtttaccatcagcagagacaacgccaagaagacactgtatctgcagatgaatagcctgaagcctgaggacaccgccgtgtactattgcgcagcaaggagaatcgatgcagcagacttcgattcctggggacagggaacccaggtgacagtgtctagcggaggaggaggaagcgccgtgcagctggtggagtccggcggcggcctggtgcaggccggcgattctctgcggctgacctgtacagcctccggcagagccttctctacctactttatggcctggtttagacaggcccctggcaaggagagggagtttgtggcaggaatcgcatggagcggaggatccacagcatacgccgactccgtgaagggcaggttcaccatctctcgcgataacgccaagaatacagtgtatctgcagatgaactctctgaagagcgaggacacagccgtgtactattgtgccagccggggaatcgaggtggaggaatttggggcttgggggcagggaactcaggtgaccgtctcatcaactagtaccacgacgccagcgccgcgaccaccaacaccggcgcccaccatcgcgtcgcagcccctgtccctgcgcccagaggcgtgccggccagcggcggggggcgcagtgcacacgagggggctggacttcgcctgtgatatctacatctgggcgcccttggccgggacttgtggggtccttctcctgtcactggttatcaccctttactgcaaacggggcagaaagaaactcctgtatatattcaaacaaccatttatgagaccagtacaaactactcaagaggaagatggctgtagctgccgatttccagaagaagaagaaggaggatgtgaactgagagtgaagttcagcaggagcgcagacgcccccgcgtaccagcagggccagaaccagctctataacgagctcaatctaggacgaagagaggagtacgatgttttggacaagagacgtggccgggaccctgagatggggggaaagccgagaaggaagaaccctcaggaaggcctgtacaatgaactgcagaaagataagatggcggaggcctacagtgagattgggatgaaaggcgagcgccggaggggcaaggggcacgatggcctttaccagggtctcagtacagccaccaaggacacctacgacgcccttcacatgcaggccctgccccctcgctaa

SEQ ID NO: 345 - DNA, 1500 bp, Artificial Sequence
  Synthetic Construct
atggctctgcccgtcaccgctctgctgctgcctctggctctgctgctgcacgctgctcgccctcaggtcaaactggaagaatctggcggaggcctggtgcaggcaggcaggtccctgaggctgtcttgcgcagcaagcgagcacacctttagctcccacgtgatgggatggttcaggcaggcaccaggcaaggagagagagagcgtggccgtgatcggctggagggacatctccacatcttacgccgatagcgtgaagggccggtttaccatctccagagacaacgccaagaagacactgtatctgcagatgaatagcctgaagcctgaggacaccgccgtgtactattgcgcagcaaggagaatcgatgcagcagacttcgattcctggggacagggaacccaggtgacagtgtctagcggaggaggaggatccggaggaggaggatctggcggcggcggcagcgccgtgcagctggtggagtccggcggcggcctggtgcaggccggcgactctctgaggctgacctgtacagcctccggcagagccttctctacctactttatggcctggtttagacaggcccctggcaaggagagggagtttgtggcaggaatcgcatggagcggaggatccacagcatacgcagactctgtgaagggcaggttcaccatcagccgcgataacgccaagaatacagtgtatctgcagatgaactctctgaagagcgaggatacagccgtgtactattgtgcctcccgggggattgaagtcgaggaatttggggcttgggggcagggcactcaggtcaccgtctcatctactagtaccacgacgccagcgccgcgaccaccaacaccggcgcccaccatcgcgtcgcagcccctgtccctgcgcccagaggcgtgccggccagcggcggggggcgcagtgcacacgagggggctggacttcgcctgtgatatctacatctgggcgcccttggccgggacttgtggggtccttctcctgtcactggttatcaccctttactgcaaacggggcagaaagaaactcctgtatatattcaaacaaccatttatgagaccagtacaaactactcaagaggaagatggctgtagctgccgatttccagaagaagaagaaggaggatgtgaactgagagtgaagttcagcaggagcgcagacgcccccgcgtaccagcagggccagaaccagctctataacgagctcaatctaggacgaagagaggagtacgatgttttggacaagagacgtggccgggaccctgagatggggggaaagccgagaaggaagaaccctcaggaaggcctgtacaatgaactgcagaaagataagatggcggaggcctacagtgagattgggatgaaaggcgagcgccggaggggcaaggggcacgatggcctttaccagggtctcagtacagccaccaaggacacctacgacgcccttcacatgcaggccctgccccctcgctaa

SEQ ID NO: 346 - DNA, 1530 bp, Artificial Sequence
  Synthetic Construct
atggctctgcccgtcactgctctgctgctgcctctggctctgctgctgcacgctgctagaccacaggtcaaactggaggagtcagggggaggcctggtgcaggcaggcaggtccctgaggctgtcttgcgcagcaagcgagcacacctttagctcccacgtgatgggatggttcaggcaggcaccaggcaaggagagagagagcgtggccgtgatcggctggagggacatctccacatcttacgccgattctgtgaagggccggtttaccatcagcagagacaacgccaagaagacactgtatctgcagatgaacagcctgaagcctgaggacaccgccgtgtactattgcgcagcaaggagaatcgatgcagcagacttcgattcctggggacagggaacccaggtgacagtgtctagcggaggaggaggatccggaggaggaggatctggcggcggcggcagtggcggcggcggctccggcggcggcggctctgccgtgcagctggtggagtccggcggcggcctggtgcaggccggcgactccctgaggctgacctgtacagccagcggcagagccttctccacctactttatggcctggtttagacaggcccctggcaaggagagggagtttgtggcaggaatcgcatggagcggaggatccacagcatacgccgactccgtgaagggcaggttcaccatctctcgcgataacgccaagaatacagtgtatctgcagatgaactctctgaagagcgaggatacagccgtgtactattgtgcctcccggggcattgaagtggaagaatttggggcttggggacaggggactcaggtcaccgtcagcagcactagtaccacgacgccagcgccgcgaccaccaacaccggcgcccaccatcgcgtcgcagcccctgtccctgcgcccagaggcgtgccggccagcggcggggggcgcagtgcacacgagggggctggacttcgcctgtgatatctacatctgggcgcccttggccgggacttgtggggtccttctcctgtcactggttatcaccctttactgcaaacggggcagaaagaaactcctgtatatattcaaacaaccatttatgagaccagtacaaactactcaagaggaagatggctgtagctgccgatttccagaagaagaagaaggaggatgtgaactgagagtgaagttcagcaggagcgcagacgcccccgcgtaccagcagggccagaaccagctctataacgagctcaatctaggacgaagagaggagtacgatgttttggacaagagacgtggccgggaccctgagatggggggaaagccgagaaggaagaaccctcaggaaggcctgtacaatgaactgcagaaagataagatggcggaggcctacagtgagattgggatgaaaggcgagcgccggaggggcaaggggcacgatggcctttaccagggtctcagtacagccaccaaggacacctacgacgcccttcacatgcaggccctgccccctcgctaa

SEQ ID NO: 347 - DNA, 1485 bp, Artificial Sequence
  Synthetic Construct
atggctctgcccgtgaccgctctgctgctgcctctggctctgctgctgcatgctgctcgccctcaggtgaaactggaagaatctggcggaggcctggtgcaggcaggcaggtccctgaggctgtcttgcgcagcaagcgagcacacctttagctcccacgtgatgggatggttcaggcaggcaccaggcaaggagagagagtccgtggccgtgatcggctggagggacatctccacatcttacgccgattctgtgaagggccggtttaccatcagcagagacaacgccaagaagacactgtatctgcagatgaacagcctgaagcctgaggacaccgccgtgtactattgcgcagcaaggagaatcgatgcagcagacttcgatagctggggacagggaacccaggtgacagtgtctagcggaggaggaggatccggaggaggaggatctgccgtgcagctggtggagagcggcggcggcctggtgcaggccggcgattccctgaggctgacctgtacagccagcggcagagccttctccacctactttatggcctggtttagacaggcccctggcaaggagagggagtttgtggcaggaatcgcatggagcggaggatccacagcatacgccgactccgtgaagggcaggttcaccatctctcgcgataacgccaagaatacagtgtatctgcagatgaactctctgaagagcgaggacacagccgtgtactattgtgccagccgggggattgaagtggaagaatttggggcttgggggcaggggactcaggtcacagtgtcatctactagtaccacgacgccagcgccgcgaccaccaacaccggcgcccaccatcgcgtcgcagcccctgtccctgcgcccagaggcgtgccggccagcggcggggggcgcagtgcacacgagggggctggacttcgcctgtgatatctacatctgggcgcccttggccgggacttgtggggtccttctcctgtcactggttatcaccctttactgcaaacggggcagaaagaaactcctgtatatattcaaacaaccatttatgagaccagtacaaactactcaagaggaagatggctgtagctgccgatttccagaagaagaagaaggaggatgtgaactgagagtgaagttcagcaggagcgcagacgcccccgcgtaccagcagggccagaaccagctctataacgagctcaatctaggacgaagagaggagtacgatgttttggacaagagacgtggccgggaccctgagatggggggaaagccgagaaggaagaaccctcaggaaggcctgtacaatgaactgcagaaagataagatggcggaggcctacagtgagattgggatgaaaggcgagcgccggaggggcaaggggcacgatggcctttaccagggtctcagtacagccaccaaggacacctacgacgcccttcacatgcaggccctgccccctcgctaa

SEQ ID NO: 348 - DNA, 1500 bp, Artificial Sequence
  Synthetic Construct
atggctctgcccgtcaccgcactgctgctgcccctggctctgctgctgcacgctgctcgccctcaggtcaaactggaagaatctggaggaggcctggtgcaggcaggcaggtccctgaggctgtcttgcgcagcaagcgagcacacctttagctcccacgtgatgggatggttcaggcaggcaccaggcaaggagagagagagcgtggccgtgatcggctggagggacatctccacatcttacgccgatagcgtgaagggccggtttaccatctccagagacaacgccaagaagacactgtatctgcagatgaatagcctgaagcctgaggacaccgccgtgtactattgcgcagcaaggagaatcgatgcagcagacttcgattcctggggacagggaacccaggtgacagtgtctagcggaggaggaggatccggaggaggaggatctggcggcggcggcagcgccgtgcagctggtggagtccggcggcggcctggtgcaggccggcgactctctgaggctgacctgtacagcctccggcagagccttctctacctactttatggcctggtttagacaggcccctggcaaggagagggagtttgtggcaggaatcgcatggagcggaggatccacagcatacgcagactctgtgaagggcaggttcaccatcagccgcgataacgccaagaatacagtgtatctgcagatgaactctctgaagagcgaggatacagccgtgtactattgtgcctcccgggggattgaagtggaagaatttggggcttgggggcaggggactcaggtcaccgtcagcagcactagtaccacgacgccagcgccgcgaccaccaacaccggcgcccaccatcgcgtcgcagcccctgtccctgcgcccagaggcgtgccggccagcggcggggggcgcagtgcacacgagggggctggacttcgcctgtgatatctacatctgggcgcccttggccgggacttgtggggtccttctcctgtcactggttatcaccctttactgcaaacggggcagaaagaaactcctgtatatattcaaacaaccatttatgagaccagtacaaactactcaagaggaagatggctgtagctgccgatttccagaagaagaagaaggaggatgtgaactgagagtgaagttcagcaggagcgcagacgcccccgcgtaccagcagggccagaaccagctctataacgagctcaatctaggacgaagagaggagtacgatgttttggacaagagacgtggccgggaccctgagatggggggaaagccgagaaggaagaaccctcaggaaggcctgtacaatgaactgcagaaagataagatggcggaggcctacagtgagattgggatgaaaggcgagcgccggaggggcaaggggcacgatggcctttaccagggtctcagtacagccaccaaggacacctacgacgcccttcacatgcaggccctgccccctcgctaa

SEQ ID NO: 349 - DNA, 1515 bp, Artificial Sequence
  Synthetic Construct
atggctctgcctgtgaccgctctgctgctgcctctggctctgctgctgcacgccgctcgccctcaggtgaaactggaagaatctggaggaggcctggtgcaggcaggcaggtccctgaggctgtcttgcgcagcaagcgagcacacctttagctcccacgtgatgggatggttcaggcaggcaccaggcaaggagagagagtccgtggccgtgatcggctggagggacatctccacatcttacgccgattccgtgaagggccggtttaccatcagccgggacaacgccaagaagacactgtatctgcagatgaacagcctgaagcctgaggacaccgccgtgtactattgcgcagcaaggagaatcgatgcagcagacttcgattcttggggccagggcacccaggtgacagtgtctagcggaggaggaggatccggaggaggaggatctggcggcggcggctccggcggcggcggctccgccgtgcagctggtggagtctggcggcggcctggtgcaggccggcgacagcctgaggctgacctgtacagcctctggcagagccttcagcacctactttatggcctggtttagacaggcccctggcaaggagagggagtttgtggcaggaatcgcatggagcggaggatccacagcatacgccgacagcgtgaagggcaggttcaccatctcccgcgataacgccaagaatacagtgtatctgcagatgaactctctgaagagcgaggatacagccgtgtactattgtgccagccgggggattgaagtggaagaatttggggcatgggggcaggggactcaggtcaccgtcagtagcactagtaccacgacgccagcgccgcgaccaccaacaccggcgcccaccatcgcgtcgcagcccctgtccctgcgcccagaggcgtgccggccagcggcggggggcgcagtgcacacgagggggctggacttcgcctgtgatatctacatctgggcgcccttggccgggacttgtggggtccttctcctgtcactggttatcaccctttactgcaaacggggcagaaagaaactcctgtatatattcaaacaaccatttatgagaccagtacaaactactcaagaggaagatggctgtagctgccgatttccagaagaagaagaaggaggatgtgaactgagagtgaagttcagcaggagcgcagacgcccccgcgtaccagcagggccagaaccagctctataacgagctcaatctaggacgaagagaggagtacgatgttttggacaagagacgtggccgggaccctgagatggggggaaagccgagaaggaagaaccctcaggaaggcctgtacaatgaactgcagaaagataagatggcggaggcctacagtgagattgggatgaaaggcgagcgccggaggggcaaggggcacgatggcctttaccagggtctcagtacagccaccaaggacacctacgacgcccttcacatgcaggccctgccccctcgctaa

SEQ ID NO: 350 - DNA, 1470 bp, Artificial Sequence
  Synthetic Construct
atggctctgcccgtcaccgctctgctgctgcctctggctctgctgctgcacgctgctcgccctgaggtgcagctggtggagtctgggggaggaatggtgcaggctggggactctctgagactatcctgtgtgcagtctacttacaccgtcaatagcgatgtcatgggctggttccgccaggctccagggaaggagcgtgagtttgtaggagcgattatgtggaatgatggtattacatacttgcaagactccgtgaagggccgatttaccatcttcagagacaacgccaagaacacggtgtatctgcaaatgaacagcctgaaacttgaggatacggccgtttattactgtgcagcatccaagggtagatactcggaatatgagtactggggccaggggacccaggtcaccgtctcctcaggaggaggaggatctgcggtgcagctggtggagtctgggggaggattggtgcaggctggggactctctgagactcacctgtacagcctctggacgcgccttcagtacctatttcatggcctggttccgccaggctccagggaaggagcgtgagtttgtagcaggaattgcatggagtggtggtagcacggcgtatgcagactccgtgaagggccgattcaccatctccagagacaacgccaagaacacggtgtatctgcaaatgaacagcctgaaatctgaggacacggccgtttattactgtgccagcagggggattgaggtcgaagagtttggtgcctggggccaggggacccaggtcaccgtctcgtcgactagtaccacgacgccagcgccgcgaccaccaacaccggcgcccaccatcgcgtcgcagcccctgtccctgcgcccagaggcgtgccggccagcggcggggggcgcagtgcacacgagggggctggacttcgcctgtgatatctacatctgggcgcccttggccgggacttgtggggtccttctcctgtcactggttatcaccctttactgcaaacggggcagaaagaaactcctgtatatattcaaacaaccatttatgagaccagtacaaactactcaagaggaagatggctgtagctgccgatttccagaagaagaagaaggaggatgtgaactgagagtgaagttcagcaggagcgcagacgcccccgcgtaccagcagggccagaaccagctctataacgagctcaatctaggacgaagagaggagtacgatgttttggacaagagacgtggccgggaccctgagatggggggaaagccgagaaggaagaaccctcaggaaggcctgtacaatgaactgcagaaagataagatggcggaggcctacagtgagattgggatgaaaggcgagcgccggaggggcaaggggcacgatggcctttaccagggtctcagtacagccaccaaggacacctacgacgcccttcacatgcaggccctgccccctcgctaa

SEQ ID NO: 351 - DNA, 1500 bp, Artificial Sequence
  Synthetic Construct
atggctctgcccgtcaccgctctgctgctgcctctggctctgctgctgcacgctgctcgccctgaggtgcagctggtggagtctgggggaggaatggtgcaggctggggactctctgagactatcctgtgtgcagtctacttacaccgtcaatagcgatgtcatgggctggttccgccaggctccagggaaggagcgtgagtttgtaggagcgattatgtggaatgatggtattacatacttgcaagactccgtgaagggccgatttaccatcttcagagacaacgccaagaacacggtgtatctgcaaatgaacagcctgaaacttgaggatacggccgtttattactgtgcagcatccaagggtagatactcggaatatgagtactggggccaggggacccaggtcaccgtctcctcaggaggaggaggatctggaggaggaggaagcggaggaggaggatccgcggtgcagctggtggagtctgggggaggattggtgcaggctggggactctctgagactcacctgtacagcctctggacgcgccttcagtacctatttcatggcctggttccgccaggctccagggaaggagcgtgagtttgtagcaggaattgcatggagtggtggtagcacggcgtatgcagactccgtgaagggccgattcaccatctccagagacaacgccaagaacacggtgtatctgcaaatgaacagcctgaaatctgaggacacggccgtttattactgtgccagcagggggattgaggtcgaagagtttggtgcctggggccaggggacccaggtcaccgtctcgtcgactagtaccacgacgccagcgccgcgaccaccaacaccggcgcccaccatcgcgtcgcagcccctgtccctgcgcccagaggcgtgccggccagcggcggggggcgcagtgcacacgagggggctggacttcgcctgtgatatctacatctgggcgcccttggccgggacttgtggggtccttctcctgtcactggttatcaccctttactgcaaacggggcagaaagaaactcctgtatatattcaaacaaccatttatgagaccagtacaaactactcaagaggaagatggctgtagctgccgatttccagaagaagaagaaggaggatgtgaactgagagtgaagttcagcaggagcgcagacgcccccgcgtaccagcagggccagaaccagctctataacgagctcaatctaggacgaagagaggagtacgatgttttggacaagagacgtggccgggaccctgagatggggggaaagccgagaaggaagaaccctcaggaaggcctgtacaatgaactgcagaaagataagatggcggaggcctacagtgagattgggatgaaaggcgagcgccggaggggcaaggggcacgatggcctttaccagggtctcagtacagccaccaaggacacctacgacgcccttcacatgcaggccctgccccctcgctaa

SEQ ID NO: 352 - DNA, 1530 bp, Artificial Sequence
  Synthetic Construct
atggctctgcccgtcaccgctctgctgctgcctctggctctgctgctgcacgctgctcgccctgaggtgcagctggtggagtctgggggaggaatggtgcaggctggggactctctgagactatcctgtgtgcagtctacttacaccgtcaatagcgatgtcatgggctggttccgccaggctccagggaaggagcgtgagtttgtaggagcgattatgtggaatgatggtattacatacttgcaagactccgtgaagggccgatttaccatcttcagagacaacgccaagaacacggtgtatctgcaaatgaacagcctgaaacttgaggatacggccgtttattactgtgcagcatccaagggtagatactcggaatatgagtactggggccaggggacccaggtcaccgtctcctcaggaggaggaggatctggaggaggaggaagcggaggaggaggaagcggcggcggcggctctggcggcggcggcagcgcggtgcagctggtggagtctgggggaggattggtgcaggctggggactctctgagactcacctgtacagcctctggacgcgccttcagtacctatttcatggcctggttccgccaggctccagggaaggagcgtgagtttgtagcaggaattgcatggagtggtggtagcacggcgtatgcagactccgtgaagggccgattcaccatctccagagacaacgccaagaacacggtgtatctgcaaatgaacagcctgaaatctgaggacacggccgtttattactgtgccagcagggggattgaggtcgaagagtttggtgcctggggccaggggacccaggtcaccgtctcgtcgactagtaccacgacgccagcgccgcgaccaccaacaccggcgcccaccatcgcgtcgcagcccctgtccctgcgcccagaggcgtgccggccagcggcggggggcgcagtgcacacgagggggctggacttcgcctgtgatatctacatctgggcgcccttggccgggacttgtggggtccttctcctgtcactggttatcaccctttactgcaaacggggcagaaagaaactcctgtatatattcaaacaaccatttatgagaccagtacaaactactcaagaggaagatggctgtagctgccgatttccagaagaagaagaaggaggatgtgaactgagagtgaagttcagcaggagcgcagacgcccccgcgtaccagcagggccagaaccagctctataacgagctcaatctaggacgaagagaggagtacgatgttttggacaagagacgtggccgggaccctgagatggggggaaagccgagaaggaagaaccctcaggaaggcctgtacaatgaactgcagaaagataagatggcggaggcctacagtgagattgggatgaaaggcgagcgccggaggggcaaggggcacgatggcctttaccagggtctcagtacagccaccaaggacacctacgacgcccttcacatgcaggccctgccccctcgctaa

SEQ ID NO: 353 - DNA, 1485 bp, Artificial Sequence
  Synthetic Construct
atggctctgcccgtcaccgctctgctgctgcctctggctctgctgctgcacgctgctcgccctgaggtgcagctggtggagtctgggggaggaatggtgcaggctggggactctctgagactatcctgtgtgcagtctacttacaccgtcaatagcgatgtcatgggctggttccgccaggctccagggaaggagcgtgagtttgtaggagcgattatgtggaatgatggtattacatacttgcaagactccgtgaagggccgatttaccatcttcagagacaacgccaagaacacggtgtatctgcaaatgaacagcctgaaacttgaggatacggccgtttattactgtgcagcatccaagggtagatactcggaatatgagtactggggccaggggacccaggtcaccgtctcctcaggaggaggaggatccggcggaggaggctctgcggtgcagctggtggagtctgggggaggattggtgcaggctggggactctctgagactcacctgtacagcctctggacgcgccttcagtacctatttcatggcctggttccgccaggctccagggaaggagcgtgagtttgtagcaggaattgcatggagtggtggtagcacggcgtatgcagactccgtgaagggccgattcaccatctccagagacaacgccaagaacacggtgtatctgcaaatgaacagcctgaaatctgaggacacggccgtttattactgtgccagcagggggattgaggtcgaagagtttggtgcctggggccaggggacccaggtcaccgtctcgtcgactagtaccacgacgccagcgccgcgaccaccaacaccggcgcccaccatcgcgtcgcagcccctgtccctgcgcccagaggcgtgccggccagcggcggggggcgcagtgcacacgagggggctggacttcgcctgtgatatctacatctgggcgcccttggccgggacttgtggggtccttctcctgtcactggttatcaccctttactgcaaacggggcagaaagaaactcctgtatatattcaaacaaccatttatgagaccagtacaaactactcaagaggaagatggctgtagctgccgatttccagaagaagaagaaggaggatgtgaactgagagtgaagttcagcaggagcgcagacgcccccgcgtaccagcagggccagaaccagctctataacgagctcaatctaggacgaagagaggagtacgatgttttggacaagagacgtggccgggaccctgagatggggggaaagccgagaaggaagaaccctcaggaaggcctgtacaatgaactgcagaaagataagatggcggaggcctacagtgagattgggatgaaaggcgagcgccggaggggcaaggggcacgatggcctttaccagggtctcagtacagccaccaaggacacctacgacgcccttcacatgcaggccctgccccctcgctaa

SEQ ID NO: 354 - DNA, 1500 bp, Artificial Sequence
  Synthetic Construct
atggctctgcccgtcaccgctctgctgctgcctctggctctgctgctgcacgctgctcgccctgaggtgcagctggtggagtctgggggaggaatggtgcaggctggggactctctgagactatcctgtgtgcagtctacttacaccgtcaatagcgatgtcatgggctggttccgccaggctccagggaaggagcgtgagtttgtaggagcgattatgtggaatgatggtattacatacttgcaagactccgtgaagggccgatttaccatcttcagagacaacgccaagaacacggtgtatctgcaaatgaacagcctgaaacttgaggatacggccgtttattactgtgcagcatccaagggtagatactcggaatatgagtactggggccaggggacccaggtcaccgtctcctcaggaggaggaggatccggcggaggaggctctggcggcggcggcagcgcggtgcagctggtggagtctgggggaggattggtgcaggctggggactctctgagactcacctgtacagcctctggacgcgccttcagtacctatttcatggcctggttccgccaggctccagggaaggagcgtgagtttgtagcaggaattgcatggagtggtggtagcacggcgtatgcagactccgtgaagggccgattcaccatctccagagacaacgccaagaacacggtgtatctgcaaatgaacagcctgaaatctgaggacacggccgtttattactgtgccagcagggggattgaggtcgaagagtttggtgcctggggccaggggacccaggtcaccgtctcgtcgactagtaccacgacgccagcgccgcgaccaccaacaccggcgcccaccatcgcgtcgcagcccctgtccctgcgcccagaggcgtgccggccagcggcggggggcgcagtgcacacgagggggctggacttcgcctgtgatatctacatctgggcgcccttggccgggacttgtggggtccttctcctgtcactggttatcaccctttactgcaaacggggcagaaagaaactcctgtatatattcaaacaaccatttatgagaccagtacaaactactcaagaggaagatggctgtagctgccgatttccagaagaagaagaaggaggatgtgaactgagagtgaagttcagcaggagcgcagacgcccccgcgtaccagcagggccagaaccagctctataacgagctcaatctaggacgaagagaggagtacgatgttttggacaagagacgtggccgggaccctgagatggggggaaagccgagaaggaagaaccctcaggaaggcctgtacaatgaactgcagaaagataagatggcggaggcctacagtgagattgggatgaaaggcgagcgccggaggggcaaggggcacgatggcctttaccagggtctcagtacagccaccaaggacacctacgacgcccttcacatgcaggccctgccccctcgctaa

SEQ ID NO: 355 - DNA, 1515 bp, Artificial Sequence
  Synthetic Construct
atggctctgcccgtcaccgctctgctgctgcctctggctctgctgctgcacgctgctcgccctgaggtgcagctggtggagtctgggggaggaatggtgcaggctggggactctctgagactatcctgtgtgcagtctacttacaccgtcaatagcgatgtcatgggctggttccgccaggctccagggaaggagcgtgagtttgtaggagcgattatgtggaatgatggtattacatacttgcaagactccgtgaagggccgatttaccatcttcagagacaacgccaagaacacggtgtatctgcaaatgaacagcctgaaacttgaggatacggccgtttattactgtgcagcatccaagggtagatactcggaatatgagtactggggccaggggacccaggtcaccgtctcctcaggaggaggaggatccggcggaggaggctctggcggcggcggctccggcggcggcggctccgcggtgcagctggtggagtctgggggaggattggtgcaggctggggactctctgagactcacctgtacagcctctggacgcgccttcagtacctatttcatggcctggttccgccaggctccagggaaggagcgtgagtttgtagcaggaattgcatggagtggtggtagcacggcgtatgcagactccgtgaagggccgattcaccatctccagagacaacgccaagaacacggtgtatctgcaaatgaacagcctgaaatctgaggacacggccgtttattactgtgccagcagggggattgaggtcgaagagtttggtgcctggggccaggggacccaggtcaccgtctcgtcgactagtaccacgacgccagcgccgcgaccaccaacaccggcgcccaccatcgcgtcgcagcccctgtccctgcgcccagaggcgtgccggccagcggcggggggcgcagtgcacacgagggggctggacttcgcctgtgatatctacatctgggcgcccttggccgggacttgtggggtccttctcctgtcactggttatcaccctttactgcaaacggggcagaaagaaactcctgtatatattcaaacaaccatttatgagaccagtacaaactactcaagaggaagatggctgtagctgccgatttccagaagaagaagaaggaggatgtgaactgagagtgaagttcagcaggagcgcagacgcccccgcgtaccagcagggccagaaccagctctataacgagctcaatctaggacgaagagaggagtacgatgttttggacaagagacgtggccgggaccctgagatggggggaaagccgagaaggaagaaccctcaggaaggcctgtacaatgaactgcagaaagataagatggcggaggcctacagtgagattgggatgaaaggcgagcgccggaggggcaaggggcacgatggcctttaccagggtctcagtacagccaccaaggacacctacgacgcccttcacatgcaggccctgccccctcgctaa

SEQ ID NO: 356 - DNA, 1479 bp, Artificial Sequence
  Synthetic Construct
atggctctgcccgtcaccgctctgctgctgcctctggctctgctgctgcacgctgctcgccctcaggtaaagctggaggagtctgggggaggattggtgcaggctgggggctctctgagactctcctgtgcagcctctggaggcaccttaagtaagaataccgtggcttgggtccgccaggctccagggaaggagcgtgggtttgtaacgtctattacctgtgatggtcgtacgacatactatgcgaactccgtaaacggccgattccccatcaaccgaaacaacgccgagaatttggtggttttgcaaatgaacagcctgaaacctgacgacacggccctttattactgtgcagcataccggaagtcaataatgtctattcagcccgactactggggccaggggacccaggtcaccgtctcctcaggaggaggaggatctcaggtacagctggtggagtctgggggaggattggtgcaggctgggggctctctgagactctcctgtgcagcctctggaggcaccttaagtaaaaataccgtggcttggttccgccaggctccagggaaggagcgtgggtttgtagcgtctattacctgggatggtcgtacgacatactatgcagactccgtgaagggccgattcaccatctccagagacaacgccaagaacacagtgtatctgcaaatgaacagcctgaaacctgaggatacggccgtttatgtctgtgcagacttagggaaatggcctgcgggcccggcggactactggggccaggggacccaggtcaccgtctcctcaactagtaccacgacgccagcgccgcgaccaccaacaccggcgcccaccatcgcgtcgcagcccctgtccctgcgcccagaggcgtgccggccagcggcggggggcgcagtgcacacgagggggctggacttcgcctgtgatatctacatctgggcgcccttggccgggacttgtggggtccttctcctgtcactggttatcaccctttactgcaaacggggcagaaagaaactcctgtatatattcaaacaaccatttatgagaccagtacaaactactcaagaggaagatggctgtagctgccgatttccagaagaagaagaaggaggatgtgaactgagagtgaagttcagcaggagcgcagacgcccccgcgtaccagcagggccagaaccagctctataacgagctcaatctaggacgaagagaggagtacgatgttttggacaagagacgtggccgggaccctgagatggggggaaagccgagaaggaagaaccctcaggaaggcctgtacaatgaactgcagaaagataagatggcggaggcctacagtgagattgggatgaaaggcgagcgccggaggggcaaggggcacgatggcctttaccagggtctcagtacagccaccaaggacacctacgacgcccttcacatgcaggccctgccccctcgctaa

SEQ ID NO: 357 - DNA, 1509 bp, Artificial Sequence
  Synthetic Construct
atggctctgcccgtcaccgctctgctgctgcctctggctctgctgctgcacgctgctcgccctcaggtaaagctggaggagtctgggggaggattggtgcaggctgggggctctctgagactctcctgtgcagcctctggaggcaccttaagtaagaataccgtggcttgggtccgccaggctccagggaaggagcgtgggtttgtaacgtctattacctgtgatggtcgtacgacatactatgcgaactccgtaaacggccgattccccatcaaccgaaacaacgccgagaatttggtggttttgcaaatgaacagcctgaaacctgacgacacggccctttattactgtgcagcataccggaagtcaataatgtctattcagcccgactactggggccaggggacccaggtcaccgtctcctcaggaggaggaggatctggaggaggaggaagcggaggaggaggatcccaggtacagctggtggagtctgggggaggattggtgcaggctgggggctctctgagactctcctgtgcagcctctggaggcaccttaagtaaaaataccgtggcttggttccgccaggctccagggaaggagcgtgggtttgtagcgtctattacctgggatggtcgtacgacatactatgcagactccgtgaagggccgattcaccatctccagagacaacgccaagaacacagtgtatctgcaaatgaacagcctgaaacctgaggatacggccgtttatgtctgtgcagacttagggaaatggcctgcgggcccggcggactactggggccaggggacccaggtcaccgtctcctcaactagtaccacgacgccagcgccgcgaccaccaacaccggcgcccaccatcgcgtcgcagcccctgtccctgcgcccagaggcgtgccggccagcggcggggggcgcagtgcacacgagggggctggacttcgcctgtgatatctacatctgggcgcccttggccgggacttgtggggtccttctcctgtcactggttatcaccctttactgcaaacggggcagaaagaaactcctgtatatattcaaacaaccatttatgagaccagtacaaactactcaagaggaagatggctgtagctgccgatttccagaagaagaagaaggaggatgtgaactgagagtgaagttcagcaggagcgcagacgcccccgcgtaccagcagggccagaaccagctctataacgagctcaatctaggacgaagagaggagtacgatgttttggacaagagacgtggccgggaccctgagatggggggaaagccgagaaggaagaaccctcaggaaggcctgtacaatgaactgcagaaagataagatggcggaggcctacagtgagattgggatgaaaggcgagcgccggaggggcaaggggcacgatggcctttaccagggtctcagtacagccaccaaggacacctacgacgcccttcacatgcaggccctgccccctcgctaa

SEQ ID NO: 358 - DNA, 1539 bp, Artificial Sequence
  Synthetic Construct
atggctctgcccgtcaccgctctgctgctgcctctggctctgctgctgcacgctgctcgccctcaggtaaagctggaggagtctgggggaggattggtgcaggctgggggctctctgagactctcctgtgcagcctctggaggcaccttaagtaagaataccgtggcttgggtccgccaggctccagggaaggagcgtgggtttgtaacgtctattacctgtgatggtcgtacgacatactatgcgaactccgtaaacggccgattccccatcaaccgaaacaacgccgagaatttggtggttttgcaaatgaacagcctgaaacctgacgacacggccctttattactgtgcagcataccggaagtcaataatgtctattcagcccgactactggggccaggggacccaggtcaccgtctcctcaggaggaggaggatctggaggaggaggaagcggaggaggaggaagcggcggcggcggctctggcggcggcggcagccaggtacagctggtggagtctgggggaggattggtgcaggctgggggctctctgagactctcctgtgcagcctctggaggcaccttaagtaaaaataccgtggcttggttccgccaggctccagggaaggagcgtgggtttgtagcgtctattacctgggatggtcgtacgacatactatgcagactccgtgaagggccgattcaccatctccagagacaacgccaagaacacagtgtatctgcaaatgaacagcctgaaacctgaggatacggccgtttatgtctgtgcagacttagggaaatggcctgcgggcccggcggactactggggccaggggacccaggtcaccgtctcctcaactagtaccacgacgccagcgccgcgaccaccaacaccggcgcccaccatcgcgtcgcagcccctgtccctgcgcccagaggcgtgccggccagcggcggggggcgcagtgcacacgagggggctggacttcgcctgtgatatctacatctgggcgcccttggccgggacttgtggggtccttctcctgtcactggttatcaccctttactgcaaacggggcagaaagaaactcctgtatatattcaaacaaccatttatgagaccagtacaaactactcaagaggaagatggctgtagctgccgatttccagaagaagaagaaggaggatgtgaactgagagtgaagttcagcaggagcgcagacgcccccgcgtaccagcagggccagaaccagctctataacgagctcaatctaggacgaagagaggagtacgatgttttggacaagagacgtggccgggaccctgagatggggggaaagccgagaaggaagaaccctcaggaaggcctgtacaatgaactgcagaaagataagatggcggaggcctacagtgagattgggatgaaaggcgagcgccggaggggcaaggggcacgatggcctttaccagggtctcagtacagccaccaaggacacctacgacgcccttcacatgcaggccctgccccctcgctaa

SEQ ID NO: 359 - DNA, 1494 bp, Artificial Sequence
  Synthetic Construct
atggctctgcccgtcaccgctctgctgctgcctctggctctgctgctgcacgctgctcgccctcaggtaaagctggaggagtctgggggaggattggtgcaggctgggggctctctgagactctcctgtgcagcctctggaggcaccttaagtaagaataccgtggcttgggtccgccaggctccagggaaggagcgtgggtttgtaacgtctattacctgtgatggtcgtacgacatactatgcgaactccgtaaacggccgattccccatcaaccgaaacaacgccgagaatttggtggttttgcaaatgaacagcctgaaacctgacgacacggccctttattactgtgcagcataccggaagtcaataatgtctattcagcccgactactggggccaggggacccaggtcaccgtctcctcaggaggaggaggatccggcggaggaggctctcaggtacagctggtggagtctgggggaggattggtgcaggctgggggctctctgagactctcctgtgcagcctctggaggcaccttaagtaaaaataccgtggcttggttccgccaggctccagggaaggagcgtgggtttgtagcgtctattacctgggatggtcgtacgacatactatgcagactccgtgaagggccgattcaccatctccagagacaacgccaagaacacagtgtatctgcaaatgaacagcctgaaacctgaggatacggccgtttatgtctgtgcagacttagggaaatggcctgcgggcccggcggactactggggccaggggacccaggtcaccgtctcctcaactagtaccacgacgccagcgccgcgaccaccaacaccggcgcccaccatcgcgtcgcagcccctgtccctgcgcccagaggcgtgccggccagcggcggggggcgcagtgcacacgagggggctggacttcgcctgtgatatctacatctgggcgcccttggccgggacttgtggggtccttctcctgtcactggttatcaccctttactgcaaacggggcagaaagaaactcctgtatatattcaaacaaccatttatgagaccagtacaaactactcaagaggaagatggctgtagctgccgatttccagaagaagaagaaggaggatgtgaactgagagtgaagttcagcaggagcgcagacgcccccgcgtaccagcagggccagaaccagctctataacgagctcaatctaggacgaagagaggagtacgatgttttggacaagagacgtggccgggaccctgagatggggggaaagccgagaaggaagaaccctcaggaaggcctgtacaatgaactgcagaaagataagatggcggaggcctacagtgagattgggatgaaaggcgagcgccggaggggcaaggggcacgatggcctttaccagggtctcagtacagccaccaaggacacctacgacgcccttcacatgcaggccctgccccctcgctaa

SEQ ID NO: 360 - DNA, 1509 bp, Artificial Sequence
  Synthetic Construct
atggctctgcccgtcaccgctctgctgctgcctctggctctgctgctgcacgctgctcgccctcaggtaaagctggaggagtctgggggaggattggtgcaggctgggggctctctgagactctcctgtgcagcctctggaggcaccttaagtaagaataccgtggcttgggtccgccaggctccagggaaggagcgtgggtttgtaacgtctattacctgtgatggtcgtacgacatactatgcgaactccgtaaacggccgattccccatcaaccgaaacaacgccgagaatttggtggttttgcaaatgaacagcctgaaacctgacgacacggccctttattactgtgcagcataccggaagtcaataatgtctattcagcccgactactggggccaggggacccaggtcaccgtctcctcaggaggaggaggatccggcggaggaggctctggcggcggcggcagccaggtacagctggtggagtctgggggaggattggtgcaggctgggggctctctgagactctcctgtgcagcctctggaggcaccttaagtaaaaataccgtggcttggttccgccaggctccagggaaggagcgtgggtttgtagcgtctattacctgggatggtcgtacgacatactatgcagactccgtgaagggccgattcaccatctccagagacaacgccaagaacacagtgtatctgcaaatgaacagcctgaaacctgaggatacggccgtttatgtctgtgcagacttagggaaatggcctgcgggcccggcggactactggggccaggggacccaggtcaccgtctcctcaactagtaccacgacgccagcgccgcgaccaccaacaccggcgcccaccatcgcgtcgcagcccctgtccctgcgcccagaggcgtgccggccagcggcggggggcgcagtgcacacgagggggctggacttcgcctgtgatatctacatctgggcgcccttggccgggacttgtggggtccttctcctgtcactggttatcaccctttactgcaaacggggcagaaagaaactcctgtatatattcaaacaaccatttatgagaccagtacaaactactcaagaggaagatggctgtagctgccgatttccagaagaagaagaaggaggatgtgaactgagagtgaagttcagcaggagcgcagacgcccccgcgtaccagcagggccagaaccagctctataacgagctcaatctaggacgaagagaggagtacgatgttttggacaagagacgtggccgggaccctgagatggggggaaagccgagaaggaagaaccctcaggaaggcctgtacaatgaactgcagaaagataagatggcggaggcctacagtgagattgggatgaaaggcgagcgccggaggggcaaggggcacgatggcctttaccagggtctcagtacagccaccaaggacacctacgacgcccttcacatgcaggccctgccccctcgctaa

SEQ ID NO: 361 - DNA, 1524 bp, Artificial Sequence
  Synthetic Construct
atggctctgcccgtcaccgctctgctgctgcctctggctctgctgctgcacgctgctcgccctcaggtaaagctggaggagtctgggggaggattggtgcaggctgggggctctctgagactctcctgtgcagcctctggaggcaccttaagtaagaataccgtggcttgggtccgccaggctccagggaaggagcgtgggtttgtaacgtctattacctgtgatggtcgtacgacatactatgcgaactccgtaaacggccgattccccatcaaccgaaacaacgccgagaatttggtggttttgcaaatgaacagcctgaaacctgacgacacggccctttattactgtgcagcataccggaagtcaataatgtctattcagcccgactactggggccaggggacccaggtcaccgtctcctcaggaggaggaggatccggcggaggaggctctggcggcggcggctccggcggcggcggctcccaggtacagctggtggagtctgggggaggattggtgcaggctgggggctctctgagactctcctgtgcagcctctggaggcaccttaagtaaaaataccgtggcttggttccgccaggctccagggaaggagcgtgggtttgtagcgtctattacctgggatggtcgtacgacatactatgcagactccgtgaagggccgattcaccatctccagagacaacgccaagaacacagtgtatctgcaaatgaacagcctgaaacctgaggatacggccgtttatgtctgtgcagacttagggaaatggcctgcgggcccggcggactactggggccaggggacccaggtcaccgtctcctcaactagtaccacgacgccagcgccgcgaccaccaacaccggcgcccaccatcgcgtcgcagcccctgtccctgcgcccagaggcgtgccggccagcggcggggggcgcagtgcacacgagggggctggacttcgcctgtgatatctacatctgggcgcccttggccgggacttgtggggtccttctcctgtcactggttatcaccctttactgcaaacggggcagaaagaaactcctgtatatattcaaacaaccatttatgagaccagtacaaactactcaagaggaagatggctgtagctgccgatttccagaagaagaagaaggaggatgtgaactgagagtgaagttcagcaggagcgcagacgcccccgcgtaccagcagggccagaaccagctctataacgagctcaatctaggacgaagagaggagtacgatgttttggacaagagacgtggccgggaccctgagatggggggaaagccgagaaggaagaaccctcaggaaggcctgtacaatgaactgcagaaagataagatggcggaggcctacagtgagattgggatgaaaggcgagcgccggaggggcaaggggcacgatggcctttaccagggtctcagtacagccaccaaggacacctacgacgcccttcacatgcaggccctgccccctcgctaa

SEQ ID NO: 362 - DNA, 1476 bp, Artificial Sequence
  Synthetic Construct
atggctctgcccgtcaccgctctgctgctgcctctggctctgctgctgcacgctgctcgccctcaggtacagctggtggagtctgggggaggattggtgcaggctgggggctctctgagactctcctgtgcagcctctggaggcaccttaagtaaaaataccgtggcttggttccgccaggctccagggaaggagcgtgggtttgtagcgtctattacctgggatggtcgtacgacatactatgcagactccgtgaagggccgattcaccatctccagagacaacgccaagaacacagtgtatctgcaaatgaacagcctgaaacctgaggatacggccgtttatgtctgtgcagacttagggaaatggcctgcgggcccggcggactactggggccaggggacccaggtcaccgtctcctcaggaggaggaggatctgatgtgcagctggtggagtctgggggaggattggtgcaggctgggggctctctgagactctcctgtgcagcctctggaggcaccttaagtaagaataccgtggcttgggtccgccaggctccagggaaggagcgtgggtttgtaacgtctattacctgtgatggtcgtacgacatactatgcgaactccgtgaagggccgattccccatctccagagacaacgccgagaacacagtgtatctgcaaatgaacagcctgaaacctgaggatacggccggttatgtctgtgcagacttagggaagtggcctgcgggttcggcggactactggggccaggggacccacgtcaccgtctcctccactagtaccacgacgccagcgccgcgaccaccaacaccggcgcccaccatcgcgtcgcagcccctgtccctgcgcccagaggcgtgccggccagcggcggggggcgcagtgcacacgagggggctggacttcgcctgtgatatctacatctgggcgcccttggccgggacttgtggggtccttctcctgtcactggttatcaccctttactgcaaacggggcagaaagaaactcctgtatatattcaaacaaccatttatgagaccagtacaaactactcaagaggaagatggctgtagctgccgatttccagaagaagaagaaggaggatgtgaactgagagtgaagttcagcaggagcgcagacgcccccgcgtaccagcagggccagaaccagctctataacgagctcaatctaggacgaagagaggagtacgatgttttggacaagagacgtggccgggaccctgagatggggggaaagccgagaaggaagaaccctcaggaaggcctgtacaatgaactgcagaaagataagatggcggaggcctacagtgagattgggatgaaaggcgagcgccggaggggcaaggggcacgatggcctttaccagggtctcagtacagccaccaaggacacctacgacgcccttcacatgcaggccctgccccctcgctaa

SEQ ID NO: 363 - DNA, 1506 bp, Artificial Sequence
  Synthetic Construct
atggctctgcccgtcaccgctctgctgctgcctctggctctgctgctgcacgctgctcgccctcaggtacagctggtggagtctgggggaggattggtgcaggctgggggctctctgagactctcctgtgcagcctctggaggcaccttaagtaaaaataccgtggcttggttccgccaggctccagggaaggagcgtgggtttgtagcgtctattacctgggatggtcgtacgacatactatgcagactccgtgaagggccgattcaccatctccagagacaacgccaagaacacagtgtatctgcaaatgaacagcctgaaacctgaggatacggccgtttatgtctgtgcagacttagggaaatggcctgcgggcccggcggactactggggccaggggacccaggtcaccgtctcctcaggaggaggaggatctggaggaggaggaagcggaggaggaggatccgatgtgcagctggtggagtctgggggaggattggtgcaggctgggggctctctgagactctcctgtgcagcctctggaggcaccttaagtaagaataccgtggcttgggtccgccaggctccagggaaggagcgtgggtttgtaacgtctattacctgtgatggtcgtacgacatactatgcgaactccgtgaagggccgattccccatctccagagacaacgccgagaacacagtgtatctgcaaatgaacagcctgaaacctgaggatacggccggttatgtctgtgcagacttagggaagtggcctgcgggttcggcggactactggggccaggggacccacgtcaccgtctcctccactagtaccacgacgccagcgccgcgaccaccaacaccggcgcccaccatcgcgtcgcagcccctgtccctgcgcccagaggcgtgccggccagcggcggggggcgcagtgcacacgagggggctggacttcgcctgtgatatctacatctgggcgcccttggccgggacttgtggggtccttctcctgtcactggttatcaccctttactgcaaacggggcagaaagaaactcctgtatatattcaaacaaccatttatgagaccagtacaaactactcaagaggaagatggctgtagctgccgatttccagaagaagaagaaggaggatgtgaactgagagtgaagttcagcaggagcgcagacgcccccgcgtaccagcagggccagaaccagctctataacgagctcaatctaggacgaagagaggagtacgatgttttggacaagagacgtggccgggaccctgagatggggggaaagccgagaaggaagaaccctcaggaaggcctgtacaatgaactgcagaaagataagatggcggaggcctacagtgagattgggatgaaaggcgagcgccggaggggcaaggggcacgatggcctttaccagggtctcagtacagccaccaaggacacctacgacgcccttcacatgcaggccctgccccctcgctaa

SEQ ID NO: 364 - DNA, 1536 bp, Artificial Sequence
  Synthetic Construct
atggctctgcccgtcaccgctctgctgctgcctctggctctgctgctgcacgctgctcgccctcaggtacagctggtggagtctgggggaggattggtgcaggctgggggctctctgagactctcctgtgcagcctctggaggcaccttaagtaaaaataccgtggcttggttccgccaggctccagggaaggagcgtgggtttgtagcgtctattacctgggatggtcgtacgacatactatgcagactccgtgaagggccgattcaccatctccagagacaacgccaagaacacagtgtatctgcaaatgaacagcctgaaacctgaggatacggccgtttatgtctgtgcagacttagggaaatggcctgcgggcccggcggactactggggccaggggacccaggtcaccgtctcctcaggaggaggaggatctggaggaggaggaagcggaggaggaggaagcggcggcggcggctctggcggcggcggcagcgatgtgcagctggtggagtctgggggaggattggtgcaggctgggggctctctgagactctcctgtgcagcctctggaggcaccttaagtaagaataccgtggcttgggtccgccaggctccagggaaggagcgtgggtttgtaacgtctattacctgtgatggtcgtacgacatactatgcgaactccgtgaagggccgattccccatctccagagacaacgccgagaacacagtgtatctgcaaatgaacagcctgaaacctgaggatacggccggttatgtctgtgcagacttagggaagtggcctgcgggttcggcggactactggggccaggggacccacgtcaccgtctcctccactagtaccacgacgccagcgccgcgaccaccaacaccggcgcccaccatcgcgtcgcagcccctgtccctgcgcccagaggcgtgccggccagcggcggggggcgcagtgcacacgagggggctggacttcgcctgtgatatctacatctgggcgcccttggccgggacttgtggggtccttctcctgtcactggttatcaccctttactgcaaacggggcagaaagaaactcctgtatatattcaaacaaccatttatgagaccagtacaaactactcaagaggaagatggctgtagctgccgatttccagaagaagaagaaggaggatgtgaactgagagtgaagttcagcaggagcgcagacgcccccgcgtaccagcagggccagaaccagctctataacgagctcaatctaggacgaagagaggagtacgatgttttggacaagagacgtggccgggaccctgagatggggggaaagccgagaaggaagaaccctcaggaaggcctgtacaatgaactgcagaaagataagatggcggaggcctacagtgagattgggatgaaaggcgagcgccggaggggcaaggggcacgatggcctttaccagggtctcagtacagccaccaaggacacctacgacgcccttcacatgcaggccctgccccctcgctaa

SEQ ID NO: 365 - DNA, 1491 bp, Artificial Sequence
  Synthetic Construct
atggctctgcccgtcaccgctctgctgctgcctctggctctgctgctgcacgctgctcgccctcaggtacagctggtggagtctgggggaggattggtgcaggctgggggctctctgagactctcctgtgcagcctctggaggcaccttaagtaaaaataccgtggcttggttccgccaggctccagggaaggagcgtgggtttgtagcgtctattacctgggatggtcgtacgacatactatgcagactccgtgaagggccgattcaccatctccagagacaacgccaagaacacagtgtatctgcaaatgaacagcctgaaacctgaggatacggccgtttatgtctgtgcagacttagggaaatggcctgcgggcccggcggactactggggccaggggacccaggtcaccgtctcctcaggaggaggaggatccggcggaggaggctctgatgtgcagctggtggagtctgggggaggattggtgcaggctgggggctctctgagactctcctgtgcagcctctggaggcaccttaagtaagaataccgtggcttgggtccgccaggctccagggaaggagcgtgggtttgtaacgtctattacctgtgatggtcgtacgacatactatgcgaactccgtgaagggccgattccccatctccagagacaacgccgagaacacagtgtatctgcaaatgaacagcctgaaacctgaggatacggccggttatgtctgtgcagacttagggaagtggcctgcgggttcggcggactactggggccaggggacccacgtcaccgtctcctccactagtaccacgacgccagcgccgcgaccaccaacaccggcgcccaccatcgcgtcgcagcccctgtccctgcgcccagaggcgtgccggccagcggcggggggcgcagtgcacacgagggggctggacttcgcctgtgatatctacatctgggcgcccttggccgggacttgtggggtccttctcctgtcactggttatcaccctttactgcaaacggggcagaaagaaactcctgtatatattcaaacaaccatttatgagaccagtacaaactactcaagaggaagatggctgtagctgccgatttccagaagaagaagaaggaggatgtgaactgagagtgaagttcagcaggagcgcagacgcccccgcgtaccagcagggccagaaccagctctataacgagctcaatctaggacgaagagaggagtacgatgttttggacaagagacgtggccgggaccctgagatggggggaaagccgagaaggaagaaccctcaggaaggcctgtacaatgaactgcagaaagataagatggcggaggcctacagtgagattgggatgaaaggcgagcgccggaggggcaaggggcacgatggcctttaccagggtctcagtacagccaccaaggacacctacgacgcccttcacatgcaggccctgccccctcgctaa

SEQ ID NO: 366 - DNA, 1506 bp, Artificial Sequence
  Synthetic Construct
atggctctgcccgtcaccgctctgctgctgcctctggctctgctgctgcacgctgctcgccctcaggtacagctggtggagtctgggggaggattggtgcaggctgggggctctctgagactctcctgtgcagcctctggaggcaccttaagtaaaaataccgtggcttggttccgccaggctccagggaaggagcgtgggtttgtagcgtctattacctgggatggtcgtacgacatactatgcagactccgtgaagggccgattcaccatctccagagacaacgccaagaacacagtgtatctgcaaatgaacagcctgaaacctgaggatacggccgtttatgtctgtgcagacttagggaaatggcctgcgggcccggcggactactggggccaggggacccaggtcaccgtctcctcaggaggaggaggatccggcggaggaggctctggcggcggcggcagcgatgtgcagctggtggagtctgggggaggattggtgcaggctgggggctctctgagactctcctgtgcagcctctggaggcaccttaagtaagaataccgtggcttgggtccgccaggctccagggaaggagcgtgggtttgtaacgtctattacctgtgatggtcgtacgacatactatgcgaactccgtgaagggccgattccccatctccagagacaacgccgagaacacagtgtatctgcaaatgaacagcctgaaacctgaggatacggccggttatgtctgtgcagacttagggaagtggcctgcgggttcggcggactactggggccaggggacccacgtcaccgtctcctccactagtaccacgacgccagcgccgcgaccaccaacaccggcgcccaccatcgcgtcgcagcccctgtccctgcgcccagaggcgtgccggccagcggcggggggcgcagtgcacacgagggggctggacttcgcctgtgatatctacatctgggcgcccttggccgggacttgtggggtccttctcctgtcactggttatcaccctttactgcaaacggggcagaaagaaactcctgtatatattcaaacaaccatttatgagaccagtacaaactactcaagaggaagatggctgtagctgccgatttccagaagaagaagaaggaggatgtgaactgagagtgaagttcagcaggagcgcagacgcccccgcgtaccagcagggccagaaccagctctataacgagctcaatctaggacgaagagaggagtacgatgttttggacaagagacgtggccgggaccctgagatggggggaaagccgagaaggaagaaccctcaggaaggcctgtacaatgaactgcagaaagataagatggcggaggcctacagtgagattgggatgaaaggcgagcgccggaggggcaaggggcacgatggcctttaccagggtctcagtacagccaccaaggacacctacgacgcccttcacatgcaggccctgccccctcgctaa

SEQ ID NO: 367 - DNA, 1521 bp, Artificial Sequence
  Synthetic Construct
atggctctgcccgtcaccgctctgctgctgcctctggctctgctgctgcacgctgctcgccctcaggtacagctggtggagtctgggggaggattggtgcaggctgggggctctctgagactctcctgtgcagcctctggaggcaccttaagtaaaaataccgtggcttggttccgccaggctccagggaaggagcgtgggtttgtagcgtctattacctgggatggtcgtacgacatactatgcagactccgtgaagggccgattcaccatctccagagacaacgccaagaacacagtgtatctgcaaatgaacagcctgaaacctgaggatacggccgtttatgtctgtgcagacttagggaaatggcctgcgggcccggcggactactggggccaggggacccaggtcaccgtctcctcaggaggaggaggatccggcggaggaggctctggcggcggcggctccggcggcggcggctccgatgtgcagctggtggagtctgggggaggattggtgcaggctgggggctctctgagactctcctgtgcagcctctggaggcaccttaagtaagaataccgtggcttgggtccgccaggctccagggaaggagcgtgggtttgtaacgtctattacctgtgatggtcgtacgacatactatgcgaactccgtgaagggccgattccccatctccagagacaacgccgagaacacagtgtatctgcaaatgaacagcctgaaacctgaggatacggccggttatgtctgtgcagacttagggaagtggcctgcgggttcggcggactactggggccaggggacccacgtcaccgtctcctccactagtaccacgacgccagcgccgcgaccaccaacaccggcgcccaccatcgcgtcgcagcccctgtccctgcgcccagaggcgtgccggccagcggcggggggcgcagtgcacacgagggggctggacttcgcctgtgatatctacatctgggcgcccttggccgggacttgtggggtccttctcctgtcactggttatcaccctttactgcaaacggggcagaaagaaactcctgtatatattcaaacaaccatttatgagaccagtacaaactactcaagaggaagatggctgtagctgccgatttccagaagaagaagaaggaggatgtgaactgagagtgaagttcagcaggagcgcagacgcccccgcgtaccagcagggccagaaccagctctataacgagctcaatctaggacgaagagaggagtacgatgttttggacaagagacgtggccgggaccctgagatggggggaaagccgagaaggaagaaccctcaggaaggcctgtacaatgaactgcagaaagataagatggcggaggcctacagtgagattgggatgaaaggcgagcgccggaggggcaaggggcacgatggcctttaccagggtctcagtacagccaccaaggacacctacgacgcccttcacatgcaggccctgccccctcgctaa

SEQ ID NO: 368 - DNA, 1473 bp, Artificial Sequence
  Synthetic Construct
atggctctgcccgtcaccgctctgctgctgcctctggctctgctgctgcacgctgctcgccctgatgtgcagctggtggagtctgggggaggattggtgcaggctgggggctctctgagactctcctgtgcagcctctggaggcaccttaagtaagaataccgtggcttgggtccgccaggctccagggaaggagcgtgggtttgtaacgtctattacctgtgatggtcgtacgacatactatgcgaactccgtgaagggccgattccccatctccagagacaacgccgagaacacagtgtatctgcaaatgaacagcctgaaacctgaggatacggccggttatgtctgtgcagacttagggaagtggcctgcgggttcggcggactactggggccaggggacccacgtcaccgtctcctccggaggaggaggatctgatgtgcagctggtggagtctgggggaggcttggtgcagcctggggggtctctgagactctcctgtgcagcctctggacggaccttcagtagcattgtcatgggctggttccgccaggctccagggaaggagcgtgagtttgtaggagcgattatgtggaatgatggtattacatacttgcaagactccgtgaagggccgatttaccatcttcagagacaacgccaagaacacggtgtatctgcaaatgaacagcctgaaacttgaggatacggccgtttattactgtgcagcatccaagggtagatactcggaatatgagtactggggccaggggacccaggtcaccgtctcctcaactagtaccacgacgccagcgccgcgaccaccaacaccggcgcccaccatcgcgtcgcagcccctgtccctgcgcccagaggcgtgccggccagcggcggggggcgcagtgcacacgagggggctggacttcgcctgtgatatctacatctgggcgcccttggccgggacttgtggggtccttctcctgtcactggttatcaccctttactgcaaacggggcagaaagaaactcctgtatatattcaaacaaccatttatgagaccagtacaaactactcaagaggaagatggctgtagctgccgatttccagaagaagaagaaggaggatgtgaactgagagtgaagttcagcaggagcgcagacgcccccgcgtaccagcagggccagaaccagctctataacgagctcaatctaggacgaagagaggagtacgatgttttggacaagagacgtggccgggaccctgagatggggggaaagccgagaaggaagaaccctcaggaaggcctgtacaatgaactgcagaaagataagatggcggaggcctacagtgagattgggatgaaaggcgagcgccggaggggcaaggggcacgatggcctttaccagggtctcagtacagccaccaaggacacctacgacgcccttcacatgcaggccctgccccctcgctaa

SEQ ID NO: 369 - DNA, 1503 bp, Artificial Sequence
  Synthetic Construct
atggctctgcccgtcaccgctctgctgctgcctctggctctgctgctgcacgctgctcgccctgatgtgcagctggtggagtctgggggaggattggtgcaggctgggggctctctgagactctcctgtgcagcctctggaggcaccttaagtaagaataccgtggcttgggtccgccaggctccagggaaggagcgtgggtttgtaacgtctattacctgtgatggtcgtacgacatactatgcgaactccgtgaagggccgattccccatctccagagacaacgccgagaacacagtgtatctgcaaatgaacagcctgaaacctgaggatacggccggttatgtctgtgcagacttagggaagtggcctgcgggttcggcggactactggggccaggggacccacgtcaccgtctcctccggaggaggaggatctggaggaggaggaagcggaggaggaggatccgatgtgcagctggtggagtctgggggaggcttggtgcagcctggggggtctctgagactctcctgtgcagcctctggacggaccttcagtagcattgtcatgggctggttccgccaggctccagggaaggagcgtgagtttgtaggagcgattatgtggaatgatggtattacatacttgcaagactccgtgaagggccgatttaccatcttcagagacaacgccaagaacacggtgtatctgcaaatgaacagcctgaaacttgaggatacggccgtttattactgtgcagcatccaagggtagatactcggaatatgagtactggggccaggggacccaggtcaccgtctcctcaactagtaccacgacgccagcgccgcgaccaccaacaccggcgcccaccatcgcgtcgcagcccctgtccctgcgcccagaggcgtgccggccagcggcggggggcgcagtgcacacgagggggctggacttcgcctgtgatatctacatctgggcgcccttggccgggacttgtggggtccttctcctgtcactggttatcaccctttactgcaaacggggcagaaagaaactcctgtatatattcaaacaaccatttatgagaccagtacaaactactcaagaggaagatggctgtagctgccgatttccagaagaagaagaaggaggatgtgaactgagagtgaagttcagcaggagcgcagacgcccccgcgtaccagcagggccagaaccagctctataacgagctcaatctaggacgaagagaggagtacgatgttttggacaagagacgtggccgggaccctgagatggggggaaagccgagaaggaagaaccctcaggaaggcctgtacaatgaactgcagaaagataagatggcggaggcctacagtgagattgggatgaaaggcgagcgccggaggggcaaggggcacgatggcctttaccagggtctcagtacagccaccaaggacacctacgacgcccttcacatgcaggccctgccccctcgctaa

SEQ ID NO: 370 - DNA, 1533 bp, Artificial Sequence
  Synthetic Construct
atggctctgcccgtcaccgctctgctgctgcctctggctctgctgctgcacgctgctcgccctgatgtgcagctggtggagtctgggggaggattggtgcaggctgggggctctctgagactctcctgtgcagcctctggaggcaccttaagtaagaataccgtggcttgggtccgccaggctccagggaaggagcgtgggtttgtaacgtctattacctgtgatggtcgtacgacatactatgcgaactccgtgaagggccgattccccatctccagagacaacgccgagaacacagtgtatctgcaaatgaacagcctgaaacctgaggatacggccggttatgtctgtgcagacttagggaagtggcctgcgggttcggcggactactggggccaggggacccacgtcaccgtctcctccggaggaggaggatctggaggaggaggaagcggaggaggaggaagcggcggcggcggctctggcggcggcggcagcgatgtgcagctggtggagtctgggggaggcttggtgcagcctggggggtctctgagactctcctgtgcagcctctggacggaccttcagtagcattgtcatgggctggttccgccaggctccagggaaggagcgtgagtttgtaggagcgattatgtggaatgatggtattacatacttgcaagactccgtgaagggccgatttaccatcttcagagacaacgccaagaacacggtgtatctgcaaatgaacagcctgaaacttgaggatacggccgtttattactgtgcagcatccaagggtagatactcggaatatgagtactggggccaggggacccaggtcaccgtctcctcaactagtaccacgacgccagcgccgcgaccaccaacaccggcgcccaccatcgcgtcgcagcccctgtccctgcgcccagaggcgtgccggccagcggcggggggcgcagtgcacacgagggggctggacttcgcctgtgatatctacatctgggcgcccttggccgggacttgtggggtccttctcctgtcactggttatcaccctttactgcaaacggggcagaaagaaactcctgtatatattcaaacaaccatttatgagaccagtacaaactactcaagaggaagatggctgtagctgccgatttccagaagaagaagaaggaggatgtgaactgagagtgaagttcagcaggagcgcagacgcccccgcgtaccagcagggccagaaccagctctataacgagctcaatctaggacgaagagaggagtacgatgttttggacaagagacgtggccgggaccctgagatggggggaaagccgagaaggaagaaccctcaggaaggcctgtacaatgaactgcagaaagataagatggcggaggcctacagtgagattgggatgaaaggcgagcgccggaggggcaaggggcacgatggcctttaccagggtctcagtacagccaccaaggacacctacgacgcccttcacatgcaggccctgccccctcgctaa

SEQ ID NO: 371 - DNA, 1488 bp, Artificial Sequence
  Synthetic Construct
atggctctgcccgtcaccgctctgctgctgcctctggctctgctgctgcacgctgctcgccctgatgtgcagctggtggagtctgggggaggattggtgcaggctgggggctctctgagactctcctgtgcagcctctggaggcaccttaagtaagaataccgtggcttgggtccgccaggctccagggaaggagcgtgggtttgtaacgtctattacctgtgatggtcgtacgacatactatgcgaactccgtgaagggccgattccccatctccagagacaacgccgagaacacagtgtatctgcaaatgaacagcctgaaacctgaggatacggccggttatgtctgtgcagacttagggaagtggcctgcgggttcggcggactactggggccaggggacccacgtcaccgtctcctccggaggaggaggatccggcggaggaggctctgatgtgcagctggtggagtctgggggaggcttggtgcagcctggggggtctctgagactctcctgtgcagcctctggacggaccttcagtagcattgtcatgggctggttccgccaggctccagggaaggagcgtgagtttgtaggagcgattatgtggaatgatggtattacatacttgcaagactccgtgaagggccgatttaccatcttcagagacaacgccaagaacacggtgtatctgcaaatgaacagcctgaaacttgaggatacggccgtttattactgtgcagcatccaagggtagatactcggaatatgagtactggggccaggggacccaggtcaccgtctcctcaactagtaccacgacgccagcgccgcgaccaccaacaccggcgcccaccatcgcgtcgcagcccctgtccctgcgcccagaggcgtgccggccagcggcggggggcgcagtgcacacgagggggctggacttcgcctgtgatatctacatctgggcgcccttggccgggacttgtggggtccttctcctgtcactggttatcaccctttactgcaaacggggcagaaagaaactcctgtatatattcaaacaaccatttatgagaccagtacaaactactcaagaggaagatggctgtagctgccgatttccagaagaagaagaaggaggatgtgaactgagagtgaagttcagcaggagcgcagacgcccccgcgtaccagcagggccagaaccagctctataacgagctcaatctaggacgaagagaggagtacgatgttttggacaagagacgtggccgggaccctgagatggggggaaagccgagaaggaagaaccctcaggaaggcctgtacaatgaactgcagaaagataagatggcggaggcctacagtgagattgggatgaaaggcgagcgccggaggggcaaggggcacgatggcctttaccagggtctcagtacagccaccaaggacacctacgacgcccttcacatgcaggccctgccccctcgctaa

SEQ ID NO: 372 - DNA, 1503 bp, Artificial Sequence
  Synthetic Construct
atggctctgcccgtcaccgctctgctgctgcctctggctctgctgctgcacgctgctcgccctgatgtgcagctggtggagtctgggggaggattggtgcaggctgggggctctctgagactctcctgtgcagcctctggaggcaccttaagtaagaataccgtggcttgggtccgccaggctccagggaaggagcgtgggtttgtaacgtctattacctgtgatggtcgtacgacatactatgcgaactccgtgaagggccgattccccatctccagagacaacgccgagaacacagtgtatctgcaaatgaacagcctgaaacctgaggatacggccggttatgtctgtgcagacttagggaagtggcctgcgggttcggcggactactggggccaggggacccacgtcaccgtctcctccggaggaggaggatccggcggaggaggctctggcggcggcggcagcgatgtgcagctggtggagtctgggggaggcttggtgcagcctggggggtctctgagactctcctgtgcagcctctggacggaccttcagtagcattgtcatgggctggttccgccaggctccagggaaggagcgtgagtttgtaggagcgattatgtggaatgatggtattacatacttgcaagactccgtgaagggccgatttaccatcttcagagacaacgccaagaacacggtgtatctgcaaatgaacagcctgaaacttgaggatacggccgtttattactgtgcagcatccaagggtagatactcggaatatgagtactggggccaggggacccaggtcaccgtctcctcaactagtaccacgacgccagcgccgcgaccaccaacaccggcgcccaccatcgcgtcgcagcccctgtccctgcgcccagaggcgtgccggccagcggcggggggcgcagtgcacacgagggggctggacttcgcctgtgatatctacatctgggcgcccttggccgggacttgtggggtccttctcctgtcactggttatcaccctttactgcaaacggggcagaaagaaactcctgtatatattcaaacaaccatttatgagaccagtacaaactactcaagaggaagatggctgtagctgccgatttccagaagaagaagaaggaggatgtgaactgagagtgaagttcagcaggagcgcagacgcccccgcgtaccagcagggccagaaccagctctataacgagctcaatctaggacgaagagaggagtacgatgttttggacaagagacgtggccgggaccctgagatggggggaaagccgagaaggaagaaccctcaggaaggcctgtacaatgaactgcagaaagataagatggcggaggcctacagtgagattgggatgaaaggcgagcgccggaggggcaaggggcacgatggcctttaccagggtctcagtacagccaccaaggacacctacgacgcccttcacatgcaggccctgccccctcgctaa

SEQ ID NO: 373 - DNA, 1518 bp, Artificial Sequence
  Synthetic Construct
atggctctgcccgtcaccgctctgctgctgcctctggctctgctgctgcacgctgctcgccctgatgtgcagctggtggagtctgggggaggattggtgcaggctgggggctctctgagactctcctgtgcagcctctggaggcaccttaagtaagaataccgtggcttgggtccgccaggctccagggaaggagcgtgggtttgtaacgtctattacctgtgatggtcgtacgacatactatgcgaactccgtgaagggccgattccccatctccagagacaacgccgagaacacagtgtatctgcaaatgaacagcctgaaacctgaggatacggccggttatgtctgtgcagacttagggaagtggcctgcgggttcggcggactactggggccaggggacccacgtcaccgtctcctccggaggaggaggatccggcggaggaggctctggcggcggcggctccggcggcggcggctccgatgtgcagctggtggagtctgggggaggcttggtgcagcctggggggtctctgagactctcctgtgcagcctctggacggaccttcagtagcattgtcatgggctggttccgccaggctccagggaaggagcgtgagtttgtaggagcgattatgtggaatgatggtattacatacttgcaagactccgtgaagggccgatttaccatcttcagagacaacgccaagaacacggtgtatctgcaaatgaacagcctgaaacttgaggatacggccgtttattactgtgcagcatccaagggtagatactcggaatatgagtactggggccaggggacccaggtcaccgtctcctcaactagtaccacgacgccagcgccgcgaccaccaacaccggcgcccaccatcgcgtcgcagcccctgtccctgcgcccagaggcgtgccggccagcggcggggggcgcagtgcacacgagggggctggacttcgcctgtgatatctacatctgggcgcccttggccgggacttgtggggtccttctcctgtcactggttatcaccctttactgcaaacggggcagaaagaaactcctgtatatattcaaacaaccatttatgagaccagtacaaactactcaagaggaagatggctgtagctgccgatttccagaagaagaagaaggaggatgtgaactgagagtgaagttcagcaggagcgcagacgcccccgcgtaccagcagggccagaaccagctctataacgagctcaatctaggacgaagagaggagtacgatgttttggacaagagacgtggccgggaccctgagatggggggaaagccgagaaggaagaaccctcaggaaggcctgtacaatgaactgcagaaagataagatggcggaggcctacagtgagattgggatgaaaggcgagcgccggaggggcaaggggcacgatggcctttaccagggtctcagtacagccaccaaggacacctacgacgcccttcacatgcaggccctgccccctcgctaa

SEQ ID NO: 374 - DNA, 23 bp, Artificial Sequence
  Synthetic Construct
gtcctggctgctcttctacaagg

SEQ ID NO: 375 - DNA, 23 bp, Artificial Sequence
  Synthetic Construct
ggtacgtgctgttgaactgttcc

SEQ ID NO: 376 - DNA, 29 bp, Artificial Sequence
  Synthetic Construct
gatgtgcagctgcaggagtctggaggagg

SEQ ID NO: 377 - DNA, 29 bp, Artificial Sequence
  Synthetic Construct
gatgtgcagctgcaggagtctgggggagg

SEQ ID NO: 378 - DNA, 34 bp, Artificial Sequence
  Synthetic Construct
ctagtgcggccgctgaggagacggtgacctgggt

SEQ ID NO: 379 - DNA, 9 bp, Artificial Sequence
  Synthetic Construct
gccgccacc

SEQ ID NO: 380 - DNA, 6 bp, Artificial Sequence
  Synthetic Construct
gaattc

SEQ ID NO: 381 - DNA, 6 bp, Artificial Sequence
  Synthetic Construct
actagt

SEQ ID NO: 382 - DNA, 6 bp, Artificial Sequence
  Synthetic Construct
gttaac

SEQ ID NO: 383 - DNA, 6 bp, Artificial Sequence
  Synthetic Construct
acgcgt

SEQ ID NO: 384 - DNA, 6 bp, Artificial Sequence
  Synthetic Construct
atgcat

SEQ ID NO: 385 - protein, 21 aa, Artificial Sequence
  Synthetic Construct
GSGEGRGSLLTCGDVEENPGP

SEQ ID NO: 386 - protein, 18 aa, Homo sapiens
MKWVTFISLLFLFSSAYS

SEQ ID NO: 387 - protein, 9 aa, Artificial Sequence
  Synthetic Construct
GSGHHHHHH

SEQ ID NO: 388 - protein, 10 aa, Artificial Sequence
  Synthetic Construct
MLQMAGQCSQ

SEQ ID NO: 389 - protein, 14 aa, Artificial Sequence
  Synthetic Construct
CSQNEYFDSLLHAC

SEQ ID NO: 390 - protein, 13 aa, Artificial Sequence
  Synthetic Construct
NEYFDSLLHACIP

SEQ ID NO: 391 - protein, 11 aa, Artificial Sequence
  Synthetic Construct
ACIPCQLRCSS

SEQ ID NO: 392 - protein, 19 aa, Artificial Sequence
  Synthetic Construct
CQLRCSSNTPPLTCQRYCN

SEQ ID NO: 393 - protein, 10 aa, Artificial Sequence
  Synthetic Construct
LTCQRYCNAS

SEQ ID NO: 394 - protein, 12 aa, Artificial Sequence
  Synthetic Construct
ASVTNSVKGTNA

SEQ ID NO: 395 - protein, 54 aa, Artificial Sequence
  Synthetic Construct
MLQMAGQCSQNEYFDSLLHACIPCQLRCSSNTPPLTCQRYCNASVTNSVKGTNA

SEQ ID NO: 396 - protein, 23 aa, Artificial Sequence
  Synthetic Construct
ILWTCLGLSLIISLAVFVLMFLL

SEQ ID NO: 397 - protein, 107 aa, Artificial Sequence
  Synthetic Construct
RKINSEPLKDEFKNTGSGLLGMANIDLEKSRTGDEIILPRGLEYTVEECTCEDCIKSKPKVDSDHCFPLPAMEEGATILVTTKTNDYCKSLPAALSATEIEKSISAR

SEQ ID NO: 398 - DNA, 23 bp, Artificial Sequence
  Synthetic Construct
gtccttctcctgtcactggttat

SEQ ID NO: 399 - DNA, 23 bp, Artificial Sequence
  Synthetic Construct
tcttcttcttctggaaatcggca